European Patent Specification EP 3 893 913 B1, published March 26, 2025. Title: TRANSFERRIN RECEPTOR TARGETING PEPTIDES. Applicant: FRED HUTCHINSON CANCER RESEARCH CENTER. The sequence listing filed with the application follows.

SEQUENCE LISTING (457 sequences)

SEQ ID NO: 1 - protein, 51 aa, Artificial Sequence
  Description of Artificial Sequence: Synthetic polypeptide
GSREGCASRCTKYNAELEKCEARVSSMSNTEETCVQELFDLLHCVDHCVSQ

SEQ ID NO: 2 - protein, 51 aa, Artificial Sequence
  Description of Artificial Sequence: Synthetic polypeptide
GSREGCASRCTKYNAELEKCEARVMSMSNTEEDCEQELEDLLHCLDHCHSQ

SEQ ID NO: 3 - protein, 51 aa, Artificial Sequence
  Description of Artificial Sequence: Synthetic polypeptide
GSREGCASRCTKYNAELEKCEARVVSMSNTEEDCEQELEDLLHCLDHCHSQ

SEQ ID NO: 4 - protein, 51 aa, Artificial Sequence
  Description of Artificial Sequence: Synthetic polypeptide
GSREGCASRCTKYNAELEKCEARVMSMSNTEETCEQELEDLLHCLDHCHSQ

SEQ ID NO: 5 - protein, 51 aa, Artificial Sequence
  Description of Artificial Sequence: Synthetic polypeptide
GSREGCASRCTKYNAELEKCEARVMSMSNTEEDCVQELEDLLHCLDHCHSQ

SEQ ID NO: 6 - protein, 51 aa, Artificial Sequence
  Description of Artificial Sequence: Synthetic polypeptide
GSREGCASRCTKYNAELEKCEARVMSMSNTEEDCEQELFDLLHCLDHCHSQ

SEQ ID NO: 7 - protein, 51 aa, Artificial Sequence
  Description of Artificial Sequence: Synthetic polypeptide
GSREGCASRCTKYNAELEKCEARVMSMSNTEEDCEQELEDLLHCVDHCHSQ

SEQ ID NO: 8 - protein, 51 aa, Artificial Sequence
  Description of Artificial Sequence: Synthetic polypeptide
GSREGCASRCTKYNAELEKCEARVMSMSNTEEDCEQELEDLLHCLDHCVSQ

SEQ ID NO: 9 - protein, 51 aa, Artificial Sequence
  Description of Artificial Sequence: Synthetic polypeptide
GSREGCASRCTKYNAELEKCEARVVSMSNTEETCEQELEDLLHCLDHCHSQ

SEQ ID NO: 10 - protein, 51 aa, Artificial Sequence
  Description of Artificial Sequence: Synthetic polypeptide
GSREGCASRCTKYNAELEKCEARVVSMSNTEEDCVQELEDLLHCLDHCHSQ

SEQ ID NO: 11 - protein, 51 aa, Artificial Sequence
  Description of Artificial Sequence: Synthetic polypeptide
GSREGCASRCTKYNAELEKCEARVVSMSNTEEDCEQELFDLLHCLDHCHSQ

SEQ ID NO: 12 - protein, 51 aa, Artificial Sequence
  Description of Artificial Sequence: Synthetic polypeptide
GSREGCASRCTKYNAELEKCEARVVSMSNTEEDCEQELEDLLHCVDHCHSQ

SEQ ID NO: 13 - protein, 51 aa, Artificial Sequence
  Description of Artificial Sequence: Synthetic polypeptide
GSREGCASRCTKYNAELEKCEARVVSMSNTEEDCEQELEDLLHCLDHCVSQ

SEQ ID NO: 14 - protein, 51 aa, Artificial Sequence
  Description of Artificial Sequence: Synthetic polypeptide
GSREGCASRCTKYNAELEKCEARVMSMSNTEETCVQELEDLLHCLDHCHSQ

SEQ ID NO: 15 - protein, 51 aa, Artificial Sequence
  Description of Artificial Sequence: Synthetic polypeptide
GSREGCASRCTKYNAELEKCEARVMSMSNTEETCEQELFDLLHCLDHCHSQ

SEQ ID NO: 16 - protein, 51 aa, Artificial Sequence
  Description of Artificial Sequence: Synthetic polypeptide
GSREGCASRCTKYNAELEKCEARVMSMSNTEETCEQELEDLLHCVDHCHSQ

SEQ ID NO: 17 - protein, 51 aa, Artificial Sequence
  Description of Artificial Sequence: Synthetic polypeptide
GSREGCASRCTKYNAELEKCEARVMSMSNTEETCEQELEDLLHCLDHCVSQ

SEQ ID NO: 18 - protein, 51 aa, Artificial Sequence
  Description of Artificial Sequence: Synthetic polypeptide
GSREGCASRCTKYNAELEKCEARVMSMSNTEEDCVQELFDLLHCLDHCHSQ

SEQ ID NO: 19 - protein, 51 aa, Artificial Sequence
  Description of Artificial Sequence: Synthetic polypeptide
GSREGCASRCTKYNAELEKCEARVMSMSNTEEDCVQELEDLLHCVDHCHSQ

SEQ ID NO: 20 - protein, 51 aa, Artificial Sequence
  Description of Artificial Sequence: Synthetic polypeptide
GSREGCASRCTKYNAELEKCEARVMSMSNTEEDCVQELEDLLHCLDHCVSQ

SEQ ID NO: 21 - protein, 51 aa, Artificial Sequence
  Description of Artificial Sequence: Synthetic polypeptide
GSREGCASRCTKYNAELEKCEARVMSMSNTEEDCEQELFDLLHCVDHCHSQ

SEQ ID NO: 22 - protein, 51 aa, Artificial Sequence
  Description of Artificial Sequence: Synthetic polypeptide
GSREGCASRCTKYNAELEKCEARVMSMSNTEEDCEQELFDLLHCLDHCVSQ

SEQ ID NO: 23 - protein, 51 aa, Artificial Sequence
  Description of Artificial Sequence: Synthetic polypeptide
GSREGCASRCTKYNAELEKCEARVMSMSNTEEDCEQELEDLLHCVDHCVSQ

SEQ ID NO: 24 - protein, 51 aa, Artificial Sequence
  Description of Artificial Sequence: Synthetic polypeptide
GSREGCASRCMKYNAELEKCEARVMSMSNTEEDCEQELEDLLHCLDHCHSQ

SEQ ID NO: 25 - protein, 51 aa, Artificial Sequence
  Description of Artificial Sequence: Synthetic polypeptide
GSREGCASRCTKYNDELEKCEARVMSMSNTEEDCEQELEDLLHCLDHCHSQ

SEQ ID NO: 26 - protein, 51 aa, Artificial Sequence
  Description of Artificial Sequence: Synthetic polypeptide
GSREGCASRCTKYNAELEKCEARMMSMSNTEEDCEQELEDLLHCLDHCHSQ

SEQ ID NO: 27 - protein, 51 aa, Artificial Sequence
  Description of Artificial Sequence: Synthetic polypeptide
GSREGCASRCTKYNAELEKCEARVMSMSNTEEDCEQELEDLLYCLDHCHSQ

SEQ ID NO: 28 - protein, 51 aa, Artificial Sequence
  Description of Artificial Sequence: Synthetic polypeptide
GSREGCASRCMKYNDELEKCEARMMSMSNTEEDCEQELEDLLHCLDHCHSQ

SEQ ID NO: 29 - protein, 51 aa, Artificial Sequence
  Description of Artificial Sequence: Synthetic polypeptide
GSREGCASRCMKYNDELEKCEARVMSMSNTEEDCEQELEDLLYCLDHCHSQ

SEQ ID NO: 30 - protein, 51 aa, Artificial Sequence
  Description of Artificial Sequence: Synthetic polypeptide
GSREGCASRCMKYNAELEKCEARMMSMSNTEEDCEQELEDLLYCLDHCHSQ

SEQ ID NO: 31 - protein, 51 aa, Artificial Sequence
  Description of Artificial Sequence: Synthetic polypeptide
GSREGCASRCTKYNDELEKCEARMMSMSNTEEDCEQELEDLLYCLDHCHSQ

SEQ ID NO: 32 - protein, 51 aa, Artificial Sequence
  Description of Artificial Sequence: Synthetic polypeptide
GSREGCASRCMKYNDELEKCEARMMSMSNTEEDCEQELEDLLYCLDHCHSQ

SEQ ID NO: 33 - protein, 67 aa, Artificial Sequence
  Description of Artificial Sequence: Synthetic polypeptide
GSREGCASRCTKYNAELEKCEARVSSMSNTEETCVQELFDLLHCVDHCVSQGSSELYENKPRRPYIL

SEQ ID NO: 34 - protein, 67 aa, Artificial Sequence
  Description of Artificial Sequence: Synthetic polypeptide
GSREGCASRCTKYNAELEKCEARVMSMSNTEEDCEQELEDLLHCLDHCHSQGSSELYENKPRRPYIL

SEQ ID NO: 35 - protein, 67 aa, Artificial Sequence
  Description of Artificial Sequence: Synthetic polypeptide
GSREGCASRCMKYNDELEKCEARMMSMSNTEEDCEQELEDLLYCLDHCHSQGSSELYENKPRRPYIL

SEQ ID NO: 36 - protein, 49 aa, Artificial Sequence
  Description of Artificial Sequence: Synthetic polypeptide
REGCASRCTKYNAELEKCEARVSSMSNTEETCVQELFDLLHCVDHCVSQ

SEQ ID NO: 37 - protein, 49 aa, Artificial Sequence
  Description of Artificial Sequence: Synthetic polypeptide
REGCASRCTKYNAELEKCEARVMSMSNTEEDCEQELEDLLHCLDHCHSQ

SEQ ID NO: 38 - protein, 49 aa, Artificial Sequence
  Description of Artificial Sequence: Synthetic polypeptide
REGCASRCTKYNAELEKCEARVVSMSNTEEDCEQELEDLLHCLDHCHSQ

SEQ ID NO: 39 - protein, 49 aa, Artificial Sequence
  Description of Artificial Sequence: Synthetic polypeptide
REGCASRCTKYNAELEKCEARVMSMSNTEETCEQELEDLLHCLDHCHSQ

SEQ ID NO: 40 - protein, 49 aa, Artificial Sequence
  Description of Artificial Sequence: Synthetic polypeptide
REGCASRCTKYNAELEKCEARVMSMSNTEEDCVQELEDLLHCLDHCHSQ

SEQ ID NO: 41 - protein, 49 aa, Artificial Sequence
  Description of Artificial Sequence: Synthetic polypeptide
REGCASRCTKYNAELEKCEARVMSMSNTEEDCEQELFDLLHCLDHCHSQ

SEQ ID NO: 42 - protein, 49 aa, Artificial Sequence
  Description of Artificial Sequence: Synthetic polypeptide
REGCASRCTKYNAELEKCEARVMSMSNTEEDCEQELEDLLHCVDHCHSQ

SEQ ID NO: 43 - protein, 49 aa, Artificial Sequence
  Description of Artificial Sequence: Synthetic polypeptide
REGCASRCTKYNAELEKCEARVMSMSNTEEDCEQELEDLLHCLDHCVSQ

SEQ ID NO: 44 - protein, 49 aa, Artificial Sequence
  Description of Artificial Sequence: Synthetic polypeptide
REGCASRCTKYNAELEKCEARVVSMSNTEETCEQELEDLLHCLDHCHSQ

SEQ ID NO: 45 - protein, 49 aa, Artificial Sequence
  Description of Artificial Sequence: Synthetic polypeptide
REGCASRCTKYNAELEKCEARVVSMSNTEEDCVQELEDLLHCLDHCHSQ

SEQ ID NO: 46 - protein, 49 aa, Artificial Sequence
  Description of Artificial Sequence: Synthetic polypeptide
REGCASRCTKYNAELEKCEARVVSMSNTEEDCEQELFDLLHCLDHCHSQ

SEQ ID NO: 47 - protein, 49 aa, Artificial Sequence
  Description of Artificial Sequence: Synthetic polypeptide
REGCASRCTKYNAELEKCEARVVSMSNTEEDCEQELEDLLHCVDHCHSQ

SEQ ID NO: 48 - protein, 49 aa, Artificial Sequence
  Description of Artificial Sequence: Synthetic polypeptide
REGCASRCTKYNAELEKCEARVVSMSNTEEDCEQELEDLLHCLDHCVSQ

SEQ ID NO: 49 - protein, 49 aa, Artificial Sequence
  Description of Artificial Sequence: Synthetic polypeptide
REGCASRCTKYNAELEKCEARVMSMSNTEETCVQELEDLLHCLDHCHSQ

SEQ ID NO: 50 - protein, 49 aa, Artificial Sequence
  Description of Artificial Sequence: Synthetic polypeptide
REGCASRCTKYNAELEKCEARVMSMSNTEETCEQELFDLLHCLDHCHSQ

SEQ ID NO: 51 - protein, 49 aa, Artificial Sequence
  Description of Artificial Sequence: Synthetic polypeptide
REGCASRCTKYNAELEKCEARVMSMSNTEETCEQELEDLLHCVDHCHSQ

SEQ ID NO: 52 - protein, 49 aa, Artificial Sequence
  Description of Artificial Sequence: Synthetic polypeptide
REGCASRCTKYNAELEKCEARVMSMSNTEETCEQELEDLLHCLDHCVSQ

SEQ ID NO: 53 - protein, 49 aa, Artificial Sequence
  Description of Artificial Sequence: Synthetic polypeptide
REGCASRCTKYNAELEKCEARVMSMSNTEEDCVQELFDLLHCLDHCHSQ

SEQ ID NO: 54 - protein, 49 aa, Artificial Sequence
  Description of Artificial Sequence: Synthetic polypeptide
REGCASRCTKYNAELEKCEARVMSMSNTEEDCVQELEDLLHCVDHCHSQ

SEQ ID NO: 55 - protein, 49 aa, Artificial Sequence
  Description of Artificial Sequence: Synthetic polypeptide
REGCASRCTKYNAELEKCEARVMSMSNTEEDCVQELEDLLHCLDHCVSQ

SEQ ID NO: 56 - protein, 49 aa, Artificial Sequence
  Description of Artificial Sequence: Synthetic polypeptide
REGCASRCTKYNAELEKCEARVMSMSNTEEDCEQELFDLLHCVDHCHSQ

SEQ ID NO: 57 - protein, 49 aa, Artificial Sequence
  Description of Artificial Sequence: Synthetic polypeptide
REGCASRCTKYNAELEKCEARVMSMSNTEEDCEQELFDLLHCLDHCVSQ

SEQ ID NO: 58 - protein, 49 aa, Artificial Sequence
  Description of Artificial Sequence: Synthetic polypeptide
REGCASRCTKYNAELEKCEARVMSMSNTEEDCEQELEDLLHCVDHCVSQ

SEQ ID NO: 59 - protein, 49 aa, Artificial Sequence
  Description of Artificial Sequence: Synthetic polypeptide
REGCASRCMKYNAELEKCEARVMSMSNTEEDCEQELEDLLHCLDHCHSQ

SEQ ID NO: 60 - protein, 49 aa, Artificial Sequence
  Description of Artificial Sequence: Synthetic polypeptide
REGCASRCTKYNDELEKCEARVMSMSNTEEDCEQELEDLLHCLDHCHSQ

SEQ ID NO: 61 - protein, 49 aa, Artificial Sequence
  Description of Artificial Sequence: Synthetic polypeptide
REGCASRCTKYNAELEKCEARMMSMSNTEEDCEQELEDLLHCLDHCHSQ

SEQ ID NO: 62 - protein, 49 aa, Artificial Sequence
  Description of Artificial Sequence: Synthetic polypeptide
REGCASRCTKYNAELEKCEARVMSMSNTEEDCEQELEDLLYCLDHCHSQ

SEQ ID NO: 63 - protein, 49 aa, Artificial Sequence
  Description of Artificial Sequence: Synthetic polypeptide
REGCASRCMKYNDELEKCEARMMSMSNTEEDCEQELEDLLHCLDHCHSQ

SEQ ID NO: 64 - protein, 49 aa, Artificial Sequence
  Description of Artificial Sequence: Synthetic polypeptide
REGCASRCMKYNDELEKCEARVMSMSNTEEDCEQELEDLLYCLDHCHSQ

SEQ ID NO: 65 - protein, 49 aa, Artificial Sequence
  Description of Artificial Sequence: Synthetic polypeptide
REGCASRCMKYNAELEKCEARMMSMSNTEEDCEQELEDLLYCLDHCHSQ

SEQ ID NO: 66 - protein, 49 aa, Artificial Sequence
  Description of Artificial Sequence: Synthetic polypeptide
REGCASRCTKYNDELEKCEARMMSMSNTEEDCEQELEDLLYCLDHCHSQ

SEQ ID NO: 67 - protein, 49 aa, Artificial Sequence
  Description of Artificial Sequence: Synthetic polypeptide
REGCASRCMKYNDELEKCEARMMSMSNTEEDCEQELEDLLYCLDHCHSQ

SEQ ID NO: 68 - protein, 65 aa, Artificial Sequence
  Description of Artificial Sequence: Synthetic polypeptide
REGCASRCTKYNAELEKCEARVSSMSNTEETCVQELFDLLHCVDHCVSQGSSELYENKPRRPYIL

SEQ ID NO: 69 - protein, 65 aa, Artificial Sequence
  Description of Artificial Sequence: Synthetic polypeptide
REGCASRCTKYNAELEKCEARVMSMSNTEEDCEQELEDLLHCLDHCHSQGSSELYENKPRRPYIL

SEQ ID NO: 70 - protein, 65 aa, Artificial Sequence
  Description of Artificial Sequence: Synthetic polypeptide
REGCASRCMKYNDELEKCEARMMSMSNTEEDCEQELEDLLYCLDHCHSQGSSELYENKPRRPYIL

SEQ ID NO: 71 - protein, 11 aa, Artificial Sequence
  Description of Artificial Sequence: Synthetic peptide
CYRKKRRQRRR

SEQ ID NO: 72 - protein, 29 aa, Artificial Sequence
  Description of Artificial Sequence: Synthetic peptide
PFVIGAGVLGALGTGIGGIGRKKRRQRRR

SEQ ID NO: 73 - protein, 8 aa, Artificial Sequence
  Description of Artificial Sequence: Synthetic peptide
RRRRRRRR

SEQ ID NO: 74 - protein, 16 aa, Artificial Sequence
  Description of Artificial Sequence: Synthetic peptide
RQIKIWFQNRRMKWKK

SEQ ID NO: 75 - protein, 17 aa, Artificial Sequence
  Description of Artificial Sequence: Synthetic peptide
FFLIPKGGRKKRRQRRR

SEQ ID NO: 76 - protein, 15 aa, Artificial Sequence
  Description of Artificial Sequence: Synthetic peptide
FFLIPKGRRRRRRRR

SEQ ID NO: 77 - protein, 22 aa, Artificial Sequence
  Description of Artificial Sequence: Synthetic peptide
FFLIPKGRRRRNRTRRNRRRVR

SEQ ID NO: 78 - protein, 23 aa, Artificial Sequence
  Description of Artificial Sequence: Synthetic peptide
FFLIPKGRQIKIWFQNRRMKWKK

SEQ ID NO: 79 - protein, 6 aa, Artificial Sequence
  Description of Artificial Sequence: Synthetic peptide
FFRRRR

SEQ ID NO: 80 - protein, 55 aa, Artificial Sequence
  Description of Artificial Sequence: Synthetic polypeptide
KAVLGATKIDLPVDINDPYDLGLLLRHLRHHSNLLANIGDPAVREQVLSAMQEEE

SEQ ID NO: 81 - protein, 28 aa, Artificial Sequence
  Description of Artificial Sequence: Synthetic peptide
LSTAADMQGVVTDGMASGLDKDYLKPDD

SEQ ID NO: 82 - protein, 15 aa, Artificial Sequence
  Description of Artificial Sequence: Synthetic peptide
RRWRRWNRFNRRRCR

SEQ ID NO: 83 - protein, 17 aa, Artificial Sequence
  Description of Artificial Sequence: Synthetic peptide
RAGLQFPVGRLLRRLLR

SEQ ID NO: 84 - protein, 13 aa, Artificial Sequence
  Description of Artificial Sequence: Synthetic peptide
KRAHHNALERKRR

SEQ ID NO: 85 - protein, 13 aa, Artificial Sequence
  Description of Artificial Sequence: Synthetic peptide
RRMKANARERNRM

SEQ ID NO: 86 - protein, 18 aa, Artificial Sequence
  Description of Artificial Sequence: Synthetic peptide
LLIILRRRIRKQAHAHSK

SEQ ID NO: 87 - protein, 10 aa, Artificial Sequence
  Description of Artificial Sequence: Synthetic peptide
RRLSYSRRRF

SEQ ID NO: 88 - protein, 19 aa, Artificial Sequence
  Description of Artificial Sequence: Synthetic peptide
VKRGLKLRHVRPRVTRMDV

SEQ ID NO: 89 - protein, 17 aa, Artificial Sequence
  Description of Artificial Sequence: Synthetic peptide
CSIPPEVKFNKPFVYLI

SEQ ID NO: 90 - protein, 27 aa, Artificial Sequence
  Description of Artificial Sequence: Synthetic peptide
GWTLNSAGYLLGKINLKALAALAKKIL

SEQ ID NO: 91 - protein, 17 aa, Artificial Sequence
  Description of Artificial Sequence: Synthetic peptide
KGEGAAVLLPVLLAAPG

SEQ ID NO: 92 - protein, 22 aa, Artificial Sequence
  Description of Artificial Sequence: Synthetic peptide
KCFQWQRNMRKVRGPPVSCIKR

SEQ ID NO: 93 - protein, 6 aa, Artificial Sequence
  Description of Artificial Sequence: Synthetic peptide
PFVYLI

SEQ ID NO: 94 - protein, 12 aa, Artificial Sequence
  Description of Artificial Sequence: Synthetic peptide
VLDSLEFIASKL

SEQ ID NO: 95 - protein, 11 aa, Unknown
  Description of Unknown: DRI-TAT31 sequence
  MOD_RES (1)..(11): D-amino acids
RRRQRRKKRGY

SEQ ID NO: 96 - protein, 7 aa, Artificial Sequence
  Description of Artificial Sequence: Synthetic peptide
  MOD_RES (2)..(2): l-2-naphthylalanine
FARRRRQ

SEQ ID NO: 97 - skipped

SEQ ID NO: 98 - protein, 10 aa, Artificial Sequence
  Description of Artificial Sequence: Synthetic peptide
  MISC_FEATURE (1)..(10): This sequence may encompass 2-10 residues
RRRRRRRRRR

SEQ ID NO: 99 - protein, 11 aa, Human immunodeficiency virus
YGRKKRRQRRR

SEQ ID NO: 100 - protein, 10 aa, Human immunodeficiency virus
GRKKRRQRRR

SEQ ID NO: 101 - protein, 12 aa, Human immunodeficiency virus
GRKKRRQRRRPQ

SEQ ID NO: 102 - skipped

SEQ ID NO: 103 - protein, 4 aa, Artificial Sequence
  Description of Artificial Sequence: Synthetic peptide
GGGS

SEQ ID NO: 104 - protein, 20 aa, Artificial Sequence
  Description of Artificial Sequence: Synthetic peptide
  MISC_FEATURE (1)..(10): This region may encompass 1-10 residues
  MISC_FEATURE (11)..(20): This region may encompass 1-10 residues
  See specification as filed for detailed description of substitutions and preferred embodiments
GGGGGGGGGGSSSSSSSSSS

SEQ ID NO: 105 - protein, 20 aa, Artificial Sequence
  Description of Artificial Sequence: Synthetic peptide
  MISC_FEATURE (1)..(20): This sequence may encompass 1-10 "Gly Ser" repeating units
  See specification as filed for detailed description of substitutions and preferred embodiments
GSGSGSGSGSGSGSGSGSGS

SEQ ID NO: 106 - protein, 5 aa, Artificial Sequence
  Description of Artificial Sequence: Synthetic peptide
GGSSG

SEQ ID NO: 107 - protein, 5 aa, Artificial Sequence
  Description of Artificial Sequence: Synthetic peptide
GGGGG

SEQ ID NO: 108 - protein, 8 aa, Artificial Sequence
  Description of Artificial Sequence: Synthetic peptide
GSGSGSGS

SEQ ID NO: 109 - protein, 4 aa, Artificial Sequence
  Description of Artificial Sequence: Synthetic peptide
GSGG

SEQ ID NO: 110 - protein, 5 aa, Artificial Sequence
  Description of Artificial Sequence: Synthetic peptide
GGGGS

SEQ ID NO: 111 - skipped

SEQ ID NO: 112 - protein, 3 aa, Artificial Sequence
  Description of Artificial Sequence: Synthetic peptide
GGS

SEQ ID NO: 113 - protein, 12 aa, Artificial Sequence
  Description of Artificial Sequence: Synthetic peptide
GGGSGGGSGGGS

SEQ ID NO: 114 - protein, 12 aa, Haplopelma sp.
KKYKPYVPVTTN

SEQ ID NO: 115 - protein, 10 aa, Homo sapiens
EPKSSDKTHT

SEQ ID NO: 116 - protein, 33 aa, Maurus palmatus
GDCLPHLKLCKENKDCCSKKCKRRGTNIEKRCR

SEQ ID NO: 117 - protein, 33 aa, Pandinus imperator
GDCLPHLKRCKADNDCCGKKCKRRGTNAEKRCR

SEQ ID NO: 118 - protein, 35 aa, Hadrurus gertschi
SEKDCIKHLQRCRENKDCCSKKCSRRGTNPEKRCR

SEQ ID NO: 119 - protein, 33 aa, Hemiscorpius lepturus
GDCLPHLKLCKADKDCCSKKCKRRGTNPEKRCR

SEQ ID NO: 120 - protein, 33 aa, Unknown
  Description of Unknown: opicalcin-1 sequence
GDCLPHLKRCKENNDCCSKKCKRRGTNPEKRCR

SEQ ID NO: 121 - protein, 33 aa, Unknown
  Description of Unknown: opicalcin-2 sequence
GDCLPHLKRCKENNDCCSKKCKRRGANPEKRCR

SEQ ID NO: 122 - protein, 43 aa, Unknown
  Description of Unknown: midkine sequence
CKYKFENWGACDGGTGTKVRQGTLKKARYNAQCQETIRVTKPC

SEQ ID NO: 123 - protein, 34 aa, Momordica cochinchinensis
SGSDGGVCPKILKKCRRDSDCPGACICRGNGYCG

SEQ ID NO: 124 - protein, 36 aa, Leiurus quinquestriatus
MCMPCFTTDHQMARKCDDCCGGKGRGKCYGPQCLCR

SEQ ID NO: 125 - protein, 11 aa, Artificial Sequence
  Description of Artificial Sequence: Synthetic peptide
GGGSGGSGGGS

SEQ ID NO: 126 - protein, 6 aa, Artificial Sequence
  Description of Artificial Sequence: Synthetic peptide
MLICLF

SEQ ID NO: 127 - DNA, 20 bp, Artificial Sequence
  Description of Artificial Sequence: Synthetic primer
tgtacttccagggaggatcc

SEQ ID NO: 128 - DNA, 17 bp, Artificial Sequence
  Description of Artificial Sequence: Synthetic primer
aatggtgatgagcggcc

SEQ ID NO: 129 - protein, 4 aa, Artificial Sequence
  Description of Artificial Sequence: Synthetic peptide
  MOD_RES (2)..(2): K or R
  MOD_RES (3)..(3): Any amino acid
  MOD_RES (4)..(4): K or R
KXXX

SEQ ID NO: 130 - protein, 7 aa, Artificial Sequence
  Description of Artificial Sequence: Synthetic peptide
PKKKRRV

SEQ ID NO: 131 - protein, 16 aa, Artificial Sequence
  Description of Artificial Sequence: Synthetic peptide
KRPAATKKAGQAKKKK

SEQ ID NO: 132 - protein, 20 aa, Artificial Sequence
  Description of Artificial Sequence: Synthetic peptide
  MISC_FEATURE (1)..(10): This region may encompass 0-10 residues
  MISC_FEATURE (11)..(20): This region may encompass 0-10 residues
KKKKKKKKKKRRRRRRRRRR

SEQ ID NO: 133 - protein, 4 aa, Artificial Sequence
  Description of Artificial Sequence: Synthetic peptide
KKRR

SEQ ID NO: 134 - protein, 5 aa, Artificial Sequence
  Description of Artificial Sequence: Synthetic peptide
KKKRR

SEQ ID NO: 135 - protein, 4 aa, Artificial Sequence
  Description of Artificial Sequence: Synthetic peptide
KKKK

SEQ ID NO: 136 - protein, 51 aa, Artificial Sequence
  Description of Artificial Sequence: Synthetic polypeptide
GSREGCASRCTRYNAELERCEARVSSMSNTEETCVQELFDLLHCVDHCVSQ

SEQ ID NO: 137 - protein, 51 aa, Artificial Sequence
  Description of Artificial Sequence: Synthetic polypeptide
GSREGCASRCTRYNAELERCEARVMSMSNTEEDCEQELEDLLHCLDHCHSQ

SEQ ID NO: 138 - protein, 51 aa, Artificial Sequence
  Description of Artificial Sequence: Synthetic polypeptide
GSREGCASRCTRYNAELERCEARVVSMSNTEEDCEQELEDLLHCLDHCHSQ

SEQ ID NO: 139 - protein, 51 aa, Artificial Sequence
  Description of Artificial Sequence: Synthetic polypeptide
GSREGCASRCTRYNAELERCEARVMSMSNTEETCEQELEDLLHCLDHCHSQ

SEQ ID NO: 140 - protein, 51 aa, Artificial Sequence
  Description of Artificial Sequence: Synthetic polypeptide
GSREGCASRCTRYNAELERCEARVMSMSNTEEDCVQELEDLLHCLDHCHSQ

SEQ ID NO: 141 - protein, 51 aa, Artificial Sequence
  Description of Artificial Sequence: Synthetic polypeptide
GSREGCASRCTRYNAELERCEARVMSMSNTEEDCEQELFDLLHCLDHCHSQ

SEQ ID NO: 142 - protein, 51 aa, Artificial Sequence
  Description of Artificial Sequence: Synthetic polypeptide
GSREGCASRCTRYNAELERCEARVMSMSNTEEDCEQELEDLLHCVDHCHSQ

SEQ ID NO: 143 - protein, 51 aa, Artificial Sequence
  Description of Artificial Sequence: Synthetic polypeptide
GSREGCASRCTRYNAELERCEARVMSMSNTEEDCEQELEDLLHCLDHCVSQ

SEQ ID NO: 144 - protein, 51 aa, Artificial Sequence
  Description of Artificial Sequence: Synthetic polypeptide
GSREGCASRCTRYNAELERCEARVVSMSNTEETCEQELEDLLHCLDHCHSQ

SEQ ID NO: 145 - protein, 51 aa, Artificial Sequence
  Description of Artificial Sequence: Synthetic polypeptide
GSREGCASRCTRYNAELERCEARVVSMSNTEEDCVQELEDLLHCLDHCHSQ

SEQ ID NO: 146 - protein, 51 aa, Artificial Sequence
  Description of Artificial Sequence: Synthetic polypeptide
GSREGCASRCTRYNAELERCEARVVSMSNTEEDCEQELFDLLHCLDHCHSQ

SEQ ID NO: 147 - protein, 51 aa, Artificial Sequence
  Description of Artificial Sequence: Synthetic polypeptide
GSREGCASRCTRYNAELERCEARVVSMSNTEEDCEQELEDLLHCVDHCHSQ

SEQ ID NO: 148 - protein, 51 aa, Artificial Sequence
  Description of Artificial Sequence: Synthetic polypeptide
GSREGCASRCTRYNAELERCEARVVSMSNTEEDCEQELEDLLHCLDHCVSQ

SEQ ID NO: 149 - protein, 51 aa, Artificial Sequence
  Description of Artificial Sequence: Synthetic polypeptide
GSREGCASRCTRYNAELERCEARVMSMSNTEETCVQELEDLLHCLDHCHSQ

SEQ ID NO: 150 - protein, 51 aa, Artificial Sequence
  Description of Artificial Sequence: Synthetic polypeptide
GSREGCASRCTRYNAELERCEARVMSMSNTEETCEQELFDLLHCLDHCHSQ

SEQ ID NO: 151 - protein, 51 aa, Artificial Sequence
  Description of Artificial Sequence: Synthetic polypeptide
GSREGCASRCTRYNAELERCEARVMSMSNTEETCEQELEDLLHCVDHCHSQ

SEQ ID NO: 152 - protein, 51 aa, Artificial Sequence
  Description of Artificial Sequence: Synthetic polypeptide
GSREGCASRCTRYNAELERCEARVMSMSNTEETCEQELEDLLHCLDHCVSQ

SEQ ID NO: 153 - protein, 51 aa, Artificial Sequence
  Description of Artificial Sequence: Synthetic polypeptide
GSREGCASRCTRYNAELERCEARVMSMSNTEEDCVQELFDLLHCLDHCHSQ

SEQ ID NO: 154 - protein, 51 aa, Artificial Sequence
  Description of Artificial Sequence: Synthetic polypeptide
GSREGCASRCTRYNAELERCEARVMSMSNTEEDCVQELEDLLHCVDHCHSQ

SEQ ID NO: 155 - protein, 51 aa, Artificial Sequence
  Description of Artificial Sequence: Synthetic polypeptide
GSREGCASRCTRYNAELERCEARVMSMSNTEEDCVQELEDLLHCLDHCVSQ

SEQ ID NO: 156 - protein, 51 aa, Artificial Sequence
  Description of Artificial Sequence: Synthetic polypeptide
GSREGCASRCTRYNAELERCEARVMSMSNTEEDCEQELFDLLHCVDHCHSQ

SEQ ID NO: 157 - protein, 51 aa, Artificial Sequence
  Description of Artificial Sequence: Synthetic polypeptide
GSREGCASRCTRYNAELERCEARVMSMSNTEEDCEQELFDLLHCLDHCVSQ

SEQ ID NO: 158 - protein, 51 aa, Artificial Sequence
  Description of Artificial Sequence: Synthetic polypeptide
GSREGCASRCTRYNAELERCEARVMSMSNTEEDCEQELEDLLHCVDHCVSQ

SEQ ID NO: 159 - protein, 51 aa, Artificial Sequence
  Description of Artificial Sequence: Synthetic polypeptide
GSREGCASRCMRYNAELERCEARVMSMSNTEEDCEQELEDLLHCLDHCHSQ

SEQ ID NO: 160 - protein, 51 aa, Artificial Sequence
  Description of Artificial Sequence: Synthetic polypeptide
GSREGCASRCTRYNDELERCEARVMSMSNTEEDCEQELEDLLHCLDHCHSQ

SEQ ID NO: 161 - protein, 51 aa, Artificial Sequence
  Description of Artificial Sequence: Synthetic polypeptide
GSREGCASRCTRYNAELERCEARMMSMSNTEEDCEQELEDLLHCLDHCHSQ

SEQ ID NO: 162 - protein, 51 aa, Artificial Sequence
  Description of Artificial Sequence: Synthetic polypeptide
GSREGCASRCTRYNAELERCEARVMSMSNTEEDCEQELEDLLYCLDHCHSQ

SEQ ID NO: 163 - protein, 51 aa, Artificial Sequence
  Description of Artificial Sequence: Synthetic polypeptide
GSREGCASRCMRYNDELERCEARMMSMSNTEEDCEQELEDLLHCLDHCHSQ

SEQ ID NO: 164 - protein, 51 aa, Artificial Sequence
  Description of Artificial Sequence: Synthetic polypeptide
GSREGCASRCMRYNDELERCEARVMSMSNTEEDCEQELEDLLYCLDHCHSQ

SEQ ID NO: 165 - protein, 51 aa, Artificial Sequence
  Description of Artificial Sequence: Synthetic polypeptide
GSREGCASRCMRYNAELERCEARMMSMSNTEEDCEQELEDLLYCLDHCHSQ

SEQ ID NO: 166 - protein, 51 aa, Artificial Sequence
  Description of Artificial Sequence: Synthetic polypeptide
GSREGCASRCTRYNDELERCEARMMSMSNTEEDCEQELEDLLYCLDHCHSQ

SEQ ID NO: 167 - protein, 51 aa, Artificial Sequence
  Description of Artificial Sequence: Synthetic polypeptide
GSREGCASRCMRYNDELERCEARMMSMSNTEEDCEQELEDLLYCLDHCHSQ

SEQ ID NO: 168 - protein, 67 aa, Artificial Sequence
  Description of Artificial Sequence: Synthetic polypeptide
GSREGCASRCTRYNAELERCEARVSSMSNTEETCVQELFDLLHCVDHCVSQGSSELYENRPRRPYIL

SEQ ID NO: 169 - protein, 67 aa, Artificial Sequence
  Description of Artificial Sequence: Synthetic polypeptide
GSREGCASRCTRYNAELERCEARVMSMSNTEEDCEQELEDLLHCLDHCHSQGSSELYENRPRRPYIL

SEQ ID NO: 170 - protein, 67 aa, Artificial Sequence
  Description of Artificial Sequence: Synthetic polypeptide
GSREGCASRCMRYNDELERCEARMMSMSNTEEDCEQELEDLLYCLDHCHSQGSSELYENRPRRPYIL

SEQ ID NO: 171 - protein, 49 aa, Artificial Sequence
  Description of Artificial Sequence: Synthetic polypeptide
REGCASRCTRYNAELERCEARVSSMSNTEETCVQELFDLLHCVDHCVSQ

SEQ ID NO: 172 - protein, 49 aa, Artificial Sequence
  Description of Artificial Sequence: Synthetic polypeptide
REGCASRCTRYNAELERCEARVMSMSNTEEDCEQELEDLLHCLDHCHSQ

SEQ ID NO: 173 - protein, 49 aa, Artificial Sequence
  Description of Artificial Sequence: Synthetic polypeptide
REGCASRCTRYNAELERCEARVVSMSNTEEDCEQELEDLLHCLDHCHSQ

SEQ ID NO: 174 - protein, 49 aa, Artificial Sequence
  Description of Artificial Sequence: Synthetic polypeptide
REGCASRCTRYNAELERCEARVMSMSNTEETCEQELEDLLHCLDHCHSQ

SEQ ID NO: 175 - protein, 49 aa, Artificial Sequence
  Description of Artificial Sequence: Synthetic polypeptide
REGCASRCTRYNAELERCEARVMSMSNTEEDCVQELEDLLHCLDHCHSQ

SEQ ID NO: 176 - protein, 49 aa, Artificial Sequence
  Description of Artificial Sequence: Synthetic polypeptide
REGCASRCTRYNAELERCEARVMSMSNTEEDCEQELFDLLHCLDHCHSQ

SEQ ID NO: 177 - protein, 49 aa, Artificial Sequence
  Description of Artificial Sequence: Synthetic polypeptide
REGCASRCTRYNAELERCEARVMSMSNTEEDCEQELEDLLHCVDHCHSQ

SEQ ID NO: 178 - protein, 49 aa, Artificial Sequence
  Description of Artificial Sequence: Synthetic polypeptide
REGCASRCTRYNAELERCEARVMSMSNTEEDCEQELEDLLHCLDHCVSQ

SEQ ID NO: 179 - protein, 49 aa, Artificial Sequence
  Description of Artificial Sequence: Synthetic polypeptide
REGCASRCTRYNAELERCEARVVSMSNTEETCEQELEDLLHCLDHCHSQ

SEQ ID NO: 180 - protein, 49 aa, Artificial Sequence
  Description of Artificial Sequence: Synthetic polypeptide
REGCASRCTRYNAELERCEARVVSMSNTEEDCVQELEDLLHCLDHCHSQ

SEQ ID NO: 181 - protein, 49 aa, Artificial Sequence
  Description of Artificial Sequence: Synthetic polypeptide
REGCASRCTRYNAELERCEARVVSMSNTEEDCEQELFDLLHCLDHCHSQ

SEQ ID NO: 182 - protein, 49 aa, Artificial Sequence
  Description of Artificial Sequence: Synthetic polypeptide
REGCASRCTRYNAELERCEARVVSMSNTEEDCEQELEDLLHCVDHCHSQ

SEQ ID NO: 183 - protein, 49 aa, Artificial Sequence
  Description of Artificial Sequence: Synthetic polypeptide
REGCASRCTRYNAELERCEARVVSMSNTEEDCEQELEDLLHCLDHCVSQ

SEQ ID NO: 184 - protein, 49 aa, Artificial Sequence
  Description of Artificial Sequence: Synthetic polypeptide
REGCASRCTRYNAELERCEARVMSMSNTEETCVQELEDLLHCLDHCHSQ

SEQ ID NO: 185 - protein, 49 aa, Artificial Sequence
  Description of Artificial Sequence: Synthetic polypeptide
REGCASRCTRYNAELERCEARVMSMSNTEETCEQELFDLLHCLDHCHSQ

SEQ ID NO: 186 - protein, 49 aa, Artificial Sequence
  Description of Artificial Sequence: Synthetic polypeptide
REGCASRCTRYNAELERCEARVMSMSNTEETCEQELEDLLHCVDHCHSQ

SEQ ID NO: 187 - protein, 49 aa, Artificial Sequence
  Description of Artificial Sequence: Synthetic polypeptide
REGCASRCTRYNAELERCEARVMSMSNTEETCEQELEDLLHCLDHCVSQ

SEQ ID NO: 188 - protein, 49 aa, Artificial Sequence
  Description of Artificial Sequence: Synthetic polypeptide
REGCASRCTRYNAELERCEARVMSMSNTEEDCVQELFDLLHCLDHCHSQ

SEQ ID NO: 189 - protein, 49 aa, Artificial Sequence
  Description of Artificial Sequence: Synthetic polypeptide
REGCASRCTRYNAELERCEARVMSMSNTEEDCVQELEDLLHCVDHCHSQ

SEQ ID NO: 190 - protein, 49 aa, Artificial Sequence
  Description of Artificial Sequence: Synthetic polypeptide
REGCASRCTRYNAELERCEARVMSMSNTEEDCVQELEDLLHCLDHCVSQ

SEQ ID NO: 191 - protein, 49 aa, Artificial Sequence
  Description of Artificial Sequence: Synthetic polypeptide
REGCASRCTRYNAELERCEARVMSMSNTEEDCEQELFDLLHCVDHCHSQ

SEQ ID NO: 192 - protein, 49 aa, Artificial Sequence
  Description of Artificial Sequence: Synthetic polypeptide
REGCASRCTRYNAELERCEARVMSMSNTEEDCEQELFDLLHCLDHCVSQ

SEQ ID NO: 193 - protein, 49 aa, Artificial Sequence
  Description of Artificial Sequence: Synthetic polypeptide
REGCASRCTRYNAELERCEARVMSMSNTEEDCEQELEDLLHCVDHCVSQ

SEQ ID NO: 194 - protein, 49 aa, Artificial Sequence
  Description of Artificial Sequence: Synthetic polypeptide
REGCASRCMRYNAELERCEARVMSMSNTEEDCEQELEDLLHCLDHCHSQ

SEQ ID NO: 195 - protein, 49 aa, Artificial Sequence
  Description of Artificial Sequence: Synthetic polypeptide
REGCASRCTRYNDELERCEARVMSMSNTEEDCEQELEDLLHCLDHCHSQ

SEQ ID NO: 196 - protein, 49 aa, Artificial Sequence
  Description of Artificial Sequence: Synthetic polypeptide
REGCASRCTRYNAELERCEARMMSMSNTEEDCEQELEDLLHCLDHCHSQ

SEQ ID NO: 197 - protein, 49 aa, Artificial Sequence
  Description of Artificial Sequence: Synthetic polypeptide
REGCASRCTRYNAELERCEARVMSMSNTEEDCEQELEDLLYCLDHCHSQ

SEQ ID NO: 198 - protein, 49 aa, Artificial Sequence
  Description of Artificial Sequence: Synthetic polypeptide
REGCASRCMRYNDELERCEARMMSMSNTEEDCEQELEDLLHCLDHCHSQ

SEQ ID NO: 199 - protein, 49 aa, Artificial Sequence
  Description of Artificial Sequence: Synthetic polypeptide
REGCASRCMRYNDELERCEARVMSMSNTEEDCEQELEDLLYCLDHCHSQ

SEQ ID NO: 200 - protein, 49 aa, Artificial Sequence
  Description of Artificial Sequence: Synthetic polypeptide
REGCASRCMRYNAELERCEARMMSMSNTEEDCEQELEDLLYCLDHCHSQ

SEQ ID NO: 201 - protein, 49 aa, Artificial Sequence
  Description of Artificial Sequence: Synthetic polypeptide
REGCASRCTRYNDELERCEARMMSMSNTEEDCEQELEDLLYCLDHCHSQ

SEQ ID NO: 202 - protein, 49 aa, Artificial Sequence
  Description of Artificial Sequence: Synthetic polypeptide
REGCASRCMRYNDELERCEARMMSMSNTEEDCEQELEDLLYCLDHCHSQ

SEQ ID NO: 203 - protein, 65 aa, Artificial Sequence
  Description of Artificial Sequence: Synthetic polypeptide
REGCASRCTRYNAELERCEARVSSMSNTEETCVQELFDLLHCVDHCVSQGSSELYENRPRRPYIL

SEQ ID NO: 204 - protein, 65 aa, Artificial Sequence
  Description of Artificial Sequence: Synthetic polypeptide
REGCASRCTRYNAELERCEARVMSMSNTEEDCEQELEDLLHCLDHCHSQGSSELYENRPRRPYIL

SEQ ID NO: 205 - protein, 65 aa, Artificial Sequence
  Description of Artificial Sequence: Synthetic polypeptide
REGCASRCMRYNDELERCEARMMSMSNTEEDCEQELEDLLYCLDHCHSQGSSELYENRPRRPYIL

SEQ ID NO: 206 - protein, 51 aa, Artificial Sequence
  Description of Artificial Sequence: Synthetic polypeptide
  MOD_RES (8)..(8): S, T, D, or N
  MOD_RES (11)..(11): A, M, I, L, or V
  MOD_RES (14)..(14): D, E, H, K, R, N, Q, S, or T
  MOD_RES (17)..(17): A, M, I, L, or V
  MOD_RES (18)..(18): D, E, N, Q, S, or T
  MOD_RES (21)..(21): D, E, N, Q, S, or T
  MOD_RES (38)..(38): A, M, I, L, or V
  MOD_RES (41)..(41): A, M, I, L, or V
  MOD_RES (42)..(42): A, M, I, L, or V
  MOD_RES (45)..(45): A, M, I, L, or V
  MOD_RES (46)..(46): D, E, N, Q, S, or T
  MOD_RES (47)..(47): H, K, R, N, Q, S, or T
  MOD_RES (49)..(49): H, K, R, N, Q, S, or T
  MOD_RES (50)..(50): S, T, D, or N
  MOD_RES (51)..(51): D, E, H, K, R, N, Q, S, or T
GSREGCAXRCXKYXDEXXKCXARMMSMSNTEEDCEQEXEDXXYCXXXCXXX

SEQ ID NO: 207 - protein, 51 aa, Artificial Sequence
  Description of Artificial Sequence: Synthetic polypeptide
  MOD_RES (5)..(5): Any amino acid
  MOD_RES (7)..(7): Any amino acid
  MOD_RES (8)..(8): Any amino acid
  MOD_RES (11)..(11): Any amino acid
  MOD_RES (14)..(14): Any amino acid
  MOD_RES (17)..(17): Any amino acid
  MOD_RES (18)..(18): Any amino acid
  MOD_RES (21)..(21): Any amino acid
GSREXCXXRCXKYXDEXXKCXARMMSMSNTEEDCEQELEDLLYCLDHCHSQ

SEQ ID NO: 208 - protein, 51 aa, Artificial Sequence
  Description of Artificial Sequence: Synthetic polypeptide
  MOD_RES (38)..(38): Any amino acid
  MOD_RES (41)..(41): Any amino acid
  MOD_RES (42)..(42): Any amino acid
  MOD_RES (45)..(45): Any amino acid
  MOD_RES (46)..(46): Any amino acid
  MOD_RES (47)..(47): Any amino acid
  MOD_RES (49)..(49): Any amino acid
  MOD_RES (50)..(50): Any amino acid
  MOD_RES (51)..(51): Any amino acid
GSREGCASRCMKYNDELEKCEARMMSMSNTEEDCEQEXEDXXYCXXXCXXX

SEQ ID NO: 209 - protein, 51 aa, Artificial Sequence
  Description of Artificial Sequence: Synthetic polypeptide
  MOD_RES (5)..(5): Any amino acid
  MOD_RES (7)..(7): Any amino acid
  MOD_RES (8)..(8): Any amino acid
  MOD_RES (11)..(11): Any amino acid
  MOD_RES (14)..(14): Any amino acid
  MOD_RES (17)..(17): Any amino acid
  MOD_RES (18)..(18): Any amino acid
  MOD_RES (21)..(21): Any amino acid
  MOD_RES (38)..(38): Any amino acid
  MOD_RES (41)..(41): Any amino acid
  MOD_RES (42)..(42): Any amino acid
  MOD_RES (45)..(45): Any amino acid
  MOD_RES (46)..(46): Any amino acid
  MOD_RES (47)..(47): Any amino acid
  MOD_RES (49)..(49): Any amino acid
  MOD_RES (50)..(50): Any amino acid
  MOD_RES (51)..(51): Any amino acid
GSREXCXXRCXKYXDEXXKCXARMMSMSNTEEDCEQEXEDXXYCXXXCXXX

SEQ ID NO: 210 - protein, 51 aa, Artificial Sequence
  Description of Artificial Sequence: Synthetic polypeptide
  MOD_RES (1)..(1): Any amino acid
  MOD_RES (2)..(2): Any amino acid
  MOD_RES (3)..(3): Any amino acid
  MOD_RES (4)..(4): Any amino acid
  MOD_RES (6)..(6): Any amino acid
  MOD_RES (9)..(9): Any amino acid
  MOD_RES (10)..(10): Any amino acid
  MOD_RES (12)..(12): Any amino acid
  MOD_RES (13)..(13): Any amino acid
  MOD_RES (15)..(15): Any amino acid
  MOD_RES (16)..(16): Any amino acid
  MOD_RES (19)..(19): Any amino acid
  MOD_RES (20)..(20): Any amino acid
  MOD_RES (22)..(22): Any amino acid
  MOD_RES (23)..(23): Any amino acid
  MOD_RES (24)..(24): Any amino acid
  MOD_RES (25)..(25): Any amino acid
  MOD_RES (26)..(26): Any amino acid
  MOD_RES (27)..(27): Any amino acid
  MOD_RES (28)..(28): Any amino acid
  MOD_RES (29)..(29): Any amino acid
  MOD_RES (30)..(30): Any amino acid
  MOD_RES (31)..(31): Any amino acid
  MOD_RES (32)..(32): Any amino acid
  MOD_RES (33)..(33): Any amino acid
  MOD_RES (34)..(34): Any amino acid
  MOD_RES (35)..(35): Any amino acid
  MOD_RES (36)..(36): Any amino acid
  MOD_RES (37)..(37): Any amino acid
  MOD_RES (38)..(38): Any amino acid
  MOD_RES (39)..(39): Any amino acid
  MOD_RES (40)..(40): Any amino acid
  MOD_RES (41)..(41): Any amino acid
  MOD_RES (42)..(42): Any amino acid
  MOD_RES (43)..(43): Any amino acid
  MOD_RES (44)..(44): Any amino acid
  MOD_RES (45)..(45): Any amino acid
  MOD_RES (46)..(46): Any amino acid
  MOD_RES (47)..(47): Any amino acid
  MOD_RES (48)..(48): Any amino acid
  MOD_RES (49)..(49): Any amino acid
  MOD_RES (50)..(50): Any amino acid
  MOD_RES (51)..(51): Any amino acid
XXXXGXASXXMXXNXXLEXXEXXXXXXXXXXXXXXXXXXXXXXXXXXXXXX

SEQ ID NO: 211 - protein, 51 aa, Artificial Sequence
  Description of Artificial Sequence: Synthetic polypeptide
  MOD_RES (1)..(1): Any amino acid
  MOD_RES (2)..(2): Any amino acid
  MOD_RES (3)..(3): Any amino acid
  MOD_RES (4)..(4): Any amino acid
  MOD_RES (5)..(5): Any amino acid
  MOD_RES (6)..(6): Any amino acid
  MOD_RES (7)..(7): Any amino acid
  MOD_RES (8)..(8): Any amino acid
  MOD_RES (9)..(9): Any amino acid
  MOD_RES (10)..(10): Any amino acid
  MOD_RES (11)..(11): Any amino acid
  MOD_RES (12)..(12): Any amino acid
  MOD_RES (13)..(13): Any amino acid
  MOD_RES (14)..(14): Any amino acid
  MOD_RES (15)..(15): Any amino acid
  MOD_RES (16)..(16): Any amino acid
  MOD_RES (17)..(17): Any amino acid
  MOD_RES (18)..(18): Any amino acid
  MOD_RES (19)..(19): Any amino acid
  MOD_RES (20)..(20): Any amino acid
  MOD_RES (21)..(21): Any amino acid
  MOD_RES (22)..(22): Any amino acid
  MOD_RES (23)..(23): Any amino acid
  MOD_RES (24)..(24): Any amino acid
  MOD_RES (25)..(25): Any amino acid
  MOD_RES (26)..(26): Any amino acid
  MOD_RES (27)..(27): Any amino acid
  MOD_RES (28)..(28): Any amino acid
  MOD_RES (29)..(29): Any amino acid
  MOD_RES (30)..(30): Any amino acid
  MOD_RES (31)..(31): Any amino acid
  MOD_RES (32)..(32): Any amino acid
  MOD_RES (33)..(33): Any amino acid
  MOD_RES (34)..(34): Any amino acid
  MOD_RES (35)..(35): Any amino acid
  MOD_RES (36)..(36): Any amino acid
  MOD_RES (37)..(37): Any amino acid
  MOD_RES (39)..(39): Any amino acid
  MOD_RES (40)..(40): Any amino acid
  MOD_RES (43)..(43): Any amino acid
  MOD_RES (44)..(44): Any amino acid
  MOD_RES (48)..(48): Any amino acid
XXXXXXXXXXXXXXXXXXXXXXXXXXXXXXXXXXXXXLXXLLXXLDHXHSQ

SEQ ID NO: 212 - protein, 51 aa, Artificial Sequence
  Description of Artificial Sequence: Synthetic polypeptide
  MOD_RES (1)..(1): Any amino acid
  MOD_RES (2)..(2): Any amino acid
  MOD_RES (3)..(3): Any amino acid
  MOD_RES (4)..(4): Any amino acid
  MOD_RES (6)..(6): Any amino acid
  MOD_RES (9)..(9): Any amino acid
  MOD_RES (10)..(10): Any amino acid
  MOD_RES (12)..(12): Any amino acid
  MOD_RES (13)..(13): Any amino acid
  MOD_RES (15)..(15): Any amino acid
  MOD_RES (16)..(16): Any amino acid
  MOD_RES (19)..(19): Any amino acid
  MOD_RES (20)..(20): Any amino acid
  MOD_RES (22)..(22): Any amino acid
  MOD_RES (23)..(23): Any amino acid
  MOD_RES (24)..(24): Any amino acid
  MOD_RES (25)..(25): Any amino acid
  MOD_RES (26)..(26): Any amino acid
  MOD_RES (27)..(27): Any amino acid
  MOD_RES (28)..(28): Any amino acid
  MOD_RES (29)..(29): Any amino acid
  MOD_RES (30)..(30): Any amino acid
  MOD_RES (31)..(31): Any amino acid
  MOD_RES (32)..(32): Any amino acid
  MOD_RES (33)..(33): Any amino acid
  MOD_RES (34)..(34): Any amino acid
  MOD_RES (35)..(35): Any amino acid
  MOD_RES (36)..(36): Any amino acid
  MOD_RES (37)..(37): Any amino acid
  MOD_RES (39)..(39): Any amino acid
  MOD_RES (40)..(40): Any amino acid
  MOD_RES (43)..(43): Any amino acid
  MOD_RES (44)..(44): Any amino acid
  MOD_RES (48)..(48): Any amino acid
XXXXGXASXXMXXNXXLEXXEXXXXXXXXXXXXXXXXLXXLLXXLDHXHSQ

SEQ ID NO: 213 - protein, 51 aa, Artificial Sequence
  Description of Artificial Sequence: Synthetic polypeptide
  MOD_RES (1)..(1): Any amino acid
  MOD_RES (2)..(2): Any amino acid
  MOD_RES (3)..(3): Any amino acid
  MOD_RES (4)..(4): Any amino acid
  MOD_RES (6)..(6): Any amino acid
  MOD_RES (9)..(9): Any amino acid
  MOD_RES (10)..(10): Any amino acid
  MOD_RES (11)..(11): Any amino acid
  MOD_RES (12)..(12): Any amino acid
  MOD_RES (13)..(13): Any amino acid
  MOD_RES (15)..(15): Any amino acid
  MOD_RES (16)..(16): Any amino acid
  MOD_RES (19)..(19): Any amino acid
  MOD_RES (20)..(20): Any amino acid
  MOD_RES (22)..(22): Any amino acid
  MOD_RES (23)..(23): Any amino acid
  MOD_RES (24)..(24): Any amino acid
  MOD_RES (25)..(25): Any amino acid
  MOD_RES (26)..(26): Any amino acid
  MOD_RES (27)..(27): Any amino acid
  MOD_RES (28)..(28): Any amino acid
  MOD_RES (29)..(29): Any amino acid
  MOD_RES (30)..(30): Any amino acid
  MOD_RES (31)..(31): Any amino acid
  MOD_RES (32)..(32): Any amino acid
  MOD_RES (33)..(33): Any amino acid
  MOD_RES (34)..(34): Any amino acid
  MOD_RES (35)..(35): Any amino acid
  MOD_RES (36)..(36): Any amino acid
  MOD_RES (37)..(37): Any amino acid
  MOD_RES (39)..(39): Any amino acid
  MOD_RES (40)..(40): Any amino acid
  MOD_RES (41)..(41): Any amino acid
  MOD_RES (43)..(43): Any amino acid
  MOD_RES (44)..(44): Any amino acid
  MOD_RES (48)..(48): Any amino acid
  MOD_RES (49)..(49): Any amino acid
XXXXGXASXXXXXNXXLEXXEXXXXXXXXXXXXXXXXLXXXLXXLDHXXSQ

SEQ ID NO: 214 - protein, 51 aa, Artificial Sequence
  Description of Artificial Sequence: Synthetic polypeptide
  MOD_RES (1)..(1): Any amino acid
  MOD_RES (2)..(2): Any amino acid
  MOD_RES (5)..(5): Any amino acid
  MOD_RES (6)..(6): Any amino acid
  MOD_RES (7)..(7): Any amino acid
  MOD_RES (8)..(8): Any amino acid
  MOD_RES (10)..(10): Any amino acid
  MOD_RES (11)..(11): Any amino acid
  MOD_RES (13)..(13): Any amino acid
  MOD_RES (14)..(14): Any amino acid
  MOD_RES (17)..(17): Any amino acid
  MOD_RES (18)..(18): Any amino acid
  MOD_RES (20)..(20): Any amino acid
  MOD_RES (21)..(21): Any amino acid
  MOD_RES (22)..(22): Any amino acid
  MOD_RES (24)..(24): Any amino acid
  MOD_RES (25)..(25): Any amino acid
  MOD_RES (27)..(27): Any amino acid
  MOD_RES (34)..(34): Any amino acid
  MOD_RES (38)..(38): Any amino acid
  MOD_RES (41)..(41): Any amino acid
  MOD_RES (42)..(42): Any amino acid
  MOD_RES (43)..(43): Any amino acid
  MOD_RES (44)..(44): Any amino acid
  MOD_RES (45)..(45): Any amino acid
  MOD_RES (46)..(46): Any amino acid
  MOD_RES (47)..(47): Any amino acid
  MOD_RES (48)..(48): Any amino acid
  MOD_RES (49)..(49): Any amino acid
  MOD_RES (50)..(50): Any amino acid
  MOD_RES (51)..(51): Any amino acid
XXREXXXXRXXKXXDEXXKXXXRXXSXSNTEEDXEQEXEDXXXXXXXXXXX

SEQ ID NO: 215 - protein, 51 aa, Artificial Sequence
  Description of Artificial Sequence: Synthetic polypeptide
  MOD_RES (3)..(3): D, E, H, K, R, N, Q, S, or T
  MOD_RES (4)..(4): D, E, H, K, R, N, Q, S, or T
  MOD_RES (9)..(9): D, E, H, K, R, N, Q, S, or T
  MOD_RES (12)..(12): D, E, H, K, R, N, Q, S, or T
  MOD_RES (15)..(15): D, E, H, K, R, N, Q, S, or T
  MOD_RES (16)..(16): D, E, H, K, R, N, Q, S, or T
  MOD_RES (19)..(19): D, E, H, K, R, N, Q, S, or T
  MOD_RES (23)..(23): D, E, H, K, R, N, Q, S, or T
  MOD_RES (26)..(26): D, E, H, K, R, N, Q, S, or T
  MOD_RES (28)..(28): D, E, H, K, R, N, Q, S, or T
  MOD_RES (29)..(29): D, E, H, K, R, N, Q, S, or T
  MOD_RES (30)..(30): D, E, H, K, R, N, Q, S, or T
  MOD_RES (31)..(31): D, E, H, K, R, N, Q, S, or T
  MOD_RES (32)..(32): D, E, H, K, R, N, Q, S, or T
  MOD_RES (33)..(33): D, E, H, K, R, N, Q, S, or T
  MOD_RES (35)..(35): D, E, H, K, R, N, Q, S, or T
  MOD_RES (36)..(36): D, E, H, K, R, N, Q, S, or T
  MOD_RES (37)..(37): D, E, H, K, R, N, Q, S, or T
  MOD_RES (39)..(39): D, E, H, K, R, N, Q, S, or T
  MOD_RES (40)..(40): D, E, H, K, R, N, Q, S, or T
GSXXGCASXCMXYNXXLEXCEAXMMXMXXXXXXCXXXLXXLLYCLDHCHSQ

SEQ ID NO: 216 - protein, 51 aa, Artificial Sequence
  Description of Artificial Sequence: Synthetic polypeptide
  MOD_RES (1)..(1): Any amino acid
  MOD_RES (2)..(2): Any amino acid
  MOD_RES (3)..(3): Any amino acid
  MOD_RES (4)..(4): Any amino acid
  MOD_RES (5)..(5): Any amino acid
  MOD_RES (6)..(6): Any amino acid
  MOD_RES (7)..(7): Any amino acid
  MOD_RES (8)..(8): Any amino acid
  MOD_RES (9)..(9): Any amino acid
  MOD_RES (10)..(10): Any amino acid
  MOD_RES (11)..(11): Any amino acid
  MOD_RES (12)..(12): Any amino acid
  MOD_RES (13)..(13): Any amino acid
  MOD_RES (14)..(14): Any amino acid
  MOD_RES (16)..(16): Any amino acid
  MOD_RES (17)..(17): Any amino acid
  MOD_RES (18)..(18): Any amino acid
  MOD_RES (19)..(19): Any amino acid
  MOD_RES (20)..(20): Any amino acid
  MOD_RES (21)..(21): Any amino acid
  MOD_RES (22)..(22): Any amino acid
  MOD_RES (23)..(23): Any amino acid
  MOD_RES (24)..(24): Any amino acid
  MOD_RES (25)..(25): Any amino acid
  MOD_RES (26)..(26): Any amino acid
  MOD_RES (27)..(27): Any amino acid
  MOD_RES (28)..(28): Any amino acid
  MOD_RES (29)..(29): Any amino acid
  MOD_RES (30)..(30): Any amino acid
  MOD_RES (31)..(31): Any amino acid
  MOD_RES (32)..(32): Any amino acid
  MOD_RES (33)..(33): Any amino acid
  MOD_RES (34)..(34): Any amino acid
  MOD_RES (36)..(36): Any amino acid
  MOD_RES (37)..(37): Any amino acid
  MOD_RES (38)..(38): Any amino acid
  MOD_RES (40)..(40): Any amino acid
  MOD_RES (41)..(41): Any amino acid
  MOD_RES (42)..(42): Any amino acid
  MOD_RES (43)..(43): Any amino acid
  MOD_RES (44)..(44): Any amino acid
  MOD_RES (45)..(45): Any amino acid
  MOD_RES (46)..(46): Any amino acid
  MOD_RES (47)..(47): Any amino acid
  MOD_RES (48)..(48): Any amino acid
  MOD_RES (50)..(50): Any amino acid
  MOD_RES (51)..(51): Any amino acid
XXXXXXXXXXXXXXDXXXXXXXXXXXXXXXXXXXEXXXEXXXXXXXXXHXX

SEQ ID NO: 217 - protein, 51 aa, Artificial Sequence
  Description of Artificial Sequence: Synthetic polypeptide
  MOD_RES (15)..(15): D, E, H, K, R, N, Q, S, or T
  MOD_RES (35)..(35): D, E, H, K, R, N, Q, S, or T
  MOD_RES (39)..(39): D, E, H, K, R, N, Q, S, or T
  MOD_RES (49)..(49): D, E, H, K, R, N, Q, S, or T
GSREGCASRCMKYNXELEKCEARMMSMSNTEEDCXQELXDLLYCLDHCXSQ

SEQ ID NO: 218 - protein, 51 aa, Artificial Sequence; identical to SEQ ID NO: 217
  Description of Artificial Sequence: Synthetic polypeptide
  MOD_RES (15)..(15): A, M, I, L, V, F, W, or Y
  MOD_RES (35)..(35): A, M, I, L, V, F, W, or Y
  MOD_RES (39)..(39): A, M, I, L, V, F, W, or Y
  MOD_RES (49)..(49): A, M, I, L, V, F, W, or Y

SEQ ID NO: 219 - protein, 51 aa, Artificial Sequence
  Description of Artificial Sequence: Synthetic polypeptide
  MOD_RES (1)..(1): Any amino acid
  MOD_RES (2)..(2): Any amino acid
  MOD_RES (3)..(3): Any amino acid
  MOD_RES (4)..(4): Any amino acid
  MOD_RES (5)..(5): Any amino acid
  MOD_RES (6)..(6): Any amino acid
  MOD_RES (7)..(7): Any amino acid
  MOD_RES (8)..(8): Any amino acid
  MOD_RES (9)..(9): Any amino acid
  MOD_RES (10)..(10): Any amino acid
  MOD_RES (12)..(12): Any amino acid
  MOD_RES (13)..(13): Any amino acid
  MOD_RES (14)..(14): Any amino acid
  MOD_RES (15)..(15): Any amino acid
  MOD_RES (16)..(16): Any amino acid
  MOD_RES (17)..(17): Any amino acid
  MOD_RES (18)..(18): Any amino acid
  MOD_RES (19)..(19): Any amino acid
  MOD_RES (20)..(20): Any amino acid
  MOD_RES (21)..(21): Any amino acid
  MOD_RES (22)..(22): Any amino acid
  MOD_RES (23)..(23): Any amino acid
  MOD_RES (24)..(24): Any amino acid
  MOD_RES (26)..(26): Any amino acid
  MOD_RES (28)..(28): Any amino acid
  MOD_RES (29)..(29): Any amino acid
  MOD_RES (30)..(30): Any amino acid
  MOD_RES (31)..(31): Any amino acid
  MOD_RES (32)..(32): Any amino acid
  MOD_RES (33)..(33): Any amino acid
  MOD_RES (34)..(34): Any amino acid
  MOD_RES (35)..(35): Any amino acid
  MOD_RES (36)..(36): Any amino acid
  MOD_RES (37)..(37): Any amino acid
  MOD_RES (38)..(38): Any amino acid
  MOD_RES (39)..(39): Any amino acid
  MOD_RES (40)..(40): Any amino acid
  MOD_RES (41)..(41): Any amino acid
  MOD_RES (42)..(42): Any amino acid
  MOD_RES (43)..(43): Any amino acid
  MOD_RES (44)..(44): Any amino acid
  MOD_RES (45)..(45): Any amino acid
  MOD_RES (46)..(46): Any amino acid
  MOD_RES (47)..(47): Any amino acid
  MOD_RES (48)..(48): Any amino acid
  MOD_RES (49)..(49): Any amino acid
  MOD_RES (50)..(50): Any amino acid
  MOD_RES (51)..(51): Any amino acid
XXXXXXXXXXMXXXXXXXXXXXXXMXMXXXXXXXXXXXXXXXXXXXXXXXX

SEQ ID NO: 220 - protein, 51 aa, Artificial Sequence
  Description of Artificial Sequence: Synthetic polypeptide
  MOD_RES (11)..(11): A, M, I, L, V, F, W, or Y
  MOD_RES (25)..(25): A, M, I, L, V, F, W, or Y
  MOD_RES (27)..(27): A, M, I, L, V, F, W, or Y
GSREGCASRCXKYNDELEKCEARMXSXSNTEEDCEQELEDLLYCLDHCHSQ

SEQ ID NO: 221 - protein, 51 aa, Artificial Sequence; identical to SEQ ID NO: 220
  Description of Artificial Sequence: Synthetic polypeptide
  MOD_RES (11)..(11): D, E, H, K, R, N, Q, S, or T
  MOD_RES (25)..(25): D, E, H, K, R, N, Q, S, or T
  MOD_RES (27)..(27): D, E, H, K, R, N, Q, S, or T

SEQ ID NO: 222 - protein, 51 aa, Artificial Sequence
  Description of Artificial Sequence: Synthetic polypeptide
  MOD_RES (1)..(1): Any amino acid
  MOD_RES (2)..(2): Any amino acid
  MOD_RES (3)..(3): Any amino acid
  MOD_RES (4)..(4): Any amino acid
  MOD_RES (5)..(5): Any amino acid
  MOD_RES (6)..(6): Any amino acid
  MOD_RES (7)..(7): Any amino acid
  MOD_RES (8)..(8): Any amino acid
  MOD_RES (9)..(9): Any amino acid
  MOD_RES (10)..(10): Any amino acid
  MOD_RES (11)..(11): Any amino acid
  MOD_RES (12)..(12): Any amino acid
  MOD_RES (13)..(13): Any amino acid
  MOD_RES (14)..(14): Any amino acid
  MOD_RES (15)..(15): Any amino acid
  MOD_RES (16)..(16): Any amino acid
  MOD_RES (17)..(17): Any amino acid
  MOD_RES (18)..(18): Any amino acid
  MOD_RES (19)..(19): Any amino acid
  MOD_RES (20)..(20): Any amino acid
  MOD_RES (21)..(21): Any amino acid
  MOD_RES (22)..(22): Any amino acid
  MOD_RES (23)..(23): Any amino acid
  MOD_RES (24)..(24): Any amino acid
  MOD_RES (25)..(25): Any amino acid
  MOD_RES (26)..(26): Any amino acid
  MOD_RES (27)..(27): Any amino acid
  MOD_RES (28)..(28): Any amino acid
  MOD_RES (29)..(29): Any amino acid
  MOD_RES (30)..(30): Any amino acid
  MOD_RES (31)..(31): Any amino acid
  MOD_RES (32)..(32): Any amino acid
  MOD_RES (33)..(33): Any amino acid
  MOD_RES (34)..(34): Any amino acid
  MOD_RES (35)..(35): Any amino acid
  MOD_RES (36)..(36): Any amino acid
  MOD_RES (37)..(37): Any amino acid
  MOD_RES (38)..(38): Any amino acid
  MOD_RES (39)..(39): Any amino acid
  MOD_RES (40)..(40): Any amino acid
  MOD_RES (41)..(41): Any amino acid
  MOD_RES (42)..(42): Any amino acid
  MOD_RES (43)..(43): Any amino acid
  MOD_RES (44)..(44): Any amino acid
  MOD_RES (46)..(46): Any amino acid
  MOD_RES (47)..(47): Any amino acid
  MOD_RES (48)..(48): Any amino acid
  MOD_RES (49)..(49): Any amino acid
  MOD_RES (50)..(50): Any amino acid
  MOD_RES (51)..(51): Any amino acid
XXXXXXXXXXXXXXXXXXXXXXXXXXXXXXXXXXXXXXXXXXXXLXXXXXX

SEQ ID NO: 223 - protein, 51 aa, Artificial Sequence
  Description of Artificial Sequence: Synthetic polypeptide
  MOD_RES (45)..(45): A, M, I, L, or V
GSREGCASRCMKYNDELEKCEARMMSMSNTEEDCEQELEDLLYCXDHCHSQ

SEQ ID NO: 224 - protein, 51 aa, Artificial Sequence
  Description of Artificial Sequence: Synthetic polypeptide
  MOD_RES (12)..(12): K or R
  MOD_RES (19)..(19): K or R
GSREGCASRCMXYNDELEXCEARMMSMSNTEEDCEQELEDLLYCLDHCHSQ

SEQ ID NO: 225 - protein, 316 aa, Artificial Sequence
  Description of Artificial Sequence: Synthetic polypeptide
METDTLLLWVLLLWVPGSTGDIKLQQSGAELARPGASVKMSCKTSGYTFTRYTMHWVKQRPGQGLEWIGYINPSRGYTNYNQKFKDKATLTTDKSSSTAYMQLSSLTSEDSAVYYCARYYDDHYCLDYWGQGTTLTVSSVEGGSGHHHHHHGSGGVDDIQLTQSPAIMSASPGEKVTMTCRASSSVSYMNWYQQKSGTSPKRWIYDTSKVASGVPYRFSGSGSGTSYSLTISSMEAEDAATYYCQQWSSNPLTFGAGTKLELKGGGSREGCASRCTKYNAELEKCEARVSSMSNTEETCVQELFDLLHCVDHCVSQ

SEQ ID NO: 226 - protein, 316 aa, Artificial Sequence
  Description of Artificial Sequence: Synthetic polypeptide
METDTLLLWVLLLWVPGSTGDIKLQQSGAELARPGASVKMSCKTSGYTFTRYTMHWVKQRPGQGLEWIGYINPSRGYTNYNQKFKDKATLTTDKSSSTAYMQLSSLTSEDSAVYYCARYYDDHYCLDYWGQGTTLTVSSVEGGSGHHHHHHGSGGVDDIQLTQSPAIMSASPGEKVTMTCRASSSVSYMNWYQQKSGTSPKRWIYDTSKVASGVPYRFSGSGSGTSYSLTISSMEAEDAATYYCQQWSSNPLTFGAGTKLELKGGGSREGCASRCTKYNAELEKCEARVMSMSNTEEDCEQELEDLLHCLDHCHSQ

SEQ ID NO: 227 - protein, 316 aa, Artificial Sequence
  Description of Artificial Sequence: Synthetic polypeptide
METDTLLLWVLLLWVPGSTGDIKLQQSGAELARPGASVKMSCKTSGYTFTRYTMHWVKQRPGQGLEWIGYINPSRGYTNYNQKFKDKATLTTDKSSSTAYMQLSSLTSEDSAVYYCARYYDDHYCLDYWGQGTTLTVSSVEGGSGHHHHHHGSGGVDDIQLTQSPAIMSASPGEKVTMTCRASSSVSYMNWYQQKSGTSPKRWIYDTSKVASGVPYRFSGSGSGTSYSLTISSMEAEDAATYYCQQWSSNPLTFGAGTKLELKGGGSREGCASRCMKYNDELEKCEARMMSMSNTEEDCEQELEDLLYCLDHCHSQ

SEQ ID NO: 228 - protein, 296 aa, Artificial Sequence
  Description of Artificial Sequence: Synthetic polypeptide
DIKLQQSGAELARPGASVKMSCKTSGYTFTRYTMHWVKQRPGQGLEWIGYINPSRGYTNYNQKFKDKATLTTDKSSSTAYMQLSSLTSEDSAVYYCARYYDDHYCLDYWGQGTTLTVSSVEGGSGHHHHHHGSGGVDDIQLTQSPAIMSASPGEKVTMTCRASSSVSYMNWYQQKSGTSPKRWIYDTSKVASGVPYRFSGSGSGTSYSLTISSMEAEDAATYYCQQWSSNPLTFGAGTKLELKGGGSREGCASRCTKYNAELEKCEARVSSMSNTEETCVQELFDLLHCVDHCVSQ

SEQ ID NO: 229 - protein, 296 aa, Artificial Sequence
  Description of Artificial Sequence: Synthetic polypeptide
DIKLQQSGAELARPGASVKMSCKTSGYTFTRYTMHWVKQRPGQGLEWIGYINPSRGYTNYNQKFKDKATLTTDKSSSTAYMQLSSLTSEDSAVYYCARYYDDHYCLDYWGQGTTLTVSSVEGGSGHHHHHHGSGGVDDIQLTQSPAIMSASPGEKVTMTCRASSSVSYMNWYQQKSGTSPKRWIYDTSKVASGVPYRFSGSGSGTSYSLTISSMEAEDAATYYCQQWSSNPLTFGAGTKLELKGGGSREGCASRCTKYNAELEKCEARVMSMSNTEEDCEQELEDLLHCLDHCHSQ

SEQ ID NO: 230 - protein, 296 aa, Artificial Sequence
  Description of Artificial Sequence: Synthetic polypeptide
DIKLQQSGAELARPGASVKMSCKTSGYTFTRYTMHWVKQRPGQGLEWIGYINPSRGYTNYNQKFKDKATLTTDKSSSTAYMQLSSLTSEDSAVYYCARYYDDHYCLDYWGQGTTLTVSSVEGGSGHHHHHHGSGGVDDIQLTQSPAIMSASPGEKVTMTCRASSSVSYMNWYQQKSGTSPKRWIYDTSKVASGVPYRFSGSGSGTSYSLTISSMEAEDAATYYCQQWSSNPLTFGAGTKLELKGGGSREGCASRCMKYNDELEKCEARMMSMSNTEEDCEQELEDLLYCLDHCHSQ

SEQ ID NO: 231 - protein, 316 aa, Artificial Sequence
  Description of Artificial Sequence: Synthetic polypeptide
METDTLLLWVLLLWVPGSTGDIRLQQSGAELARPGASVRMSCRTSGYTFTRYTMHWVRQRPGQGLEWIGYINPSRGYTNYNQRFRDRATLTTDRSSSTAYMQLSSLTSEDSAVYYCARYYDDHYCLDYWGQGTTLTVSSVEGGSGHHHHHHGSGGVDDIQLTQSPAIMSASPGERVTMTCRASSSVSYMNWYQQRSGTSPRRWIYDTSRVASGVPYRFSGSGSGTSYSLTISSMEAEDAATYYCQQWSSNPLTFGAGTRLELRGGGSREGCASRCTRYNAELERCEARVSSMSNTEETCVQELFDLLHCVDHCVSQ

SEQ ID NO: 232 - protein, 316 aa, Artificial Sequence
  Description of Artificial Sequence: Synthetic polypeptide
METDTLLLWVLLLWVPGSTGDIRLQQSGAELARPGASVRMSCRTSGYTFTRYTMHWVRQRPGQGLEWIGYINPSRGYTNYNQRFRDRATLTTDRSSSTAYMQLSSLTSEDSAVYYCARYYDDHYCLDYWGQGTTLTVSSVEGGSGHHHHHHGSGGVDDIQLTQSPAIMSASPGERVTMTCRASSSVSYMNWYQQRSGTSPRRWIYDTSRVASGVPYRFSGSGSGTSYSLTISSMEAEDAATYYCQQWSSNPLTFGAGTRLELRGGGSREGCASRCTRYNAELERCEARVMSMSNTEEDCEQELEDLLHCLDHCHSQ

SEQ ID NO: 233 - protein, 316 aa, Artificial Sequence
  Description of Artificial Sequence: Synthetic polypeptide
METDTLLLWVLLLWVPGSTGDIRLQQSGAELARPGASVRMSCRTSGYTFTRYTMHWVRQRPGQGLEWIGYINPSRGYTNYNQRFRDRATLTTDRSSSTAYMQLSSLTSEDSAVYYCARYYDDHYCLDYWGQGTTLTVSSVEGGSGHHHHHHGSGGVDDIQLTQSPAIMSASPGERVTMTCRASSSVSYMNWYQQRSGTSPRRWIYDTSRVASGVPYRFSGSGSGTSYSLTISSMEAEDAATYYCQQWSSNPLTFGAGTRLELRGGGSREGCASRCMRYNDELERCEARMMSMSNTEEDCEQELEDLLYCLDHCHSQ

SEQ ID NO: 234 - protein, 296 aa, Artificial Sequence
  Description of Artificial Sequence: Synthetic polypeptide
DIRLQQSGAELARPGASVRMSCRTSGYTFTRYTMHWVRQRPGQGLEWIGYINPSRGYTNYNQRFRDRATLTTDRSSSTAYMQLSSLTSEDSAVYYCARYYDDHYCLDYWGQGTTLTVSSVEGGSGHHHHHHGSGGVDDIQLTQSPAIMSASPGERVTMTCRASSSVSYMNWYQQRSGTSPRRWIYDTSRVASGVPYRFSGSGSGTSYSLTISSMEAEDAATYYCQQWSSNPLTFGAGTRLELRGGGSREGCASRCTRYNAELERCEARVSSMSNTEETCVQELFDLLHCVDHCVSQ

SEQ ID NO: 235 - protein, 296 aa, Artificial Sequence
  Description of Artificial Sequence: Synthetic polypeptide
DIRLQQSGAELARPGASVRMSCRTSGYTFTRYTMHWVRQRPGQGLEWIGYINPSRGYTNYNQRFRDRATLTTDRSSSTAYMQLSSLTSEDSAVYYCARYYDDHYCLDYWGQGTTLTVSSVEGGSGHHHHHHGSGGVDDIQLTQSPAIMSASPGERVTMTCRASSSVSYMNWYQQRSGTSPRRWIYDTSRVASGVPYRFSGSGSGTSYSLTISSMEAEDAATYYCQQWSSNPLTFGAGTRLELRGGGSREGCASRCTRYNAELERCEARVMSMSNTEEDCEQELEDLLHCLDHCHSQ

SEQ ID NO: 236 - protein, 296 aa, Artificial Sequence
  Description of Artificial Sequence: Synthetic polypeptide
DIRLQQSGAELARPGASVRMSCRTSGYTFTRYTMHWVRQRPGQGLEWIGYINPSRGYTNYNQRFRDRATLTTDRSSSTAYMQLSSLTSEDSAVYYCARYYDDHYCLDYWGQGTTLTVSSVEGGSGHHHHHHGSGGVDDIQLTQSPAIMSASPGERVTMTCRASSSVSYMNWYQQRSGTSPRRWIYDTSRVASGVPYRFSGSGSGTSYSLTISSMEAEDAATYYCQQWSSNPLTFGAGTRLELRGGGSREGCASRCMRYNDELERCEARMMSMSNTEEDCEQELEDLLYCLDHCHSQ

SEQ ID NO: 237 - protein, 291 aa, Artificial Sequence
  Description of Artificial Sequence: Synthetic polypeptide
METDTLLLWVLLLWVPGSTGDYKDEHHHHHHGSGTTCPPPVSIEHADIRVKNYSVNSRERYVCNSGFKRKAGTSTLIECVINKNTNVAHWTTPSLKCIRDPSLAGGGGSGGGGSGGGGSGGGGSNWIDVRYDLEKIESLIQSIHIDTTLYTDSDFHPSCKVTAMNCFLLELQVILHEYSNMTLNETVRNVLYLANSTLSSNKNVAESGCKECEELEEKTFTEFLQSFIRIVQMFINTSGGGSREGCASRCTKYNAELEKCEARVSSMSNTEETCVQELFDLLHCVDHCVSQ

SEQ ID NO: 238 - protein, 291 aa, Artificial Sequence
  Description of Artificial Sequence: Synthetic polypeptide
METDTLLLWVLLLWVPGSTGDYKDEHHHHHHGSGTTCPPPVSIEHADIRVKNYSVNSRERYVCNSGFKRKAGTSTLIECVINKNTNVAHWTTPSLKCIRDPSLAGGGGSGGGGSGGGGSGGGGSNWIDVRYDLEKIESLIQSIHIDTTLYTDSDFHPSCKVTAMNCFLLELQVILHEYSNMTLNETVRNVLYLANSTLSSNKNVAESGCKECEELEEKTFTEFLQSFIRIVQMFINTSGGGSREGCASRCTKYNAELEKCEARVMSMSNTEEDCEQELEDLLHCLDHCHSQ

SEQ ID NO: 239 - protein, 291 aa, Artificial Sequence
  Description of Artificial Sequence: Synthetic polypeptide
METDTLLLWVLLLWVPGSTGDYKDEHHHHHHGSGTTCPPPVSIEHADIRVKNYSVNSRERYVCNSGFKRKAGTSTLIECVINKNTNVAHWTTPSLKCIRDPSLAGGGGSGGGGSGGGGSGGGGSNWIDVRYDLEKIESLIQSIHIDTTLYTDSDFHPSCKVTAMNCFLLELQVILHEYSNMTLNETVRNVLYLANSTLSSNKNVAESGCKECEELEEKTFTEFLQSFIRIVQMFINTSGGGSREGCASRCMKYNDELEKCEARMMSMSNTEEDCEQELEDLLYCLDHCHSQ

SEQ ID NO: 240 - protein, 271 aa, Artificial Sequence
  Description of Artificial Sequence: Synthetic polypeptide
DYKDEHHHHHHGSGTTCPPPVSIEHADIRVKNYSVNSRERYVCNSGFKRKAGTSTLIECVINKNTNVAHWTTPSLKCIRDPSLAGGGGSGGGGSGGGGSGGGGSNWIDVRYDLEKIESLIQSIHIDTTLYTDSDFHPSCKVTAMNCFLLELQVILHEYSNMTLNETVRNVLYLANSTLSSNKNVAESGCKECEELEEKTFTEFLQSFIRIVQMFINTSGGGSREGCASRCTKYNAELEKCEARVSSMSNTEETCVQELFDLLHCVDHCVSQ

SEQ ID NO: 241 - protein, 271 aa, Artificial Sequence
  Description of Artificial Sequence: Synthetic polypeptide
DYKDEHHHHHHGSGTTCPPPVSIEHADIRVKNYSVNSRERYVCNSGFKRKAGTSTLIECVINKNTNVAHWTTPSLKCIRDPSLAGGGGSGGGGSGGGGSGGGGSNWIDVRYDLEKIESLIQSIHIDTTLYTDSDFHPSCKVTAMNCFLLELQVILHEYSNMTLNETVRNVLYLANSTLSSNKNVAESGCKECEELEEKTFTEFLQSFIRIVQMFINTSGGGSREGCASRCTKYNAELEKCEARVMSMSNTEEDCEQELEDLLHCLDHCHSQ

SEQ ID NO: 242 - protein, 271 aa, Artificial Sequence
  Description of Artificial Sequence: Synthetic polypeptide
DYKDEHHHHHHGSGTTCPPPVSIEHADIRVKNYSVNSRERYVCNSGFKRKAGTSTLIECVINKNTNVAHWTTPSLKCIRDPSLAGGGGSGGGGSGGGGSGGGGSNWIDVRYDLEKIESLIQSIHIDTTLYTDSDFHPSCKVTAMNCFLLELQVILHEYSNMTLNETVRNVLYLANSTLSSNKNVAESGCKECEELEEKTFTEFLQSFIRIVQMFINTSGGGSREGCASRCMKYNDELEKCEARMMSMSNTEEDCEQELEDLLYCLDHCHSQ

SEQ ID NO: 243 - protein, 291 aa, Artificial Sequence
  Description of Artificial Sequence: Synthetic polypeptide
METDTLLLWVLLLWVPGSTGDYRDEHHHHHHGSGTTCPPPVSIEHADIRVRNYSVNSRERYVCNSGFRRRAGTSTLIECVINRNTNVAHWTTPSLRCIRDPSLAGGGGSGGGGSGGGGSGGGGSNWIDVRYDLERIESLIQSIHIDTTLYTDSDFHPSCRVTAMNCFLLELQVILHEYSNMTLNETVRNVLYLANSTLSSNRNVAESGCRECEELEERTFTEFLQSFIRIVQMFINTSGGGSREGCASRCTRYNAELERCEARVSSMSNTEETCVQELFDLLHCVDHCVSQ

SEQ ID NO: 244 - protein, 291 aa, Artificial Sequence
  Description of Artificial Sequence: Synthetic polypeptide
METDTLLLWVLLLWVPGSTGDYRDEHHHHHHGSGTTCPPPVSIEHADIRVRNYSVNSRERYVCNSGFRRRAGTSTLIECVINRNTNVAHWTTPSLRCIRDPSLAGGGGSGGGGSGGGGSGGGGSNWIDVRYDLERIESLIQSIHIDTTLYTDSDFHPSCRVTAMNCFLLELQVILHEYSNMTLNETVRNVLYLANSTLSSNRNVAESGCRECEELEERTFTEFLQSFIRIVQMFINTSGGGSREGCASRCTRYNAELERCEARVMSMSNTEEDCEQELEDLLHCLDHCHSQ

SEQ ID NO: 245 - protein, 291 aa, Artificial Sequence
  Description of Artificial Sequence: Synthetic polypeptide
METDTLLLWVLLLWVPGSTGDYRDEHHHHHHGSGTTCPPPVSIEHADIRVRNYSVNSRERYVCNSGFRRRAGTSTLIECVINRNTNVAHWTTPSLRCIRDPSLAGGGGSGGGGSGGGGSGGGGSNWIDVRYDLERIESLIQSIHIDTTLYTDSDFHPSCRVTAMNCFLLELQVILHEYSNMTLNETVRNVLYLANSTLSSNRNVAESGCRECEELEERTFTEFLQSFIRIVQMFINTSGGGSREGCASRCMRYNDELERCEARMMSMSNTEEDCEQELEDLLYCLDHCHSQ

SEQ ID NO: 246 - protein, 271 aa, Artificial Sequence
  Description of Artificial Sequence: Synthetic polypeptide
DYRDEHHHHHHGSGTTCPPPVSIEHADIRVRNYSVNSRERYVCNSGFRRRAGTSTLIECVINRNTNVAHWTTPSLRCIRDPSLAGGGGSGGGGSGGGGSGGGGSNWIDVRYDLERIESLIQSIHIDTTLYTDSDFHPSCRVTAMNCFLLELQVILHEYSNMTLNETVRNVLYLANSTLSSNRNVAESGCRECEELEERTFTEFLQSFIRIVQMFINTSGGGSREGCASRCTRYNAELERCEARVSSMSNTEETCVQELFDLLHCVDHCVSQ

SEQ ID NO: 247 - protein, 271 aa, Artificial Sequence
  Description of Artificial Sequence: Synthetic polypeptide
DYRDEHHHHHHGSGTTCPPPVSIEHADIRVRNYSVNSRERYVCNSGFRRRAGTSTLIECVINRNTNVAHWTTPSLRCIRDPSLAGGGGSGGGGSGGGGSGGGGSNWIDVRYDLERIESLIQSIHIDTTLYTDSDFHPSCRVTAMNCFLLELQVILHEYSNMTLNETVRNVLYLANSTLSSNRNVAESGCRECEELEERTFTEFLQSFIRIVQMFINTSGGGSREGCASRCTRYNAELERCEARVMSMSNTEEDCEQELEDLLHCLDHCHSQ

SEQ ID NO: 248 - protein, 271 aa, Artificial Sequence
  Description of Artificial Sequence: Synthetic polypeptide
DYRDEHHHHHHGSGTTCPPPVSIEHADIRVRNYSVNSRERYVCNSGFRRRAGTSTLIECVINRNTNVAHWTTPSLRCIRDPSLAGGGGSGGGGSGGGGSGGGGSNWIDVRYDLERIESLIQSIHIDTTLYTDSDFHPSCRVTAMNCFLLELQVILHEYSNMTLNETVRNVLYLANSTLSSNRNVAESGCRECEELEERTFTEFLQSFIRIVQMFINTSGGGSREGCASRCMRYNDELERCEARMMSMSNTEEDCEQELEDLLYCLDHCHSQ

SEQ ID NO: 249 - protein, 354 aa, Artificial Sequence
  Description of Artificial Sequence: Synthetic polypeptide
METDTLLLWVLLLWVPGSTGDYKDEHHHHHHGSHGTVIESLESLNNYFNSSGIDVEEKSLFLDIWRNWQKDGDMKILQSQIISFYLRLFEVLKDNQAISNNISVIESHLITTFFSNSKAKKDAFMSIAKFEVNNPQVQRQAFNELIRVVHQLLPESSLRKRKRSRGGGSHGTVIESLESLNNYFNSSGIDVEEKSLFLDIWRNWQKDGDMKILQSQIISFYLRLFEVLKDNQAISNNISVIESHLITTFFSNSKAKKDAFMSIAKFEVNNPQVQRQAFNELIRVVHQLLPESSLRKRKRSRGGGSREGCASRCTKYNAELEKCEARVSSMSNTEETCVQELFDLLHCVDHCVSQ

SEQ ID NO: 250 - protein, 354 aa, Artificial Sequence
  Description of Artificial Sequence: Synthetic polypeptide
METDTLLLWVLLLWVPGSTGDYKDEHHHHHHGSHGTVIESLESLNNYFNSSGIDVEEKSLFLDIWRNWQKDGDMKILQSQIISFYLRLFEVLKDNQAISNNISVIESHLITTFFSNSKAKKDAFMSIAKFEVNNPQVQRQAFNELIRVVHQLLPESSLRKRKRSRGGGSHGTVIESLESLNNYFNSSGIDVEEKSLFLDIWRNWQKDGDMKILQSQIISFYLRLFEVLKDNQAISNNISVIESHLITTFFSNSKAKKDAFMSIAKFEVNNPQVQRQAFNELIRVVHQLLPESSLRKRKRSRGGGSREGCASRCTKYNAELEKCEARVMSMSNTEEDCEQELEDLLHCLDHCHSQ

SEQ ID NO: 251 - protein, 354 aa, Artificial Sequence
  Description of Artificial Sequence: Synthetic polypeptide
METDTLLLWVLLLWVPGSTGDYKDEHHHHHHGSHGTVIESLESLNNYFNSSGIDVEEKSLFLDIWRNWQKDGDMKILQSQIISFYLRLFEVLKDNQAISNNISVIESHLITTFFSNSKAKKDAFMSIAKFEVNNPQVQRQAFNELIRVVHQLLPESSLRKRKRSRGGGSHGTVIESLESLNNYFNSSGIDVEEKSLFLDIWRNWQKDGDMKILQSQIISFYLRLFEVLKDNQAISNNISVIESHLITTFFSNSKAKKDAFMSIAKFEVNNPQVQRQAFNELIRVVHQLLPESSLRKRKRSRGGGSREGCASRCMKYNDELEKCEARMMSMSNTEEDCEQELEDLLYCLDHCHSQ

SEQ ID NO: 252 - protein, 334 aa, Artificial Sequence
  Description of Artificial Sequence: Synthetic polypeptide
DYKDEHHHHHHGSHGTVIESLESLNNYFNSSGIDVEEKSLFLDIWRNWQKDGDMKILQSQIISFYLRLFEVLKDNQAISNNISVIESHLITTFFSNSKAKKDAFMSIAKFEVNNPQVQRQAFNELIRVVHQLLPESSLRKRKRSRGGGSHGTVIESLESLNNYFNSSGIDVEEKSLFLDIWRNWQKDGDMKILQSQIISFYLRLFEVLKDNQAISNNISVIESHLITTFFSNSKAKKDAFMSIAKFEVNNPQVQRQAFNELIRVVHQLLPESSLRKRKRSRGGGSREGCASRCTKYNAELEKCEARVSSMSNTEETCVQELFDLLHCVDHCVSQ

SEQ ID NO: 253 - protein, 334 aa, Artificial Sequence
  Description of Artificial Sequence: Synthetic polypeptide
DYKDEHHHHHHGSHGTVIESLESLNNYFNSSGIDVEEKSLFLDIWRNWQKDGDMKILQSQIISFYLRLFEVLKDNQAISNNISVIESHLITTFFSNSKAKKDAFMSIAKFEVNNPQVQRQAFNELIRVVHQLLPESSLRKRKRSRGGGSHGTVIESLESLNNYFNSSGIDVEEKSLFLDIWRNWQKDGDMKILQSQIISFYLRLFEVLKDNQAISNNISVIESHLITTFFSNSKAKKDAFMSIAKFEVNNPQVQRQAFNELIRVVHQLLPESSLRKRKRSRGGGSREGCASRCTKYNAELEKCEARVMSMSNTEEDCEQELEDLLHCLDHCHSQ

SEQ ID NO: 254 - protein, 334 aa, Artificial Sequence
  Description of Artificial Sequence: Synthetic polypeptide
DYKDEHHHHHHGSHGTVIESLESLNNYFNSSGIDVEEKSLFLDIWRNWQKDGDMKILQSQIISFYLRLFEVLKDNQAISNNISVIESHLITTFFSNSKAKKDAFMSIAKFEVNNPQVQRQAFNELIRVVHQLLPESSLRKRKRSRGGGSHGTVIESLESLNNYFNSSGIDVEEKSLFLDIWRNWQKDGDMKILQSQIISFYLRLFEVLKDNQAISNNISVIESHLITTFFSNSKAKKDAFMSIAKFEVNNPQVQRQAFNELIRVVHQLLPESSLRKRKRSRGGGSREGCASRCMKYNDELEKCEARMMSMSNTEEDCEQELEDLLYCLDHCHSQ

SEQ ID NO: 255 - protein, 354 aa, Artificial Sequence
  Description of Artificial Sequence: Synthetic polypeptide
METDTLLLWVLLLWVPGSTGDYRDEHHHHHHGSHGTVIESLESLNNYFNSSGIDVEERSLFLDIWRNWQRDGDMRILQSQIISFYLRLFEVLRDNQAISNNISVIESHLITTFFSNSRARRDAFMSIARFEVNNPQVQRQAFNELIRVVHQLLPESSLRRRRRSRGGGSHGTVIESLESLNNYFNSSGIDVEERSLFLDIWRNWQRDGDMRILQSQIISFYLRLFEVLRDNQAISNNISVIESHLITTFFSNSRARRDAFMSIARFEVNNPQVQRQAFNELIRVVHQLLPESSLRRRRRSRGGGSREGCASRCTRYNAELERCEARVSSMSNTEETCVQELFDLLHCVDHCVSQ

SEQ ID NO: 256 - protein, 354 aa, Artificial Sequence
  Description of Artificial Sequence: Synthetic polypeptide
METDTLLLWVLLLWVPGSTGDYRDEHHHHHHGSHGTVIESLESLNNYFNSSGIDVEERSLFLDIWRNWQRDGDMRILQSQIISFYLRLFEVLRDNQAISNNISVIESHLITTFFSNSRARRDAFMSIARFEVNNPQVQRQAFNELIRVVHQLLPESSLRRRRRSRGGGSHGTVIESLESLNNYFNSSGIDVEERSLFLDIWRNWQRDGDMRILQSQIISFYLRLFEVLRDNQAISNNISVIESHLITTFFSNSRARRDAFMSIARFEVNNPQVQRQAFNELIRVVHQLLPESSLRRRRRSRGGGSREGCASRCTRYNAELERCEARVMSMSNTEEDCEQELEDLLHCLDHCHSQ

SEQ ID NO: 257 - protein, 354 aa, Artificial Sequence
  Description of Artificial Sequence: Synthetic polypeptide
METDTLLLWVLLLWVPGSTGDYRDEHHHHHHGSHGTVIESLESLNNYFNSSGIDVEERSLFLDIWRNWQRDGDMRILQSQIISFYLRLFEVLRDNQAISNNISVIESHLITTFFSNSRARRDAFMSIARFEVNNPQVQRQAFNELIRVVHQLLPESSLRRRRRSRGGGSHGTVIESLESLNNYFNSSGIDVEERSLFLDIWRNWQRDGDMRILQSQIISFYLRLFEVLRDNQAISNNISVIESHLITTFFSNSRARRDAFMSIARFEVNNPQVQRQAFNELIRVVHQLLPESSLRRRRRSRGGGSREGCASRCMRYNDELERCEARMMSMSNTEEDCEQELEDLLYCLDHCHSQ

SEQ ID NO: 258 - protein, 334 aa, Artificial Sequence
  Description of Artificial Sequence: Synthetic polypeptide
DYRDEHHHHHHGSHGTVIESLESLNNYFNSSGIDVEERSLFLDIWRNWQRDGDMRILQSQIISFYLRLFEVLRDNQAISNNISVIESHLITTFFSNSRARRDAFMSIARFEVNNPQVQRQAFNELIRVVHQLLPESSLRRRRRSRGGGSHGTVIESLESLNNYFNSSGIDVEERSLFLDIWRNWQRDGDMRILQSQIISFYLRLFEVLRDNQAISNNISVIESHLITTFFSNSRARRDAFMSIARFEVNNPQVQRQAFNELIRVVHQLLPESSLRRRRRSRGGGSREGCASRCTRYNAELERCEARVSSMSNTEETCVQELFDLLHCVDHCVSQ

SEQ ID NO: 259 - protein, 334 aa, Artificial Sequence
  Description of Artificial Sequence: Synthetic polypeptide
DYRDEHHHHHHGSHGTVIESLESLNNYFNSSGIDVEERSLFLDIWRNWQRDGDMRILQSQIISFYLRLFEVLRDNQAISNNISVIESHLITTFFSNSRARRDAFMSIARFEVNNPQVQRQAFNELIRVVHQLLPESSLRRRRRSRGGGSHGTVIESLESLNNYFNSSGIDVEERSLFLDIWRNWQRDGDMRILQSQIISFYLRLFEVLRDNQAISNNISVIESHLITTFFSNSRARRDAFMSIARFEVNNPQVQRQAFNELIRVVHQLLPESSLRRRRRSRGGGSREGCASRCTRYNAELERCEARVMSMSNTEEDCEQELEDLLHCLDHCHSQ

SEQ ID NO: 260 - protein, 334 aa, Artificial Sequence
  Description of Artificial Sequence: Synthetic polypeptide
DYRDEHHHHHHGSHGTVIESLESLNNYFNSSGIDVEERSLFLDIWRNWQRDGDMRILQSQIISFYLRLFEVLRDNQAISNNISVIESHLITTFFSNSRARRDAFMSIARFEVNNPQVQRQAFNELIRVVHQLLPESSLRRRRRSRGGGSHGTVIESLESLNNYFNSSGIDVEERSLFLDIWRNWQRDGDMRILQSQIISFYLRLFEVLRDNQAISNNISVIESHLITTFFSNSRARRDAFMSIARFEVNNPQVQRQAFNELIRVVHQLLPESSLRRRRRSRGGGSREGCASRCMRYNDELERCEARMMSMSNTEEDCEQELEDLLYCLDHCHSQ

SEQ ID NO: 261 - protein, 295 aa, Artificial Sequence
  Description of Artificial Sequence: Synthetic polypeptide
METDTLLLWVLLLWVPGSTGDYKDEHHHHHHGSGTTCPPPVSIEHADIRVKNYSVNSRERYVCNSGFKRKAGTSTLIECVINKNTNVAHWTTPSLKCIRDPSLAGGGGSGGGGSGGGGSGGGGSNWIDVRYDLEKIESLIQSIHIDTTLYTDSDFHPSCKVTAMNCFLLELQVILHEYSNMTLNETVRNVLYLANSTLSSNKNVAESGCKECEELEEKTFTEFLQSFIRIVQMFINTSGGGSGGGSREGCASRCTKYNAELEKCEARVSSMSNTEETCVQELFDLLHCVDHCVSQ

SEQ ID NO: 262 - protein, 295 aa, Artificial Sequence
  Description of Artificial Sequence: Synthetic polypeptide
METDTLLLWVLLLWVPGSTGDYKDEHHHHHHGSGTTCPPPVSIEHADIRVKNYSVNSRERYVCNSGFKRKAGTSTLIECVINKNTNVAHWTTPSLKCIRDPSLAGGGGSGGGGSGGGGSGGGGSNWIDVRYDLEKIESLIQSIHIDTTLYTDSDFHPSCKVTAMNCFLLELQVILHEYSNMTLNETVRNVLYLANSTLSSNKNVAESGCKECEELEEKTFTEFLQSFIRIVQMFINTSGGGSGGGSREGCASRCTKYNAELEKCEARVMSMSNTEEDCEQELEDLLHCLDHCHSQ

SEQ ID NO: 263 - protein, 295 aa, Artificial Sequence
  Description of Artificial Sequence: Synthetic polypeptide
METDTLLLWVLLLWVPGSTGDYKDEHHHHHHGSGTTCPPPVSIEHADIRVKNYSVNSRERYVCNSGFKRKAGTSTLIECVINKNTNVAHWTTPSLKCIRDPSLAGGGGSGGGGSGGGGSGGGGSNWIDVRYDLEKIESLIQSIHIDTTLYTDSDFHPSCKVTAMNCFLLELQVILHEYSNMTLNETVRNVLYLANSTLSSNKNVAESGCKECEELEEKTFTEFLQSFIRIVQMFINTSGGGSGGGSREGCASRCMKYNDELEKCEARMMSMSNTEEDCEQELEDLLYCLDHCHSQ

SEQ ID NO: 264 - protein, 275 aa, Artificial Sequence
  Description of Artificial Sequence: Synthetic polypeptide
DYKDEHHHHHHGSGTTCPPPVSIEHADIRVKNYSVNSRERYVCNSGFKRKAGTSTLIECVINKNTNVAHWTTPSLKCIRDPSLAGGGGSGGGGSGGGGSGGGGSNWIDVRYDLEKIESLIQSIHIDTTLYTDSDFHPSCKVTAMNCFLLELQVILHEYSNMTLNETVRNVLYLANSTLSSNKNVAESGCKECEELEEKTFTEFLQSFIRIVQMFINTSGGGSGGGSREGCASRCTKYNAELEKCEARVSSMSNTEETCVQELFDLLHCVDHCVSQ

SEQ ID NO: 265 - protein, 275 aa, Artificial Sequence
  Description of Artificial Sequence: Synthetic polypeptide
DYKDEHHHHHHGSGTTCPPPVSIEHADIRVKNYSVNSRERYVCNSGFKRKAGTSTLIECVINKNTNVAHWTTPSLKCIRDPSLAGGGGSGGGGSGGGGSGGGGSNWIDVRYDLEKIESLIQSIHIDTTLYTDSDFHPSCKVTAMNCFLLELQVILHEYSNMTLNETVRNVLYLANSTLSSNKNVAESGCKECEELEEKTFTEFLQSFIRIVQMFINTSGGGSGGGSREGCASRCTKYNAELEKCEARVMSMSNTEEDCEQELEDLLHCLDHCHSQ

SEQ ID NO: 266 - protein, 275 aa, Artificial Sequence
  Description of Artificial Sequence: Synthetic polypeptide
DYKDEHHHHHHGSGTTCPPPVSIEHADIRVKNYSVNSRERYVCNSGFKRKAGTSTLIECVINKNTNVAHWTTPSLKCIRDPSLAGGGGSGGGGSGGGGSGGGGSNWIDVRYDLEKIESLIQSIHIDTTLYTDSDFHPSCKVTAMNCFLLELQVILHEYSNMTLNETVRNVLYLANSTLSSNKNVAESGCKECEELEEKTFTEFLQSFIRIVQMFINTSGGGSGGGSREGCASRCMKYNDELEKCEARMMSMSNTEEDCEQELEDLLYCLDHCHSQ

SEQ ID NO: 267 - protein, 295 aa, Artificial Sequence
  Description of Artificial Sequence: Synthetic polypeptide
METDTLLLWVLLLWVPGSTGDYRDEHHHHHHGSGTTCPPPVSIEHADIRVRNYSVNSRERYVCNSGFRRRAGTSTLIECVINRNTNVAHWTTPSLRCIRDPSLAGGGGSGGGGSGGGGSGGGGSNWIDVRYDLERIESLIQSIHIDTTLYTDSDFHPSCRVTAMNCFLLELQVILHEYSNMTLNETVRNVLYLANSTLSSNRNVAESGCRECEELEERTFTEFLQSFIRIVQMFINTSGGGSGGGSREGCASRCTRYNAELERCEARVSSMSNTEETCVQELFDLLHCVDHCVSQ

SEQ ID NO: 268 - protein, 295 aa, Artificial Sequence
  Description of Artificial Sequence: Synthetic polypeptide
METDTLLLWVLLLWVPGSTGDYRDEHHHHHHGSGTTCPPPVSIEHADIRVRNYSVNSRERYVCNSGFRRRAGTSTLIECVINRNTNVAHWTTPSLRCIRDPSLAGGGGSGGGGSGGGGSGGGGSNWIDVRYDLERIESLIQSIHIDTTLYTDSDFHPSCRVTAMNCFLLELQVILHEYSNMTLNETVRNVLYLANSTLSSNRNVAESGCRECEELEERTFTEFLQSFIRIVQMFINTSGGGSGGGSREGCASRCTRYNAELERCEARVMSMSNTEEDCEQELEDLLHCLDHCHSQ

SEQ ID NO: 269 - protein, 295 aa, Artificial Sequence
  Description of Artificial Sequence: Synthetic polypeptide
METDTLLLWVLLLWVPGSTGDYRDEHHHHHHGSGTTCPPPVSIEHADIRVRNYSVNSRERYVCNSGFRRRAGTSTLIECVINRNTNVAHWTTPSLRCIRDPSLAGGGGSGGGGSGGGGSGGGGSNWIDVRYDLERIESLIQSIHIDTTLYTDSDFHPSCRVTAMNCFLLELQVILHEYSNMTLNETVRNVLYLANSTLSSNRNVAESGCRECEELEERTFTEFLQSFIRIVQMFINTSGGGSGGGSREGCASRCMRYNDELERCEARMMSMSNTEEDCEQELEDLLYCLDHCHSQ

SEQ ID NO: 270 - protein, 275 aa, Artificial Sequence
  Description of Artificial Sequence: Synthetic polypeptide
DYRDEHHHHHHGSGTTCPPPVSIEHADIRVRNYSVNSRERYVCNSGFRRRAGTSTLIECVINRNTNVAHWTTPSLRCIRDPSLAGGGGSGGGGSGGGGSGGGGSNWIDVRYDLERIESLIQSIHIDTTLYTDSDFHPSCRVTAMNCFLLELQVILHEYSNMTLNETVRNVLYLANSTLSSNRNVAESGCRECEELEERTFTEFLQSFIRIVQMFINTSGGGSGGGSREGCASRCTRYNAELERCEARVSSMSNTEETCVQELFDLLHCVDHCVSQ

SEQ ID NO: 271 - protein, 275 aa, Artificial Sequence
  Description of Artificial Sequence: Synthetic polypeptide
DYRDEHHHHHHGSGTTCPPPVSIEHADIRVRNYSVNSRERYVCNSGFRRRAGTSTLIECVINRNTNVAHWTTPSLRCIRDPSLAGGGGSGGGGSGGGGSGGGGSNWIDVRYDLERIESLIQSIHIDTTLYTDSDFHPSCRVTAMNCFLLELQVILHEYSNMTLNETVRNVLYLANSTLSSNRNVAESGCRECEELEERTFTEFLQSFIRIVQMFINTSGGGSGGGSREGCASRCTRYNAELERCEARVMSMSNTEEDCEQELEDLLHCLDHCHSQ

SEQ ID NO: 272 - protein, 275 aa, Artificial Sequence
  Description of Artificial Sequence: Synthetic polypeptide
DYRDEHHHHHHGSGTTCPPPVSIEHADIRVRNYSVNSRERYVCNSGFRRRAGTSTLIECVINRNTNVAHWTTPSLRCIRDPSLAGGGGSGGGGSGGGGSGGGGSNWIDVRYDLERIESLIQSIHIDTTLYTDSDFHPSCRVTAMNCFLLELQVILHEYSNMTLNETVRNVLYLANSTLSSNRNVAESGCRECEELEERTFTEFLQSFIRIVQMFINTSGGGSGGGSREGCASRCMRYNDELERCEARMMSMSNTEEDCEQELEDLLYCLDHCHSQ

SEQ ID NO: 273 - protein, 299 aa, Artificial Sequence
  Description of Artificial Sequence: Synthetic polypeptide
METDTLLLWVLLLWVPGSTGDYKDEHHHHHHGSGTTCPPPVSIEHADIRVKNYSVNSRERYVCNSGFKRKAGTSTLIECVINKNTNVAHWTTPSLKCIRDPSLAGGGGSGGGGSGGGGSGGGGSNWIDVRYDLEKIESLIQSIHIDTTLYTDSDFHPSCKVTAMNCFLLELQVILHEYSNMTLNETVRNVLYLANSTLSSNKNVAESGCKECEELEEKTFTEFLQSFIRIVQMFINTSGGGSGGGSGGGSREGCASRCTKYNAELEKCEARVSSMSNTEETCVQELFDLLHCVDHCVSQ

SEQ ID NO: 274 - protein, 299 aa, Artificial Sequence
  Description of Artificial Sequence: Synthetic polypeptide
METDTLLLWVLLLWVPGSTGDYKDEHHHHHHGSGTTCPPPVSIEHADIRVKNYSVNSRERYVCNSGFKRKAGTSTLIECVINKNTNVAHWTTPSLKCIRDPSLAGGGGSGGGGSGGGGSGGGGSNWIDVRYDLEKIESLIQSIHIDTTLYTDSDFHPSCKVTAMNCFLLELQVILHEYSNMTLNETVRNVLYLANSTLSSNKNVAESGCKECEELEEKTFTEFLQSFIRIVQMFINTSGGGSGGGSGGGSREGCASRCTKYNAELEKCEARVMSMSNTEEDCEQELEDLLHCLDHCHSQ

SEQ ID NO: 275 - protein, 299 aa, Artificial Sequence
  Description of Artificial Sequence: Synthetic polypeptide
METDTLLLWVLLLWVPGSTGDYKDEHHHHHHGSGTTCPPPVSIEHADIRVKNYSVNSRERYVCNSGFKRKAGTSTLIECVINKNTNVAHWTTPSLKCIRDPSLAGGGGSGGGGSGGGGSGGGGSNWIDVRYDLEKIESLIQSIHIDTTLYTDSDFHPSCKVTAMNCFLLELQVILHEYSNMTLNETVRNVLYLANSTLSSNKNVAESGCKECEELEEKTFTEFLQSFIRIVQMFINTSGGGSGGGSGGGSREGCASRCMKYNDELEKCEARMMSMSNTEEDCEQELEDLLYCLDHCHSQ

SEQ ID NO: 276 - protein, 279 aa, Artificial Sequence
  Description of Artificial Sequence: Synthetic polypeptide
DYKDEHHHHHHGSGTTCPPPVSIEHADIRVKNYSVNSRERYVCNSGFKRKAGTSTLIECVINKNTNVAHWTTPSLKCIRDPSLAGGGGSGGGGSGGGGSGGGGSNWIDVRYDLEKIESLIQSIHIDTTLYTDSDFHPSCKVTAMNCFLLELQVILHEYSNMTLNETVRNVLYLANSTLSSNKNVAESGCKECEELEEKTFTEFLQSFIRIVQMFINTSGGGSGGGSGGGSREGCASRCTKYNAELEKCEARVSSMSNTEETCVQELFDLLHCVDHCVSQ

SEQ ID NO: 277 - protein, 279 aa, Artificial Sequence
  Description of Artificial Sequence: Synthetic polypeptide
DYKDEHHHHHHGSGTTCPPPVSIEHADIRVKNYSVNSRERYVCNSGFKRKAGTSTLIECVINKNTNVAHWTTPSLKCIRDPSLAGGGGSGGGGSGGGGSGGGGSNWIDVRYDLEKIESLIQSIHIDTTLYTDSDFHPSCKVTAMNCFLLELQVILHEYSNMTLNETVRNVLYLANSTLSSNKNVAESGCKECEELEEKTFTEFLQSFIRIVQMFINTSGGGSGGGSGGGSREGCASRCTKYNAELEKCEARVMSMSNTEEDCEQELEDLLHCLDHCHSQ

SEQ ID NO: 278 - protein, 279 aa, Artificial Sequence
  Description of Artificial Sequence: Synthetic polypeptide
DYKDEHHHHHHGSGTTCPPPVSIEHADIRVKNYSVNSRERYVCNSGFKRKAGTSTLIECVINKNTNVAHWTTPSLKCIRDPSLAGGGGSGGGGSGGGGSGGGGSNWIDVRYDLEKIESLIQSIHIDTTLYTDSDFHPSCKVTAMNCFLLELQVILHEYSNMTLNETVRNVLYLANSTLSSNKNVAESGCKECEELEEKTFTEFLQSFIRIVQMFINTSGGGSGGGSGGGSREGCASRCMKYNDELEKCEARMMSMSNTEEDCEQELEDLLYCLDHCHSQ

SEQ ID NO: 279 - protein, 299 aa, Artificial Sequence
  Description of Artificial Sequence: Synthetic polypeptide
METDTLLLWVLLLWVPGSTGDYRDEHHHHHHGSGTTCPPPVSIEHADIRVRNYSVNSRERYVCNSGFRRRAGTSTLIECVINRNTNVAHWTTPSLRCIRDPSLAGGGGSGGGGSGGGGSGGGGSNWIDVRYDLERIESLIQSIHIDTTLYTDSDFHPSCRVTAMNCFLLELQVILHEYSNMTLNETVRNVLYLANSTLSSNRNVAESGCRECEELEERTFTEFLQSFIRIVQMFINTSGGGSGGGSGGGSREGCASRCTRYNAELERCEARVSSMSNTEETCVQELFDLLHCVDHCVSQ

SEQ ID NO: 280 - protein, 299 aa, Artificial Sequence
  Description of Artificial Sequence: Synthetic polypeptide
METDTLLLWVLLLWVPGSTGDYRDEHHHHHHGSGTTCPPPVSIEHADIRVRNYSVNSRERYVCNSGFRRRAGTSTLIECVINRNTNVAHWTTPSLRCIRDPSLAGGGGSGGGGSGGGGSGGGGSNWIDVRYDLERIESLIQSIHIDTTLYTDSDFHPSCRVTAMNCFLLELQVILHEYSNMTLNETVRNVLYLANSTLSSNRNVAESGCRECEELEERTFTEFLQSFIRIVQMFINTSGGGSGGGSGGGSREGCASRCTRYNAELERCEARVMSMSNTEEDCEQELEDLLHCLDHCHSQ

SEQ ID NO: 281 - protein, 299 aa, Artificial Sequence
  Description of Artificial Sequence: Synthetic polypeptide
METDTLLLWVLLLWVPGSTGDYRDEHHHHHHGSGTTCPPPVSIEHADIRVRNYSVNSRERYVCNSGFRRRAGTSTLIECVINRNTNVAHWTTPSLRCIRDPSLAGGGGSGGGGSGGGGSGGGGSNWIDVRYDLERIESLIQSIHIDTTLYTDSDFHPSCRVTAMNCFLLELQVILHEYSNMTLNETVRNVLYLANSTLSSNRNVAESGCRECEELEERTFTEFLQSFIRIVQMFINTSGGGSGGGSGGGSREGCASRCMRYNDELERCEARMMSMSNTEEDCEQELEDLLYCLDHCHSQ

SEQ ID NO: 282 - protein, 279 aa, Artificial Sequence
  Description of Artificial Sequence: Synthetic polypeptide
DYRDEHHHHHHGSGTTCPPPVSIEHADIRVRNYSVNSRERYVCNSGFRRRAGTSTLIECVINRNTNVAHWTTPSLRCIRDPSLAGGGGSGGGGSGGGGSGGGGSNWIDVRYDLERIESLIQSIHIDTTLYTDSDFHPSCRVTAMNCFLLELQVILHEYSNMTLNETVRNVLYLANSTLSSNRNVAESGCRECEELEERTFTEFLQSFIRIVQMFINTSGGGSGGGSGGGSREGCASRCTRYNAELERCEARVSSMSNTEETCVQELFDLLHCVDHCVSQ

SEQ ID NO: 283 - protein, 279 aa, Artificial Sequence
  Description of Artificial Sequence: Synthetic polypeptide
DYRDEHHHHHHGSGTTCPPPVSIEHADIRVRNYSVNSRERYVCNSGFRRRAGTSTLIECVINRNTNVAHWTTPSLRCIRDPSLAGGGGSGGGGSGGGGSGGGGSNWIDVRYDLERIESLIQSIHIDTTLYTDSDFHPSCRVTAMNCFLLELQVILHEYSNMTLNETVRNVLYLANSTLSSNRNVAESGCRECEELEERTFTEFLQSFIRIVQMFINTSGGGSGGGSGGGSREGCASRCTRYNAELERCEARVMSMSNTEEDCEQELEDLLHCLDHCHSQ

SEQ ID NO: 284 - protein, 279 aa, Artificial Sequence
  Description of Artificial Sequence: Synthetic polypeptide
DYRDEHHHHHHGSGTTCPPPVSIEHADIRVRNYSVNSRERYVCNSGFRRRAGTSTLIECVINRNTNVAHWTTPSLRCIRDPSLAGGGGSGGGGSGGGGSGGGGSNWIDVRYDLERIESLIQSIHIDTTLYTDSDFHPSCRVTAMNCFLLELQVILHEYSNMTLNETVRNVLYLANSTLSSNRNVAESGCRECEELEERTFTEFLQSFIRIVQMFINTSGGGSGGGSGGGSREGCASRCMRYNDELERCEARMMSMSNTEEDCEQELEDLLYCLDHCHSQ

SEQ ID NO: 285 - protein, 296 aa, Artificial Sequence
  Description of Artificial Sequence: Synthetic polypeptide
METDTLLLWVLLLWVPGSTGDYKDEHHHHHHGSGTTCPPPVSIEHADIRVKNYSVNSRERYVCNSGFKRKAGTSTLIECVINKNTNVAHWTTPSLKCIRDPSLAGGGGSGGGGSGGGGSGGGGSNWIDVRYDLEKIESLIQSIHIDTTLYTDSDFHPSCKVTAMNCFLLELQVILHEYSNMTLNETVRNVLYLANSTLSSNKNVAESGCKECEELEEKTFTEFLQSFIRIVQMFINTSEPRVPITQNREGCASRCTKYNAELEKCEARVSSMSNTEETCVQELFDLLHCVDHCVSQ

SEQ ID NO: 286 - protein, 296 aa, Artificial Sequence
  Description of Artificial Sequence: Synthetic polypeptide
METDTLLLWVLLLWVPGSTGDYKDEHHHHHHGSGTTCPPPVSIEHADIRVKNYSVNSRERYVCNSGFKRKAGTSTLIECVINKNTNVAHWTTPSLKCIRDPSLAGGGGSGGGGSGGGGSGGGGSNWIDVRYDLEKIESLIQSIHIDTTLYTDSDFHPSCKVTAMNCFLLELQVILHEYSNMTLNETVRNVLYLANSTLSSNKNVAESGCKECEELEEKTFTEFLQSFIRIVQMFINTSEPRVPITQNREGCASRCTKYNAELEKCEARVMSMSNTEEDCEQELEDLLHCLDHCHSQ

SEQ ID NO: 287 - protein, 296 aa, Artificial Sequence
  Description of Artificial Sequence: Synthetic polypeptide
METDTLLLWVLLLWVPGSTGDYKDEHHHHHHGSGTTCPPPVSIEHADIRVKNYSVNSRERYVCNSGFKRKAGTSTLIECVINKNTNVAHWTTPSLKCIRDPSLAGGGGSGGGGSGGGGSGGGGSNWIDVRYDLEKIESLIQSIHIDTTLYTDSDFHPSCKVTAMNCFLLELQVILHEYSNMTLNETVRNVLYLANSTLSSNKNVAESGCKECEELEEKTFTEFLQSFIRIVQMFINTSEPRVPITQNREGCASRCMKYNDELEKCEARMMSMSNTEEDCEQELEDLLYCLDHCHSQ

SEQ ID NO: 288 - protein, 276 aa, Artificial Sequence
  Description of Artificial Sequence: Synthetic polypeptide
DYKDEHHHHHHGSGTTCPPPVSIEHADIRVKNYSVNSRERYVCNSGFKRKAGTSTLIECVINKNTNVAHWTTPSLKCIRDPSLAGGGGSGGGGSGGGGSGGGGSNWIDVRYDLEKIESLIQSIHIDTTLYTDSDFHPSCKVTAMNCFLLELQVILHEYSNMTLNETVRNVLYLANSTLSSNKNVAESGCKECEELEEKTFTEFLQSFIRIVQMFINTSEPRVPITQNREGCASRCTKYNAELEKCEARVSSMSNTEETCVQELFDLLHCVDHCVSQ

SEQ ID NO: 289 - protein, 276 aa, Artificial Sequence
  Description of Artificial Sequence: Synthetic polypeptide
DYKDEHHHHHHGSGTTCPPPVSIEHADIRVKNYSVNSRERYVCNSGFKRKAGTSTLIECVINKNTNVAHWTTPSLKCIRDPSLAGGGGSGGGGSGGGGSGGGGSNWIDVRYDLEKIESLIQSIHIDTTLYTDSDFHPSCKVTAMNCFLLELQVILHEYSNMTLNETVRNVLYLANSTLSSNKNVAESGCKECEELEEKTFTEFLQSFIRIVQMFINTSEPRVPITQNREGCASRCTKYNAELEKCEARVMSMSNTEEDCEQELEDLLHCLDHCHSQ

SEQ ID NO: 290 - protein, 276 aa, Artificial Sequence
  Description of Artificial Sequence: Synthetic polypeptide
DYKDEHHHHHHGSGTTCPPPVSIEHADIRVKNYSVNSRERYVCNSGFKRKAGTSTLIECVINKNTNVAHWTTPSLKCIRDPSLAGGGGSGGGGSGGGGSGGGGSNWIDVRYDLEKIESLIQSIHIDTTLYTDSDFHPSCKVTAMNCFLLELQVILHEYSNMTLNETVRNVLYLANSTLSSNKNVAESGCKECEELEEKTFTEFLQSFIRIVQMFINTSEPRVPITQNREGCASRCMKYNDELEKCEARMMSMSNTEEDCEQELEDLLYCLDHCHSQ

SEQ ID NO: 291 - protein, 296 aa, Artificial Sequence
  Description of Artificial Sequence: Synthetic polypeptide
METDTLLLWVLLLWVPGSTGDYRDEHHHHHHGSGTTCPPPVSIEHADIRVRNYSVNSRERYVCNSGFRRRAGTSTLIECVINRNTNVAHWTTPSLRCIRDPSLAGGGGSGGGGSGGGGSGGGGSNWIDVRYDLERIESLIQSIHIDTTLYTDSDFHPSCRVTAMNCFLLELQVILHEYSNMTLNETVRNVLYLANSTLSSNRNVAESGCRECEELEERTFTEFLQSFIRIVQMFINTSEPRVPITQNREGCASRCTRYNAELERCEARVSSMSNTEETCVQELFDLLHCVDHCVSQ

SEQ ID NO: 292 - protein, 296 aa, Artificial Sequence
  Description of Artificial Sequence: Synthetic polypeptide
METDTLLLWVLLLWVPGSTGDYRDEHHHHHHGSGTTCPPPVSIEHADIRVRNYSVNSRERYVCNSGFRRRAGTSTLIECVINRNTNVAHWTTPSLRCIRDPSLAGGGGSGGGGSGGGGSGGGGSNWIDVRYDLERIESLIQSIHIDTTLYTDSDFHPSCRVTAMNCFLLELQVILHEYSNMTLNETVRNVLYLANSTLSSNRNVAESGCRECEELEERTFTEFLQSFIRIVQMFINTSEPRVPITQNREGCASRCTRYNAELERCEARVMSMSNTEEDCEQELEDLLHCLDHCHSQ

SEQ ID NO: 293 - protein, 296 aa, Artificial Sequence
  Description of Artificial Sequence: Synthetic polypeptide
METDTLLLWVLLLWVPGSTGDYRDEHHHHHHGSGTTCPPPVSIEHADIRVRNYSVNSRERYVCNSGFRRRAGTSTLIECVINRNTNVAHWTTPSLRCIRDPSLAGGGGSGGGGSGGGGSGGGGSNWIDVRYDLERIESLIQSIHIDTTLYTDSDFHPSCRVTAMNCFLLELQVILHEYSNMTLNETVRNVLYLANSTLSSNRNVAESGCRECEELEERTFTEFLQSFIRIVQMFINTSEPRVPITQNREGCASRCMRYNDELERCEARMMSMSNTEEDCEQELEDLLYCLDHCHSQ

SEQ ID NO: 294 - protein, 276 aa, Artificial Sequence
  Description of Artificial Sequence: Synthetic polypeptide
DYRDEHHHHHHGSGTTCPPPVSIEHADIRVRNYSVNSRERYVCNSGFRRRAGTSTLIECVINRNTNVAHWTTPSLRCIRDPSLAGGGGSGGGGSGGGGSGGGGSNWIDVRYDLERIESLIQSIHIDTTLYTDSDFHPSCRVTAMNCFLLELQVILHEYSNMTLNETVRNVLYLANSTLSSNRNVAESGCRECEELEERTFTEFLQSFIRIVQMFINTSEPRVPITQNREGCASRCTRYNAELERCEARVSSMSNTEETCVQELFDLLHCVDHCVSQ

SEQ ID NO: 295 - protein, 276 aa, Artificial Sequence
  Description of Artificial Sequence: Synthetic polypeptide
DYRDEHHHHHHGSGTTCPPPVSIEHADIRVRNYSVNSRERYVCNSGFRRRAGTSTLIECVINRNTNVAHWTTPSLRCIRDPSLAGGGGSGGGGSGGGGSGGGGSNWIDVRYDLERIESLIQSIHIDTTLYTDSDFHPSCRVTAMNCFLLELQVILHEYSNMTLNETVRNVLYLANSTLSSNRNVAESGCRECEELEERTFTEFLQSFIRIVQMFINTSEPRVPITQNREGCASRCTRYNAELERCEARVMSMSNTEEDCEQELEDLLHCLDHCHSQ

SEQ ID NO: 296 - protein, 276 aa, Artificial Sequence
  Description of Artificial Sequence: Synthetic polypeptide
DYRDEHHHHHHGSGTTCPPPVSIEHADIRVRNYSVNSRERYVCNSGFRRRAGTSTLIECVINRNTNVAHWTTPSLRCIRDPSLAGGGGSGGGGSGGGGSGGGGSNWIDVRYDLERIESLIQSIHIDTTLYTDSDFHPSCRVTAMNCFLLELQVILHEYSNMTLNETVRNVLYLANSTLSSNRNVAESGCRECEELEERTFTEFLQSFIRIVQMFINTSEPRVPITQNREGCASRCMRYNDELERCEARMMSMSNTEEDCEQELEDLLYCLDHCHSQ

SEQ ID NO: 297 - protein, 298 aa, Artificial Sequence
  Description of Artificial Sequence: Synthetic polypeptide
METDTLLLWVLLLWVPGSTGDYKDEHHHHHHENLYFQGSREGCASRCTKYNAELEKCEARVSSMSNTEETCVQELFDLLHCVDHCVSQGGGGSGTTCPPPVSIEHADIRVKNYSVNSRERYVCNSGFKRKAGTSTLIECVINKNTNVAHWTTPSLKCIRDPSLAGGGGSGGGGSGGGGSGGGGSNWIDVRYDLEKIESLIQSIHIDTTLYTDSDFHPSCKVTAMNCFLLELQVILHEYSNMTLNETVRNVLYLANSTLSSNKNVAESGCKECEELEEKTFTEFLQSFIRIVQMFINTS

SEQ ID NO: 298 - protein, 298 aa, Artificial Sequence
  Description of Artificial Sequence: Synthetic polypeptide
METDTLLLWVLLLWVPGSTGDYKDEHHHHHHENLYFQGSREGCASRCTKYNAELEKCEARVMSMSNTEEDCEQELEDLLHCLDHCHSQGGGGSGTTCPPPVSIEHADIRVKNYSVNSRERYVCNSGFKRKAGTSTLIECVINKNTNVAHWTTPSLKCIRDPSLAGGGGSGGGGSGGGGSGGGGSNWIDVRYDLEKIESLIQSIHIDTTLYTDSDFHPSCKVTAMNCFLLELQVILHEYSNMTLNETVRNVLYLANSTLSSNKNVAESGCKECEELEEKTFTEFLQSFIRIVQMFINTS

SEQ ID NO: 299 - protein, 298 aa, Artificial Sequence
  Description of Artificial Sequence: Synthetic polypeptide
METDTLLLWVLLLWVPGSTGDYKDEHHHHHHENLYFQGSREGCASRCMKYNDELEKCEARMMSMSNTEEDCEQELEDLLYCLDHCHSQGGGGSGTTCPPPVSIEHADIRVKNYSVNSRERYVCNSGFKRKAGTSTLIECVINKNTNVAHWTTPSLKCIRDPSLAGGGGSGGGGSGGGGSGGGGSNWIDVRYDLEKIESLIQSIHIDTTLYTDSDFHPSCKVTAMNCFLLELQVILHEYSNMTLNETVRNVLYLANSTLSSNKNVAESGCKECEELEEKTFTEFLQSFIRIVQMFINTS

SEQ ID NO: 300 - protein, 278 aa, Artificial Sequence
  Description of Artificial Sequence: Synthetic polypeptide
DYKDEHHHHHHENLYFQGSREGCASRCTKYNAELEKCEARVSSMSNTEETCVQELFDLLHCVDHCVSQGGGGSGTTCPPPVSIEHADIRVKNYSVNSRERYVCNSGFKRKAGTSTLIECVINKNTNVAHWTTPSLKCIRDPSLAGGGGSGGGGSGGGGSGGGGSNWIDVRYDLEKIESLIQSIHIDTTLYTDSDFHPSCKVTAMNCFLLELQVILHEYSNMTLNETVRNVLYLANSTLSSNKNVAESGCKECEELEEKTFTEFLQSFIRIVQMFINTS

SEQ ID NO: 301 - protein, 278 aa, Artificial Sequence
  Description of Artificial Sequence: Synthetic polypeptide
DYKDEHHHHHHENLYFQGSREGCASRCTKYNAELEKCEARVMSMSNTEEDCEQELEDLLHCLDHCHSQGGGGSGTTCPPPVSIEHADIRVKNYSVNSRERYVCNSGFKRKAGTSTLIECVINKNTNVAHWTTPSLKCIRDPSLAGGGGSGGGGSGGGGSGGGGSNWIDVRYDLEKIESLIQSIHIDTTLYTDSDFHPSCKVTAMNCFLLELQVILHEYSNMTLNETVRNVLYLANSTLSSNKNVAESGCKECEELEEKTFTEFLQSFIRIVQMFINTS

SEQ ID NO: 302 - protein, 278 aa, Artificial Sequence
  Description of Artificial Sequence: Synthetic polypeptide
DYKDEHHHHHHENLYFQGSREGCASRCMKYNDELEKCEARMMSMSNTEEDCEQELEDLLYCLDHCHSQGGGGSGTTCPPPVSIEHADIRVKNYSVNSRERYVCNSGFKRKAGTSTLIECVINKNTNVAHWTTPSLKCIRDPSLAGGGGSGGGGSGGGGSGGGGSNWIDVRYDLEKIESLIQSIHIDTTLYTDSDFHPSCKVTAMNCFLLELQVILHEYSNMTLNETVRNVLYLANSTLSSNKNVAESGCKECEELEEKTFTEFLQSFIRIVQMFINTS

SEQ ID NO: 303 - protein, 298 aa, Artificial Sequence
  Description of Artificial Sequence: Synthetic polypeptide
METDTLLLWVLLLWVPGSTGDYRDEHHHHHHENLYFQGSREGCASRCTRYNAELERCEARVSSMSNTEETCVQELFDLLHCVDHCVSQGGGGSGTTCPPPVSIEHADIRVRNYSVNSRERYVCNSGFRRRAGTSTLIECVINRNTNVAHWTTPSLRCIRDPSLAGGGGSGGGGSGGGGSGGGGSNWIDVRYDLERIESLIQSIHIDTTLYTDSDFHPSCRVTAMNCFLLELQVILHEYSNMTLNETVRNVLYLANSTLSSNRNVAESGCRECEELEERTFTEFLQSFIRIVQMFINTS

SEQ ID NO: 304 - protein, 298 aa, Artificial Sequence
  Description of Artificial Sequence: Synthetic polypeptide
METDTLLLWVLLLWVPGSTGDYRDEHHHHHHENLYFQGSREGCASRCTRYNAELERCEARVMSMSNTEEDCEQELEDLLHCLDHCHSQGGGGSGTTCPPPVSIEHADIRVRNYSVNSRERYVCNSGFRRRAGTSTLIECVINRNTNVAHWTTPSLRCIRDPSLAGGGGSGGGGSGGGGSGGGGSNWIDVRYDLERIESLIQSIHIDTTLYTDSDFHPSCRVTAMNCFLLELQVILHEYSNMTLNETVRNVLYLANSTLSSNRNVAESGCRECEELEERTFTEFLQSFIRIVQMFINTS

SEQ ID NO: 305 - protein, 298 aa, Artificial Sequence
  Description of Artificial Sequence: Synthetic polypeptide
METDTLLLWVLLLWVPGSTGDYRDEHHHHHHENLYFQGSREGCASRCMRYNDELERCEARMMSMSNTEEDCEQELEDLLYCLDHCHSQGGGGSGTTCPPPVSIEHADIRVRNYSVNSRERYVCNSGFRRRAGTSTLIECVINRNTNVAHWTTPSLRCIRDPSLAGGGGSGGGGSGGGGSGGGGSNWIDVRYDLERIESLIQSIHIDTTLYTDSDFHPSCRVTAMNCFLLELQVILHEYSNMTLNETVRNVLYLANSTLSSNRNVAESGCRECEELEERTFTEFLQSFIRIVQMFINTS

SEQ ID NO: 306 - protein, 278 aa, Artificial Sequence
  Description of Artificial Sequence: Synthetic polypeptide
DYRDEHHHHHHENLYFQGSREGCASRCTRYNAELERCEARVSSMSNTEETCVQELFDLLHCVDHCVSQGGGGSGTTCPPPVSIEHADIRVRNYSVNSRERYVCNSGFRRRAGTSTLIECVINRNTNVAHWTTPSLRCIRDPSLAGGGGSGGGGSGGGGSGGGGSNWIDVRYDLERIESLIQSIHIDTTLYTDSDFHPSCRVTAMNCFLLELQVILHEYSNMTLNETVRNVLYLANSTLSSNRNVAESGCRECEELEERTFTEFLQSFIRIVQMFINTS

SEQ ID NO: 307 - protein, 278 aa, Artificial Sequence
  Description of Artificial Sequence: Synthetic polypeptide
DYRDEHHHHHHENLYFQGSREGCASRCTRYNAELERCEARVMSMSNTEEDCEQELEDLLHCLDHCHSQGGGGSGTTCPPPVSIEHADIRVRNYSVNSRERYVCNSGFRRRAGTSTLIECVINRNTNVAHWTTPSLRCIRDPSLAGGGGSGGGGSGGGGSGGGGSNWIDVRYDLERIESLIQSIHIDTTLYTDSDFHPSCRVTAMNCFLLELQVILHEYSNMTLNETVRNVLYLANSTLSSNRNVAESGCRECEELEERTFTEFLQSFIRIVQMFINTS

SEQ ID NO: 308 - protein, 278 aa, Artificial Sequence
  Description of Artificial Sequence: Synthetic polypeptide
DYRDEHHHHHHENLYFQGSREGCASRCMRYNDELERCEARMMSMSNTEEDCEQELEDLLYCLDHCHSQGGGGSGTTCPPPVSIEHADIRVRNYSVNSRERYVCNSGFRRRAGTSTLIECVINRNTNVAHWTTPSLRCIRDPSLAGGGGSGGGGSGGGGSGGGGSNWIDVRYDLERIESLIQSIHIDTTLYTDSDFHPSCRVTAMNCFLLELQVILHEYSNMTLNETVRNVLYLANSTLSSNRNVAESGCRECEELEERTFTEFLQSFIRIVQMFINTS

SEQ ID NO: 309 - protein, 301 aa, Artificial Sequence
  Description of Artificial Sequence: Synthetic polypeptide
METDTLLLWVLLLWVPGSTGDYKDEHHHHHHGSGTTCPPPVSIEHADIRVKNYSVNSRERYVCNSGFKRKAGTSTLIECVINKNTNVAHWTTPSLKCIRDPSLAGGGGSGGGGSGGGGSGGGGSNWIDVRYDLEKIESLIQSIHIDTTLYTDSDFHPSCKVTAMNCFLLELQVILHEYSNMTLNETVRNVLYLANSTLSSNKNVAESGCKECEELEEKTFTEFLQSFIRIVQMFINTSEPRIPKPSTPPGSSREGCASRCTKYNAELEKCEARVSSMSNTEETCVQELFDLLHCVDHCVSQ

SEQ ID NO: 310 - protein, 301 aa, Artificial Sequence
  Description of Artificial Sequence: Synthetic polypeptide
METDTLLLWVLLLWVPGSTGDYKDEHHHHHHGSGTTCPPPVSIEHADIRVKNYSVNSRERYVCNSGFKRKAGTSTLIECVINKNTNVAHWTTPSLKCIRDPSLAGGGGSGGGGSGGGGSGGGGSNWIDVRYDLEKIESLIQSIHIDTTLYTDSDFHPSCKVTAMNCFLLELQVILHEYSNMTLNETVRNVLYLANSTLSSNKNVAESGCKECEELEEKTFTEFLQSFIRIVQMFINTSEPRIPKPSTPPGSSREGCASRCTKYNAELEKCEARVMSMSNTEEDCEQELEDLLHCLDHCHSQ

SEQ ID NO: 311 - protein, 301 aa, Artificial Sequence
  Description of Artificial Sequence: Synthetic polypeptide
METDTLLLWVLLLWVPGSTGDYKDEHHHHHHGSGTTCPPPVSIEHADIRVKNYSVNSRERYVCNSGFKRKAGTSTLIECVINKNTNVAHWTTPSLKCIRDPSLAGGGGSGGGGSGGGGSGGGGSNWIDVRYDLEKIESLIQSIHIDTTLYTDSDFHPSCKVTAMNCFLLELQVILHEYSNMTLNETVRNVLYLANSTLSSNKNVAESGCKECEELEEKTFTEFLQSFIRIVQMFINTSEPRIPKPSTPPGSSREGCASRCMKYNDELEKCEARMMSMSNTEEDCEQELEDLLYCLDHCHSQ

SEQ ID NO: 312 - protein, 281 aa, Artificial Sequence
  Description of Artificial Sequence: Synthetic polypeptide
DYKDEHHHHHHGSGTTCPPPVSIEHADIRVKNYSVNSRERYVCNSGFKRKAGTSTLIECVINKNTNVAHWTTPSLKCIRDPSLAGGGGSGGGGSGGGGSGGGGSNWIDVRYDLEKIESLIQSIHIDTTLYTDSDFHPSCKVTAMNCFLLELQVILHEYSNMTLNETVRNVLYLANSTLSSNKNVAESGCKECEELEEKTFTEFLQSFIRIVQMFINTSEPRIPKPSTPPGSSREGCASRCTKYNAELEKCEARVSSMSNTEETCVQELFDLLHCVDHCVSQ

SEQ ID NO: 313 - protein, 281 aa, Artificial Sequence
  Description of Artificial Sequence: Synthetic polypeptide
DYKDEHHHHHHGSGTTCPPPVSIEHADIRVKNYSVNSRERYVCNSGFKRKAGTSTLIECVINKNTNVAHWTTPSLKCIRDPSLAGGGGSGGGGSGGGGSGGGGSNWIDVRYDLEKIESLIQSIHIDTTLYTDSDFHPSCKVTAMNCFLLELQVILHEYSNMTLNETVRNVLYLANSTLSSNKNVAESGCKECEELEEKTFTEFLQSFIRIVQMFINTSEPRIPKPSTPPGSSREGCASRCTKYNAELEKCEARVMSMSNTEEDCEQELEDLLHCLDHCHSQ

SEQ ID NO: 314 - protein, 281 aa, Artificial Sequence
  Description of Artificial Sequence: Synthetic polypeptide
DYKDEHHHHHHGSGTTCPPPVSIEHADIRVKNYSVNSRERYVCNSGFKRKAGTSTLIECVINKNTNVAHWTTPSLKCIRDPSLAGGGGSGGGGSGGGGSGGGGSNWIDVRYDLEKIESLIQSIHIDTTLYTDSDFHPSCKVTAMNCFLLELQVILHEYSNMTLNETVRNVLYLANSTLSSNKNVAESGCKECEELEEKTFTEFLQSFIRIVQMFINTSEPRIPKPSTPPGSSREGCASRCMKYNDELEKCEARMMSMSNTEEDCEQELEDLLYCLDHCHSQ

SEQ ID NO: 315 - protein, 301 aa, Artificial Sequence
  Description of Artificial Sequence: Synthetic polypeptide
METDTLLLWVLLLWVPGSTGDYRDEHHHHHHGSGTTCPPPVSIEHADIRVRNYSVNSRERYVCNSGFRRRAGTSTLIECVINRNTNVAHWTTPSLRCIRDPSLAGGGGSGGGGSGGGGSGGGGSNWIDVRYDLERIESLIQSIHIDTTLYTDSDFHPSCRVTAMNCFLLELQVILHEYSNMTLNETVRNVLYLANSTLSSNRNVAESGCRECEELEERTFTEFLQSFIRIVQMFINTSEPRIPRPSTPPGSSREGCASRCTRYNAELERCEARVSSMSNTEETCVQELFDLLHCVDHCVSQ

SEQ ID NO: 316 - protein, 301 aa, Artificial Sequence
  Description of Artificial Sequence: Synthetic polypeptide
METDTLLLWVLLLWVPGSTGDYRDEHHHHHHGSGTTCPPPVSIEHADIRVRNYSVNSRERYVCNSGFRRRAGTSTLIECVINRNTNVAHWTTPSLRCIRDPSLAGGGGSGGGGSGGGGSGGGGSNWIDVRYDLERIESLIQSIHIDTTLYTDSDFHPSCRVTAMNCFLLELQVILHEYSNMTLNETVRNVLYLANSTLSSNRNVAESGCRECEELEERTFTEFLQSFIRIVQMFINTSEPRIPRPSTPPGSSREGCASRCTRYNAELERCEARVMSMSNTEEDCEQELEDLLHCLDHCHSQ

SEQ ID NO: 317 - protein, 301 aa, Artificial Sequence
  Description of Artificial Sequence: Synthetic polypeptide
METDTLLLWVLLLWVPGSTGDYRDEHHHHHHGSGTTCPPPVSIEHADIRVRNYSVNSRERYVCNSGFRRRAGTSTLIECVINRNTNVAHWTTPSLRCIRDPSLAGGGGSGGGGSGGGGSGGGGSNWIDVRYDLERIESLIQSIHIDTTLYTDSDFHPSCRVTAMNCFLLELQVILHEYSNMTLNETVRNVLYLANSTLSSNRNVAESGCRECEELEERTFTEFLQSFIRIVQMFINTSEPRIPRPSTPPGSSREGCASRCMRYNDELERCEARMMSMSNTEEDCEQELEDLLYCLDHCHSQ

SEQ ID NO: 318 - protein, 281 aa, Artificial Sequence
  Description of Artificial Sequence: Synthetic polypeptide
DYRDEHHHHHHGSGTTCPPPVSIEHADIRVRNYSVNSRERYVCNSGFRRRAGTSTLIECVINRNTNVAHWTTPSLRCIRDPSLAGGGGSGGGGSGGGGSGGGGSNWIDVRYDLERIESLIQSIHIDTTLYTDSDFHPSCRVTAMNCFLLELQVILHEYSNMTLNETVRNVLYLANSTLSSNRNVAESGCRECEELEERTFTEFLQSFIRIVQMFINTSEPRIPRPSTPPGSSREGCASRCTRYNAELERCEARVSSMSNTEETCVQELFDLLHCVDHCVSQ

SEQ ID NO: 319 - protein, 281 aa, Artificial Sequence
  Description of Artificial Sequence: Synthetic polypeptide
DYRDEHHHHHHGSGTTCPPPVSIEHADIRVRNYSVNSRERYVCNSGFRRRAGTSTLIECVINRNTNVAHWTTPSLRCIRDPSLAGGGGSGGGGSGGGGSGGGGSNWIDVRYDLERIESLIQSIHIDTTLYTDSDFHPSCRVTAMNCFLLELQVILHEYSNMTLNETVRNVLYLANSTLSSNRNVAESGCRECEELEERTFTEFLQSFIRIVQMFINTSEPRIPRPSTPPGSSREGCASRCTRYNAELERCEARVMSMSNTEEDCEQELEDLLHCLDHCHSQ

SEQ ID NO: 320 - protein, 281 aa, Artificial Sequence
  Description of Artificial Sequence: Synthetic polypeptide
DYRDEHHHHHHGSGTTCPPPVSIEHADIRVRNYSVNSRERYVCNSGFRRRAGTSTLIECVINRNTNVAHWTTPSLRCIRDPSLAGGGGSGGGGSGGGGSGGGGSNWIDVRYDLERIESLIQSIHIDTTLYTDSDFHPSCRVTAMNCFLLELQVILHEYSNMTLNETVRNVLYLANSTLSSNRNVAESGCRECEELEERTFTEFLQSFIRIVQMFINTSEPRIPRPSTPPGSSREGCASRCMRYNDELERCEARMMSMSNTEEDCEQELEDLLYCLDHCHSQ

SEQ ID NO: 321 - protein, 303 aa, Artificial Sequence
  Description of Artificial Sequence: Synthetic polypeptide
METDTLLLWVLLLWVPGSTGDYKDEHHHHHHENLYFQGSREGCASRCTKYNAELEKCEARVSSMSNTEETCVQELFDLLHCVDHCVSQGGGGSGGGGSGTTCPPPVSIEHADIRVKNYSVNSRERYVCNSGFKRKAGTSTLIECVINKNTNVAHWTTPSLKCIRDPSLAGGGGSGGGGSGGGGSGGGGSNWIDVRYDLEKIESLIQSIHIDTTLYTDSDFHPSCKVTAMNCFLLELQVILHEYSNMTLNETVRNVLYLANSTLSSNKNVAESGCKECEELEEKTFTEFLQSFIRIVQMFINTS

SEQ ID NO: 322 - protein, 303 aa, Artificial Sequence
  Description of Artificial Sequence: Synthetic polypeptide
METDTLLLWVLLLWVPGSTGDYKDEHHHHHHENLYFQGSREGCASRCTKYNAELEKCEARVMSMSNTEEDCEQELEDLLHCLDHCHSQGGGGSGGGGSGTTCPPPVSIEHADIRVKNYSVNSRERYVCNSGFKRKAGTSTLIECVINKNTNVAHWTTPSLKCIRDPSLAGGGGSGGGGSGGGGSGGGGSNWIDVRYDLEKIESLIQSIHIDTTLYTDSDFHPSCKVTAMNCFLLELQVILHEYSNMTLNETVRNVLYLANSTLSSNKNVAESGCKECEELEEKTFTEFLQSFIRIVQMFINTS

SEQ ID NO: 323 - protein, 303 aa, Artificial Sequence
  Description of Artificial Sequence: Synthetic polypeptide
METDTLLLWVLLLWVPGSTGDYKDEHHHHHHENLYFQGSREGCASRCMKYNDELEKCEARMMSMSNTEEDCEQELEDLLYCLDHCHSQGGGGSGGGGSGTTCPPPVSIEHADIRVKNYSVNSRERYVCNSGFKRKAGTSTLIECVINKNTNVAHWTTPSLKCIRDPSLAGGGGSGGGGSGGGGSGGGGSNWIDVRYDLEKIESLIQSIHIDTTLYTDSDFHPSCKVTAMNCFLLELQVILHEYSNMTLNETVRNVLYLANSTLSSNKNVAESGCKECEELEEKTFTEFLQSFIRIVQMFINTS

SEQ ID NO: 324 - protein, 283 aa, Artificial Sequence
  Description of Artificial Sequence: Synthetic polypeptide
DYKDEHHHHHHENLYFQGSREGCASRCTKYNAELEKCEARVSSMSNTEETCVQELFDLLHCVDHCVSQGGGGSGGGGSGTTCPPPVSIEHADIRVKNYSVNSRERYVCNSGFKRKAGTSTLIECVINKNTNVAHWTTPSLKCIRDPSLAGGGGSGGGGSGGGGSGGGGSNWIDVRYDLEKIESLIQSIHIDTTLYTDSDFHPSCKVTAMNCFLLELQVILHEYSNMTLNETVRNVLYLANSTLSSNKNVAESGCKECEELEEKTFTEFLQSFIRIVQMFINTS

SEQ ID NO: 325 - protein, 283 aa, Artificial Sequence
  Description of Artificial Sequence: Synthetic polypeptide
DYKDEHHHHHHENLYFQGSREGCASRCTKYNAELEKCEARVMSMSNTEEDCEQELEDLLHCLDHCHSQGGGGSGGGGSGTTCPPPVSIEHADIRVKNYSVNSRERYVCNSGFKRKAGTSTLIECVINKNTNVAHWTTPSLKCIRDPSLAGGGGSGGGGSGGGGSGGGGSNWIDVRYDLEKIESLIQSIHIDTTLYTDSDFHPSCKVTAMNCFLLELQVILHEYSNMTLNETVRNVLYLANSTLSSNKNVAESGCKECEELEEKTFTEFLQSFIRIVQMFINTS

SEQ ID NO: 326 - protein, 283 aa, Artificial Sequence
  Description of Artificial Sequence: Synthetic polypeptide
DYKDEHHHHHHENLYFQGSREGCASRCMKYNDELEKCEARMMSMSNTEEDCEQELEDLLYCLDHCHSQGGGGSGGGGSGTTCPPPVSIEHADIRVKNYSVNSRERYVCNSGFKRKAGTSTLIECVINKNTNVAHWTTPSLKCIRDPSLAGGGGSGGGGSGGGGSGGGGSNWIDVRYDLEKIESLIQSIHIDTTLYTDSDFHPSCKVTAMNCFLLELQVILHEYSNMTLNETVRNVLYLANSTLSSNKNVAESGCKECEELEEKTFTEFLQSFIRIVQMFINTS

SEQ ID NO: 327 - protein, 303 aa, Artificial Sequence
  Description of Artificial Sequence: Synthetic polypeptide
METDTLLLWVLLLWVPGSTGDYRDEHHHHHHENLYFQGSREGCASRCTRYNAELERCEARVSSMSNTEETCVQELFDLLHCVDHCVSQGGGGSGGGGSGTTCPPPVSIEHADIRVRNYSVNSRERYVCNSGFRRRAGTSTLIECVINRNTNVAHWTTPSLRCIRDPSLAGGGGSGGGGSGGGGSGGGGSNWIDVRYDLERIESLIQSIHIDTTLYTDSDFHPSCRVTAMNCFLLELQVILHEYSNMTLNETVRNVLYLANSTLSSNRNVAESGCRECEELEERTFTEFLQSFIRIVQMFINTS

SEQ ID NO: 328 - protein, 303 aa, Artificial Sequence
  Description of Artificial Sequence: Synthetic polypeptide
METDTLLLWVLLLWVPGSTGDYRDEHHHHHHENLYFQGSREGCASRCTRYNAELERCEARVMSMSNTEEDCEQELEDLLHCLDHCHSQGGGGSGGGGSGTTCPPPVSIEHADIRVRNYSVNSRERYVCNSGFRRRAGTSTLIECVINRNTNVAHWTTPSLRCIRDPSLAGGGGSGGGGSGGGGSGGGGSNWIDVRYDLERIESLIQSIHIDTTLYTDSDFHPSCRVTAMNCFLLELQVILHEYSNMTLNETVRNVLYLANSTLSSNRNVAESGCRECEELEERTFTEFLQSFIRIVQMFINTS

SEQ ID NO: 329 - protein, 303 aa, Artificial Sequence
  Description of Artificial Sequence: Synthetic polypeptide
METDTLLLWVLLLWVPGSTGDYRDEHHHHHHENLYFQGSREGCASRCMRYNDELERCEARMMSMSNTEEDCEQELEDLLYCLDHCHSQGGGGSGGGGSGTTCPPPVSIEHADIRVRNYSVNSRERYVCNSGFRRRAGTSTLIECVINRNTNVAHWTTPSLRCIRDPSLAGGGGSGGGGSGGGGSGGGGSNWIDVRYDLERIESLIQSIHIDTTLYTDSDFHPSCRVTAMNCFLLELQVILHEYSNMTLNETVRNVLYLANSTLSSNRNVAESGCRECEELEERTFTEFLQSFIRIVQMFINTS

SEQ ID NO: 330 - protein, 283 aa, Artificial Sequence
  Description of Artificial Sequence: Synthetic polypeptide
DYRDEHHHHHHENLYFQGSREGCASRCTRYNAELERCEARVSSMSNTEETCVQELFDLLHCVDHCVSQGGGGSGGGGSGTTCPPPVSIEHADIRVRNYSVNSRERYVCNSGFRRRAGTSTLIECVINRNTNVAHWTTPSLRCIRDPSLAGGGGSGGGGSGGGGSGGGGSNWIDVRYDLERIESLIQSIHIDTTLYTDSDFHPSCRVTAMNCFLLELQVILHEYSNMTLNETVRNVLYLANSTLSSNRNVAESGCRECEELEERTFTEFLQSFIRIVQMFINTS

SEQ ID NO: 331 - protein, 283 aa, Artificial Sequence
  Description of Artificial Sequence: Synthetic polypeptide
DYRDEHHHHHHENLYFQGSREGCASRCTRYNAELERCEARVMSMSNTEEDCEQELEDLLHCLDHCHSQGGGGSGGGGSGTTCPPPVSIEHADIRVRNYSVNSRERYVCNSGFRRRAGTSTLIECVINRNTNVAHWTTPSLRCIRDPSLAGGGGSGGGGSGGGGSGGGGSNWIDVRYDLERIESLIQSIHIDTTLYTDSDFHPSCRVTAMNCFLLELQVILHEYSNMTLNETVRNVLYLANSTLSSNRNVAESGCRECEELEERTFTEFLQSFIRIVQMFINTS

SEQ ID NO: 332 - protein, 283 aa, Artificial Sequence
  Description of Artificial Sequence: Synthetic polypeptide
DYRDEHHHHHHENLYFQGSREGCASRCMRYNDELERCEARMMSMSNTEEDCEQELEDLLYCLDHCHSQGGGGSGGGGSGTTCPPPVSIEHADIRVRNYSVNSRERYVCNSGFRRRAGTSTLIECVINRNTNVAHWTTPSLRCIRDPSLAGGGGSGGGGSGGGGSGGGGSNWIDVRYDLERIESLIQSIHIDTTLYTDSDFHPSCRVTAMNCFLLELQVILHEYSNMTLNETVRNVLYLANSTLSSNRNVAESGCRECEELEERTFTEFLQSFIRIVQMFINTS

SEQ ID NO: 333 - protein, 741 aa, Artificial Sequence
  Description of Artificial Sequence: Synthetic polypeptide
MRLAVGALLVCAVLGLCLADYKDEHHHHHHGLNDIFEAQKIEWHEGGGSKTVRWCAVSEHEATKCQSFRDHMKSVIPSDGPSVACVKKASYLDCIRAIAANEADAVTLDAGLVYDAYLAPNNLKPVVAEFYGSKEDPQTFYYAVAVVKKDSGFQMNQLRGKKSCHTGLGRSAGWNIPIGLLYCDLPEPRKPLEKAVANFFSGSCAPCADGTDFPQLCQLCPGCGCSTLNQYFGYSGAFKCLKDGAGDVAFVKHSTIFENLANKADRDQYELLCLDNTRKPVDEYKDCHLAQVPSHTVVARSMGGKEDLIWELLNQAQEHFGKDKSKEFQLFSSPHGKDLLFKDSAHGFLKVPPRMDAKMYLGYEYVTAIRNLREGTCPEAPTDECKPVKWCALSHHERLKCDEWSVNSVGKIECVSAETTEDCIAKIMNGEADAMSLDGGFVYIAGKCGLVPVLAENYDKSDNCEDTPEAGYFAVAVVKKSASDLTWDNLKGKKSCHTAVGRTAGWNIPMGLLYNKINHCRFDEFFSEGCAPGSKKDSSLCKLCMGSGLNLCEPNNKEGYYGYTGAFRCLVEKGDVAFVKHQTVPQNTGGKNPDPWAKNLNEKDYELLCLDGTRKPVEEYANCHLARAPNHAVVTRKDKEACVHKILRQQQHLFGSDVTDCSGNFCLFRSETKDLLFRDDTVCLAKLHDRNTYEKYLGEEYVKAVGNLRKCSTSSLLEACTFRRPGSSELYENKPRRPYIL

SEQ ID NO: 334 - protein, 49 aa, Artificial Sequence
  Description of Artificial Sequence: Synthetic polypeptide
  MOD_RES (6)..(6): S, T, D, or N
  MOD_RES (9)..(9): A, M, I, L, or V
  MOD_RES (12)..(12): D, E, H, K, R, N, Q, S, or T
  MOD_RES (15)..(15): A, M, I, L, or V
  MOD_RES (16)..(16): D, E, N, Q, S, or T
  MOD_RES (19)..(19): D, E, N, Q, S, or T
  MOD_RES (36)..(36): A, M, I, L, or V
  MOD_RES (39)..(39): A, M, I, L, or V
  MOD_RES (40)..(40): A, M, I, L, or V
  MOD_RES (43)..(43): A, M, I, L, or V
  MOD_RES (44)..(44): D, E, N, Q, S, or T
  MOD_RES (45)..(45): H, K, R, N, Q, S, or T
  MOD_RES (47)..(47): H, K, R, N, Q, S, or T
  MOD_RES (48)..(48): S, T, D, or N
  MOD_RES (49)..(49): D, E, H, K, R, N, Q, S, or T
REGCAXRCXKYXDEXXKCXARMMSMSNTEEDCEQEXEDXXYCXXXCXXX

SEQ ID NO: 335 - protein, 49 aa, Artificial Sequence
  Description of Artificial Sequence: Synthetic polypeptide
  MOD_RES (3)..(3): Any amino acid
  MOD_RES (5)..(5): Any amino acid
  MOD_RES (6)..(6): Any amino acid
  MOD_RES (9)..(9): Any amino acid
  MOD_RES (12)..(12): Any amino acid
  MOD_RES (15)..(15): Any amino acid
  MOD_RES (16)..(16): Any amino acid
  MOD_RES (19)..(19): Any amino acid
REXCXXRCXKYXDEXXKCXARMMSMSNTEEDCEQELEDLLYCLDHCHSQ

SEQ ID NO: 336 - protein, 49 aa, Artificial Sequence
  Description of Artificial Sequence: Synthetic polypeptide
  MOD_RES (36)..(36): Any amino acid
  MOD_RES (39)..(39): Any amino acid
  MOD_RES (40)..(40): Any amino acid
  MOD_RES (43)..(43): Any amino acid
  MOD_RES (44)..(44): Any amino acid
  MOD_RES (45)..(45): Any amino acid
  MOD_RES (47)..(47): Any amino acid
  MOD_RES (48)..(48): Any amino acid
  MOD_RES (49)..(49): Any amino acid
REGCASRCMKYNDELEKCEARMMSMSNTEEDCEQEXEDXXYCXXXCXXX

SEQ ID NO: 337 - protein, 49 aa, Artificial Sequence
  Description of Artificial Sequence: Synthetic polypeptide
  MOD_RES (3)..(3): Any amino acid
  MOD_RES (5)..(5): Any amino acid
  MOD_RES (6)..(6): Any amino acid
  MOD_RES (9)..(9): Any amino acid
  MOD_RES (12)..(12): Any amino acid
  MOD_RES (15)..(15): Any amino acid
  MOD_RES (16)..(16): Any amino acid
  MOD_RES (19)..(19): Any amino acid
  MOD_RES (36)..(36): Any amino acid
  MOD_RES (39)..(39): Any amino acid
  MOD_RES (40)..(40): Any amino acid
  MOD_RES (43)..(43): Any amino acid
  MOD_RES (44)..(44): Any amino acid
  MOD_RES (45)..(45): Any amino acid
  MOD_RES (47)..(47): Any amino acid
  MOD_RES (48)..(48): Any amino acid
  MOD_RES (49)..(49): Any amino acid
REXCXXRCXKYXDEXXKCXARMMSMSNTEEDCEQEXEDXXYCXXXCXXX

SEQ ID NO: 338 - protein, 49 aa, Artificial Sequence
  Description of Artificial Sequence: Synthetic polypeptide
  MOD_RES (1)..(1): D, E, H, K, R, N, Q, S, or T
  MOD_RES (2)..(2): D, E, H, K, R, N, Q, S, or T
  MOD_RES (7)..(7): D, E, H, K, R, N, Q, S, or T
  MOD_RES (10)..(10): D, E, H, K, R, N, Q, S, or T
  MOD_RES (13)..(13): D, E, H, K, R, N, Q, S, or T
  MOD_RES (14)..(14): D, E, H, K, R, N, Q, S, or T
  MOD_RES (17)..(17): D, E, H, K, R, N, Q, S, or T
  MOD_RES (21)..(21): D, E, H, K, R, N, Q, S, or T
  MOD_RES (24)..(24): D, E, H, K, R, N, Q, S, or T
  MOD_RES (26)..(26): D, E, H, K, R, N, Q, S, or T
  MOD_RES (27)..(27): D, E, H, K, R, N, Q, S, or T
  MOD_RES (28)..(28): D, E, H, K, R, N, Q, S, or T
  MOD_RES (29)..(29): D, E, H, K, R, N, Q, S, or T
  MOD_RES (30)..(30): D, E, H, K, R, N, Q, S, or T
  MOD_RES (31)..(31): D, E, H, K, R, N, Q, S, or T
  MOD_RES (33)..(33): D, E, H, K, R, N, Q, S, or T
  MOD_RES (34)..(34): D, E, H, K, R, N, Q, S, or T
  MOD_RES (35)..(35): D, E, H, K, R, N, Q, S, or T
  MOD_RES (37)..(37): D, E, H, K, R, N, Q, S, or T
  MOD_RES (38)..(38): D, E, H, K, R, N, Q, S, or T
XXGCASXCMXYNXXLEXCEAXMMXMXXXXXXCXXXLXXLLYCLDHCHSQ

SEQ ID NO: 339 - protein, 49 aa, Artificial Sequence
  Description of Artificial Sequence: Synthetic polypeptide
  MOD_RES (13)..(13): D, E, H, K, R, N, Q, S, or T
  MOD_RES (33)..(33): D, E, H, K, R, N, Q, S, or T
  MOD_RES (37)..(37): D, E, H, K, R, N, Q, S, or T
  MOD_RES (47)..(47): D, E, H, K, R, N, Q, S, or T
REGCASRCMKYNXELEKCEARMMSMSNTEEDCXQELXDLLYCLDHCXSQ

SEQ ID NO: 340 - protein, 49 aa, Artificial Sequence; identical to SEQ ID NO: 339
  Description of Artificial Sequence: Synthetic polypeptide
  MOD_RES (13)..(13): A, M, I, L, V, F, W, or Y
  MOD_RES (33)..(33): A, M, I, L, V, F, W, or Y
  MOD_RES (37)..(37): A, M, I, L, V, F, W, or Y
  MOD_RES (47)..(47): A, M, I, L, V, F, W, or Y

SEQ ID NO: 341 - protein, 49 aa, Artificial Sequence
  Description of Artificial Sequence: Synthetic polypeptide
  MOD_RES (9)..(9): A, M, I, L, V, F, W, or Y
  MOD_RES (23)..(23): A, M, I, L, V, F, W, or Y
  MOD_RES (25)..(25): A, M, I, L, V, F, W, or Y
REGCASRCXKYNDELEKCEARMXSXSNTEEDCEQELEDLLYCLDHCHSQ

SEQ ID NO: 342 - protein, 49 aa, Artificial Sequence; identical to SEQ ID NO: 341
  Description of Artificial Sequence: Synthetic polypeptide
  MOD_RES (9)..(9): D, E, H, K, R, N, Q, S, or T
  MOD_RES (23)..(23): D, E, H, K, R, N, Q, S, or T
  MOD_RES (25)..(25): D, E, H, K, R, N, Q, S, or T

SEQ ID NO: 343 - protein, 49 aa, Artificial Sequence
  Description of Artificial Sequence: Synthetic polypeptide
  MOD_RES (43)..(43): A, M, I, L, or V
REGCASRCMKYNDELEKCEARMMSMSNTEEDCEQELEDLLYCXDHCHSQ

SEQ ID NO: 344 - protein, 49 aa, Artificial Sequence
  Description of Artificial Sequence: Synthetic polypeptide
  MOD_RES (10)..(10): K or R
  MOD_RES (17)..(17): K or R
REGCASRCMXYNDELEXCEARMMSMSNTEEDCEQELEDLLYCLDHCHSQ

SEQ ID NO: 345 - protein, 6 aa, Artificial Sequence
  Description of Artificial Sequence: Synthetic 6xHis tag
HHHHHH

SEQ ID NO: 346 - protein, 8 aa, Artificial Sequence
  Description of Artificial Sequence: Synthetic peptide
DYKDDDDK

SEQ ID NO: 347 - protein, 5 aa, Artificial Sequence
  Description of Artificial Sequence: Synthetic peptide
DYKDE

SEQ ID NO: 348 - protein, 9 aa, Artificial Sequence
  Description of Artificial Sequence: Synthetic peptide
YPYDVPDYA

SEQ ID NO: 349 - protein, 9 aa, Artificial Sequence
  Description of Artificial Sequence: Synthetic peptide
DVEAWLGAR

SEQ ID NO: 350 - protein, 13 aa, Homo sapiens
ELYENKPRRPYIL

SEQ ID NO: 351 - protein, 221 aa, Artificial Sequence
  Description of Artificial Sequence: Synthetic polypeptide
METDTLLLWVLLLWVPGSTGDYKDEHHHHHHGGSQDSTSDLIPAPPLSKVPLQQNFQDNQFQGKWYVVGLAGNAILREDKDPQKMYATIYELKEDKSYNVTSVLFRKKKCDYWIRTFVPGSQPGEFTLGNIKSYPGLTSYLVRVVSTNYNQHAMVFFKKVSQNREYFKITLYGRTKELTSELKENFIRFSKSLGLPENHIVFPVPIDQCIDGGGSENLYFQ

SEQ ID NO: 352 - protein, 891 aa, Artificial Sequence
  Description of Artificial Sequence: Synthetic polypeptide
METDTLLLWVLLLWVPGSTGDYKDEHHHHHHGGSQDSTSDLIPAPPLSKVPLQQNFQDNQFQGKWYVVGLAGNAILREDKDPQKMYATIYELKEDKSYNVTSVLFRKKKCDYWIRTFVPGSQPGEFTLGNIKSYPGLTSYLVRVVSTNYNQHAMVFFKKVSQNREYFKITLYGRTKELTSELKENFIRFSKSLGLPENHIVFPVPIDQCIDGGGSENLYFQGSRLYWDDLKRKLSEKLDSTDFTSTIKLLNENSYVPREAGSQKDENLALYVENQFREFKLSKVWRDQHFVKIQVKDSAQNSVIIVDKNGRLVYLVENPGGYVAYSKAATVTGKLVHANFGTKKDFEDLYTPVNGSIVIVRAGKITFAEKVANAESLNAIGVLIYMDQTKFPIVNAELSFFGHAHLGTGDPYTPGFPSFNHTQFPPSRSSGLPNIPVQTISRAAAEKLFGNMEGDCPSDWKTDSTCRMVTSESKNVKLTVSNVLKEIKILNIFGVIKGFVEPDHYVVVGAQRDAWGPGAAKSGVGTALLLKLAQMFSDMVLKDGFQPSRSIIFASWSAGDFGSVGATEWLEGYLSSLHLKAFTYINLDKAVLGTSNFKVSASPLLYTLIEKTMQNVKHPVTGQFLYQDSNWASKVEKLTLDNAAFPFLAYSGIPAVSFCFCEDTDYPYLGTTMDTYKELIERIPELNKVARAAAEVAGQFVIKLTHDVELNLDYERYNSQLLSFVRDLNQYRADIKEMGLSLQWLYSARGDFFRATSRLTTDFGNAEKTDRFVMKKLNDRVMRVEYHFLSPYVSPKESPFRHVFWGSGSHTLPALLENLKLRKQNNGAFNETLFRNQLALATWTIQGAANALSGDVWDIDNEFGGGSHHHHHHGGGSLNDIFEAQKIEWHE

SEQ ID NO: 353 - protein, 725 aa, Artificial Sequence
  Description of Artificial Sequence: Synthetic polypeptide
MRLAVGALLVCAVLGLCLADYKDEHHHHHHGLNDIFEAQKIEWHEGGGSKTVRWCAVSEHEATKCQSFRDHMKSVIPSDGPSVACVKKASYLDCIRAIAANEADAVTLDAGLVYDAYLAPNNLKPVVAEFYGSKEDPQTFYYAVAVVKKDSGFQMNQLRGKKSCHTGLGRSAGWNIPIGLLYCDLPEPRKPLEKAVANFFSGSCAPCADGTDFPQLCQLCPGCGCSTLNQYFGYSGAFKCLKDGAGDVAFVKHSTIFENLANKADRDQYELLCLDNTRKPVDEYKDCHLAQVPSHTVVARSMGGKEDLIWELLNQAQEHFGKDKSKEFQLFSSPHGKDLLFKDSAHGFLKVPPRMDAKMYLGYEYVTAIRNLREGTCPEAPTDECKPVKWCALSHHERLKCDEWSVNSVGKIECVSAETTEDCIAKIMNGEADAMSLDGGFVYIAGKCGLVPVLAENYDKSDNCEDTPEAGYFAVAVVKKSASDLTWDNLKGKKSCHTAVGRTAGWNIPMGLLYNKINHCRFDEFFSEGCAPGSKKDSSLCKLCMGSGLNLCEPNNKEGYYGYTGAFRCLVEKGDVAFVKHQTVPQNTGGKNPDPWAKNLNEKDYELLCLDGTRKPVEEYANCHLARAPNHAVVTRKDKEACVHKILRQQQHLFGSDVTDCSGNFCLFRSETKDLLFRDDTVCLAKLHDRNTYEKYLGEEYVKAVGNLRKCSTSSLLEACTFRRP

SEQ ID NO: 354 - protein, 727 aa, Artificial Sequence
  Description of Artificial Sequence: Synthetic polypeptide
MRLAVGALLVCAVLGLCLADYKDEHHHHHHGLNDIFEAQKIEWHEGGGSVPDKTVKWCAVSEHENTKCISFRDHMKTVLPPDGPRLACVKKTSYPDCIKAISASEADAMTLDGGWVYDAGLTPNNLKPVAAEFYGSVEHPQTYYYAVAVVKKGTDFQLNQLEGKKSCHTGLGRSAGWVIPIGLLFCKLSEPRSPLEKAVSSFFSGSCVPCADPVAFPKLCQLCPGCGCSSTQPFFGYVGAFKCLKDGGGDVAFVKHTTIFEVLPEKADRDQYELLCLDNTRKPVDQYEDCYLARIPSHAVVARKNNGKEDLIWEILKVAQEHFGKGKSKDFQLFSSPLGKDLLFKDSAFGLLRVPPRMDYRLYLGHNYVTAIRNQQEGVCPEGSIDNSPVKWCALSHLERTKCDEWSIISEGKIECESAETTEDCIEKIVNGEADAMTLDGGHAYIAGQCGLVPVMAEYYESSNCAIPSQQGIFPKGYYAVAVVKASDTSITWNNLKGKKSCHTGVDRTAGWNIPMGMLYNRINHCKFDEFFSQGCAPGYEKNSTLCDLCIGPLKCAPNNKEEYNGYTGAFRCLVEKGDVAFVKHQTVLDNTEGKNPAEWAKNLKQEDFELLCPDGTRKPVKDFASCHLAQAPNHVVVSRKEKAARVKAVLTSQETLFGGSDCTGNFCLFKSTTKDLLFRDDTKCFVKLPEGTTPEKYLGAEYMQSVGNMRKCSTSRLLEACTFHKH

SEQ ID NO: 355 - protein, 743 aa, Artificial Sequence
  Description of Artificial Sequence: Synthetic polypeptide
MRLAVGALLVCAVLGLCLADYKDEHHHHHHGLNDIFEAQKIEWHEGGGSVPDKTVKWCAVSEHENTKCISFRDHMKTVLPPDGPRLACVKKTSYPDCIKAISASEADAMTLDGGWVYDAGLTPNNLKPVAAEFYGSVEHPQTYYYAVAVVKKGTDFQLNQLEGKKSCHTGLGRSAGWVIPIGLLFCKLSEPRSPLEKAVSSFFSGSCVPCADPVAFPKLCQLCPGCGCSSTQPFFGYVGAFKCLKDGGGDVAFVKHTTIFEVLPEKADRDQYELLCLDNTRKPVDQYEDCYLARIPSHAVVARKNNGKEDLIWEILKVAQEHFGKGKSKDFQLFSSPLGKDLLFKDSAFGLLRVPPRMDYRLYLGHNYVTAIRNQQEGVCPEGSIDNSPVKWCALSHLERTKCDEWSIISEGKIECESAETTEDCIEKIVNGEADAMTLDGGHAYIAGQCGLVPVMAEYYESSNCAIPSQQGIFPKGYYAVAVVKASDTSITWNNLKGKKSCHTGVDRTAGWNIPMGMLYNRINHCKFDEFFSQGCAPGYEKNSTLCDLCIGPLKCAPNNKEEYNGYTGAFRCLVEKGDVAFVKHQTVLDNTEGKNPAEWAKNLKQEDFELLCPDGTRKPVKDFASCHLAQAPNHVVVSRKEKAARVKAVLTSQETLFGGSDCTGNFCLFKSTTKDLLFRDDTKCFVKLPEGTTPEKYLGAEYMQSVGNMRKCSTSRLLEACTFHKHGSSELYENKPRRPYIL

SEQ ID NO: 356 - protein, 272 aa, Artificial Sequence
  Description of Artificial Sequence: Synthetic polypeptide
METDTLLLWVLLLWVPGSTGDYKDEHHHHHHGGSQDSTSDLIPAPPLSKVPLQQNFQDNQFQGKWYVVGLAGNAILREDKDPQKMYATIYELKEDKSYNVTSVLFRKKKCDYWIRTFVPGSQPGEFTLGNIKSYPGLTSYLVRVVSTNYNQHAMVFFKKVSQNREYFKITLYGRTKELTSELKENFIRFSKSLGLPENHIVFPVPIDQCIDGGGSENLYFQGSREGCASRCTKYNAELEKCEARVSSMSNTEETCVQELFDLLHCVDHCVSQ

SEQ ID NO: 357 - protein, 272 aa, Artificial Sequence
  Description of Artificial Sequence: Synthetic polypeptide
METDTLLLWVLLLWVPGSTGDYKDEHHHHHHGGSQDSTSDLIPAPPLSKVPLQQNFQDNQFQGKWYVVGLAGNAILREDKDPQKMYATIYELKEDKSYNVTSVLFRKKKCDYWIRTFVPGSQPGEFTLGNIKSYPGLTSYLVRVVSTNYNQHAMVFFKKVSQNREYFKITLYGRTKELTSELKENFIRFSKSLGLPENHIVFPVPIDQCIDGGGSENLYFQGSREGCASRCTKYNAELEKCEARVMSMSNTEEDCEQELEDLLHCLDHCHSQ

SEQ ID NO: 358 - protein, 272 aa, Artificial Sequence
  Description of Artificial Sequence: Synthetic polypeptide
METDTLLLWVLLLWVPGSTGDYKDEHHHHHHGGSQDSTSDLIPAPPLSKVPLQQNFQDNQFQGKWYVVGLAGNAILREDKDPQKMYATIYELKEDKSYNVTSVLFRKKKCDYWIRTFVPGSQPGEFTLGNIKSYPGLTSYLVRVVSTNYNQHAMVFFKKVSQNREYFKITLYGRTKELTSELKENFIRFSKSLGLPENHIVFPVPIDQCIDGGGSENLYFQGSREGCASRCMKYNDELEKCEARMMSMSNTEEDCEQELEDLLYCLDHCHSQ

SEQ ID NO: 359 - protein, 288 aa, Artificial Sequence
  Description of Artificial Sequence: Synthetic polypeptide
METDTLLLWVLLLWVPGSTGDYKDEHHHHHHGGSQDSTSDLIPAPPLSKVPLQQNFQDNQFQGKWYVVGLAGNAILREDKDPQKMYATIYELKEDKSYNVTSVLFRKKKCDYWIRTFVPGSQPGEFTLGNIKSYPGLTSYLVRVVSTNYNQHAMVFFKKVSQNREYFKITLYGRTKELTSELKENFIRFSKSLGLPENHIVFPVPIDQCIDGGGSENLYFQGSREGCASRCTKYNAELEKCEARVSSMSNTEETCVQELFDLLHCVDHCVSQGSSELYENKPRRPYIL

SEQ ID NO: 360 - protein, 288 aa, Artificial Sequence
  Description of Artificial Sequence: Synthetic polypeptide
METDTLLLWVLLLWVPGSTGDYKDEHHHHHHGGSQDSTSDLIPAPPLSKVPLQQNFQDNQFQGKWYVVGLAGNAILREDKDPQKMYATIYELKEDKSYNVTSVLFRKKKCDYWIRTFVPGSQPGEFTLGNIKSYPGLTSYLVRVVSTNYNQHAMVFFKKVSQNREYFKITLYGRTKELTSELKENFIRFSKSLGLPENHIVFPVPIDQCIDGGGSENLYFQGSREGCASRCTKYNAELEKCEARVMSMSNTEEDCEQELEDLLHCLDHCHSQGSSELYENKPRRPYIL

SEQ ID NO: 361 - protein, 288 aa, Artificial Sequence
  Description of Artificial Sequence: Synthetic polypeptide
METDTLLLWVLLLWVPGSTGDYKDEHHHHHHGGSQDSTSDLIPAPPLSKVPLQQNFQDNQFQGKWYVVGLAGNAILREDKDPQKMYATIYELKEDKSYNVTSVLFRKKKCDYWIRTFVPGSQPGEFTLGNIKSYPGLTSYLVRVVSTNYNQHAMVFFKKVSQNREYFKITLYGRTKELTSELKENFIRFSKSLGLPENHIVFPVPIDQCIDGGGSENLYFQGSREGCASRCMKYNDELEKCEARMMSMSNTEEDCEQELEDLLYCLDHCHSQGSSELYENKPRRPYIL

SEQ ID NO: 362 - protein, 51 aa, Artificial Sequence
  Description of Artificial Sequence: Synthetic polypeptide
GSREGCASHCTKYKAELEKCEARVSSRSNTEETCVQELFDFLHCVDHCVSQ

SEQ ID NO: 363 - protein, 760 aa, Homo sapiens
MMDQARSAFSNLFGGEPLSYTRFSLARQVDGDNSHVEMKLAVDEEENADNNTKANVTKPKRCSGSICYGTIAVIVFFLIGFMIGYLGYCKGVEPKTECERLAGTESPVREEPGEDFPAARRLYWDDLKRKLSEKLDSTDFTGTIKLLNENSYVPREAGSQKDENLALYVENQFREFKLSKVWRDQHFVKIQVKDSAQNSVIIVDKNGRLVYLVENPGGYVAYSKAATVTGKLVHANFGTKKDFEDLYTPVNGSIVIVRAGKITFAEKVANAESLNAIGVLIYMDQTKFPIVNAELSFFGHAHLGTGDPYTPGFPSFNHTQFPPSRSSGLPNIPVQTISRAAAEKLFGNMEGDCPSDWKTDSTCRMVTSESKNVKLTVSNVLKEIKILNIFGVIKGFVEPDHYVVVGAQRDAWGPGAAKSGVGTALLLKLAQMFSDMVLKDGFQPSRSIIFASWSAGDFGSVGATEWLEGYLSSLHLKAFTYINLDKAVLGTSNFKVSASPLLYTLIEKTMQNVKHPVTGQFLYQDSNWASKVEKLTLDNAAFPFLAYSGIPAVSFCFCEDTDYPYLGTTMDTYKELIERIPELNKVARAAAEVAGQFVIKLTHDVELNLDYERYNSQLLSFVRDLNQYRADIKEMGLSLQWLYSARGDFFRATSRLTTDFGNAEKTDRFVMKKLNDRVMRVEYHFLSPYVSPKESPFRHVFWGSGSHTLPALLENLKLRKQNNGAFNETLFRNQLALATWTIQGAANALSGDVWDIDNEF

SEQ ID NO: 364 - protein, 676 aa, Homo sapiens
KTVRWCAVSEHEATKCQSFRDHMKSVIPSDGPSVACVKKASYLDCIRAIAANEADAVTLDAGLVYDAYLAPNNLKPVVAEFYGSKEDPQTFYYAVAVVKKDSGFQMNQLRGKKSCHTGLGRSAGWNIPIGLLYCDLPEPRKPLEKAVANFFSGSCAPCADGTDFPQLCQLCPGCGCSTLNQYFGYSGAFKCLKDGAGDVAFVKHSTIFENLANKADRDQYELLCLDNTRKPVDEYKDCHLAQVPSHTVVARSMGGKEDLIWELLNQAQEHFGKDKSKEFQLFSSPHGKDLLFKDSAHGFLKVPPRMDAKMYLGYEYVTAIRNLREGTCPEAPTDECKPVKWCALSHHERLKCDEWSVNSVGKIECVSAETTEDCIAKIMNGEADAMSLDGGFVYIAGKCGLVPVLAENYNKSDNCEDTPEAGYFAIAVVKKSASDLTWDNLKGKKSCHTAVGRTAGWNIPMGLLYNKINHCRFDEFFSEGCAPGSKKDSSLCKLCMGSGLNLCEPNNKEGYYGYTGAFRCLVEKGDVAFVKHQTVPQNTGGKNPDPWAKNLNEKDYELLCLDGTRKPVEEYANCHLARAPNHAVVTRKDKEACVHKILRQQQHLFGSNVTDCSGNFCLFRSETKDLLFRDDTVCLAKLHDRNTYEKYLGEEYVKAVGNLRKCSTSSLLEACTFRRP

SEQ ID NO: 365 - protein, 13 aa, Artificial Sequence
  Description of Artificial Sequence: Synthetic peptide
  MOD_RES (8)..(8): N-methyl-Arg
  MOD_RES (11)..(11): l-neo-Trp
  MOD_RES (12)..(12): tert-Leu
ELYENKPRKPWLL

SEQ ID NO: 366 - protein, 13 aa, Artificial Sequence
  Description of Artificial Sequence: Synthetic peptide
  MOD_RES (9)..(9): d-Lys
  MOD_RES (11)..(11): l-neo-Trp
  MOD_RES (12)..(12): tert-Ile
ELYENKPRKPWIL

SEQ ID NO: 367 - protein, 13 aa, Artificial Sequence
  Description of Artificial Sequence: Synthetic peptide
  MOD_RES (9)..(9): d-Orn
  MOD_RES (11)..(11): l-neo-Trp
  MOD_RES (12)..(12): tert-Leu
ELYENKPRXPWLL

SEQ ID NO: 368 - protein, 13 aa, Artificial Sequence
  Description of Artificial Sequence: Synthetic peptide
  MOD_RES (8)..(8): N-methyl-Arg
  MOD_RES (11)..(11): d-3,1-Nal
  MOD_RES (12)..(12): tert-Leu
ELYENKPRRPXLL

SEQ ID NO: 369 - protein, 13 aa, Artificial Sequence
  Description of Artificial Sequence: Synthetic peptide
  MOD_RES (8)..(8): H-Lys-psi[CH2NH]
  MOD_RES (12)..(12): Tle
  MOD_RES (13)..(13): Leu-Oet
ELYENKPKKPYXL

SEQ ID NO: 370 - protein, 7 aa, Artificial Sequence
  Description of Artificial Sequence: Synthetic peptide
ELYENKP

SEQ ID NO: 371 - protein, 13 aa, Artificial Sequence
  Description of Artificial Sequence: Synthetic peptide
  MOD_RES (8)..(8): K or R
  MOD_RES (9)..(9): K or R
  MOD_RES (11)..(11): W or Y
  MOD_RES (12)..(12): I or L
ELYENKPXXPXXL

SEQ ID NO: 372 - protein, 58 aa, Artificial Sequence
  Description of Artificial Sequence: Synthetic polypeptide
GSRLIEDICLPRWGCLWEDDGGGGSGGGGSKCLPPGKPCYGATQKIPCCGVCSHNNCT

SEQ ID NO: 373 - protein, 79 aa, Artificial Sequence
  Description of Artificial Sequence: Synthetic polypeptide
GSRLIEDICLPRWGCLWEDDGGGGSGGGGSREGCASRCMKYNDELEKCEARMMSMSNTEEDCEQELEDLLYCLDHCHSQ

SEQ ID NO: 374 - protein, 56 aa, Artificial Sequence
  Description of Artificial Sequence: Synthetic polypeptide
RLIEDICLPRWGCLWEDDGGGGSGGGGSKCLPPGKPCYGATQKIPCCGVCSHNNCT

SEQ ID NO: 375 - protein, 77 aa, Artificial Sequence
  Description of Artificial Sequence: Synthetic polypeptide
RLIEDICLPRWGCLWEDDGGGGSGGGGSREGCASRCMKYNDELEKCEARMMSMSNTEEDCEQELEDLLYCLDHCHSQ

SEQ ID NO: 376 - protein, 18 aa, Artificial Sequence
  Description of Artificial Sequence: Synthetic peptide
RLIEDICLPRWGCLWEDD

SEQ ID NO: 377 - protein, 38 aa, Artificial Sequence
  Description of Artificial Sequence: Synthetic polypeptide
GGGGSGGGGSRLIEDICLPRWGCLWEDDGGGGSGGGGS

SEQ ID NO: 378 - protein, 36 aa, Artificial Sequence
  Description of Artificial Sequence: Synthetic polypeptide
AAAISCVGSPECPPKCRAQGCKNGKCMNRKCKCYYC

SEQ ID NO: 379 - protein, 35 aa, Artificial Sequence
  Description of Artificial Sequence: Synthetic polypeptide
RSCIDTIPKSRCTAFQCKHSMKYRLSFCRKTCGTC

SEQ ID NO: 380 - protein, 104 aa, Artificial Sequence
  Description of Artificial Sequence: Synthetic polypeptide
GSAAAISCVGSPECPPKCRAQGCKNGKCMNRKCKCYYCGGGGSGGGGSRLIEDICLPRWGCLWEDDGGGGSGGGGSKCLPPGKPCYGATQKIPCCGVCSHNNCT

SEQ ID NO: 381 - protein, 125 aa, Artificial Sequence
  Description of Artificial Sequence: Synthetic polypeptide
GSAAAISCVGSPECPPKCRAQGCKNGKCMNRKCKCYYCGGGGSGGGGSRLIEDICLPRWGCLWEDDGGGGSGGGGSREGCASRCMKYNDELEKCEARMMSMSNTEEDCEQELEDLLYCLDHCHSQ

SEQ ID NO: 382 - protein, 84 aa, Artificial Sequence
  Description of Artificial Sequence: Synthetic polypeptide
GSEWSSRSCIDTIPKSRCTAFQCKHSMKYRLSFCRKTCGTCGGGGSGGGGSGGGGSKCLPPGKPCYGATQKIPCCGVCSHNNCT

SEQ ID NO: 383 - protein, 81 aa, Artificial Sequence
  Description of Artificial Sequence: Synthetic polypeptide
GSEWSSRSCIDTIPKSRCTAFQCKHSMKYRLSFCRKTCGTCKKYKPYVPVTTNKCLPPGKPCYGATQKIPCCGVCSHNNCT

SEQ ID NO: 384 - protein, 105 aa, Artificial Sequence
  Description of Artificial Sequence: Synthetic polypeptide
GSEWSSRSCIDTIPKSRCTAFQCKHSMKYRLSFCRKTCGTCGGGGSGGGGSGGGGSREGCASRCMKYNDELEKCEARMMSMSNTEEDCEQELEDLLYCLDHCHSQ

SEQ ID NO: 385 - protein, 102 aa, Artificial Sequence
  Description of Artificial Sequence: Synthetic polypeptide
GSEWSSRSCIDTIPKSRCTAFQCKHSMKYRLSFCRKTCGTCKKYKPYVPVTTNREGCASRCMKYNDELEKCEARMMSMSNTEEDCEQELEDLLYCLDHCHSQ

SEQ ID NO: 386 - protein, 81 aa, Artificial Sequence
  Description of Artificial Sequence: Synthetic polypeptide
GSAAAISCVGSPECPPKCRAQGCKNGKCMNRKCKCYYCGGGGSGGGGSGGGGSKCLPPGKPCYGATQKIPCCGVCSHNNCT

SEQ ID NO: 387 - protein, 78 aa, Artificial Sequence
  Description of Artificial Sequence: Synthetic polypeptide
GSAAAISCVGSPECPPKCRAQGCKNGKCMNRKCKCYYCKKYKPYVPVTTNKCLPPGKPCYGATQKIPCCGVCSHNNCT

SEQ ID NO: 388 - protein, 102 aa, Artificial Sequence
  Description of Artificial Sequence: Synthetic polypeptide
GSAAAISCVGSPECPPKCRAQGCKNGKCMNRKCKCYYCGGGGSGGGGSGGGGSREGCASRCMKYNDELEKCEARMMSMSNTEEDCEQELEDLLYCLDHCHSQ

SEQ ID NO: 389 - protein, 99 aa, Artificial Sequence
  Description of Artificial Sequence: Synthetic polypeptide
GSAAAISCVGSPECPPKCRAQGCKNGKCMNRKCKCYYCKKYKPYVPVTTNREGCASRCMKYNDELEKCEARMMSMSNTEEDCEQELEDLLYCLDHCHSQ

SEQ ID NO: 390 - protein, 41 aa, Artificial Sequence
  Description of Artificial Sequence: Synthetic polypeptide
GSEWSSRSCIDTIPKSRCTAFQCKHSMKYRLSFCRKTCGTC

SEQ ID NO: 391 - protein, 38 aa, Artificial Sequence
  Description of Artificial Sequence: Synthetic polypeptide
GSAAAISCVGSPECPPKCRAQGCKNGKCMNRKCKCYYC

SEQ ID NO: 392 - protein, 102 aa, Artificial Sequence
  Description of Artificial Sequence: Synthetic polypeptide
AAAISCVGSPECPPKCRAQGCKNGKCMNRKCKCYYCGGGGSGGGGSRLIEDICLPRWGCLWEDDGGGGSGGGGSKCLPPGKPCYGATQKIPCCGVCSHNNCT

SEQ ID NO: 393 - protein, 123 aa, Artificial Sequence
  Description of Artificial Sequence: Synthetic polypeptide
AAAISCVGSPECPPKCRAQGCKNGKCMNRKCKCYYCGGGGSGGGGSRLIEDICLPRWGCLWEDDGGGGSGGGGSREGCASRCMKYNDELEKCEARMMSMSNTEEDCEQELEDLLYCLDHCHSQ

SEQ ID NO: 394 - protein, 82 aa, Artificial Sequence
  Description of Artificial Sequence: Synthetic polypeptide
EWSSRSCIDTIPKSRCTAFQCKHSMKYRLSFCRKTCGTCGGGGSGGGGSGGGGSKCLPPGKPCYGATQKIPCCGVCSHNNCT

SEQ ID NO: 395 - protein, 79 aa, Artificial Sequence
  Description of Artificial Sequence: Synthetic polypeptide
EWSSRSCIDTIPKSRCTAFQCKHSMKYRLSFCRKTCGTCKKYKPYVPVTTNKCLPPGKPCYGATQKIPCCGVCSHNNCT

SEQ ID NO: 396 - protein, 103 aa, Artificial Sequence
  Description of Artificial Sequence: Synthetic polypeptide
EWSSRSCIDTIPKSRCTAFQCKHSMKYRLSFCRKTCGTCGGGGSGGGGSGGGGSREGCASRCMKYNDELEKCEARMMSMSNTEEDCEQELEDLLYCLDHCHSQ

SEQ ID NO: 397 - protein, 100 aa, Artificial Sequence
  Description of Artificial Sequence: Synthetic polypeptide
EWSSRSCIDTIPKSRCTAFQCKHSMKYRLSFCRKTCGTCKKYKPYVPVTTNREGCASRCMKYNDELEKCEARMMSMSNTEEDCEQELEDLLYCLDHCHSQ

SEQ ID NO: 398 - protein, 79 aa, Artificial Sequence
  Description of Artificial Sequence: Synthetic polypeptide
AAAISCVGSPECPPKCRAQGCKNGKCMNRKCKCYYCGGGGSGGGGSGGGGSKCLPPGKPCYGATQKIPCCGVCSHNNCT

SEQ ID NO: 399 - protein, 76 aa, Artificial Sequence
  Description of Artificial Sequence: Synthetic polypeptide
AAAISCVGSPECPPKCRAQGCKNGKCMNRKCKCYYCKKYKPYVPVTTNKCLPPGKPCYGATQKIPCCGVCSHNNCT

SEQ ID NO: 400 - protein, 100 aa, Artificial Sequence
  Description of Artificial Sequence: Synthetic polypeptide
AAAISCVGSPECPPKCRAQGCKNGKCMNRKCKCYYCGGGGSGGGGSGGGGSREGCASRCMKYNDELEKCEARMMSMSNTEEDCEQELEDLLYCLDHCHSQ

SEQ ID NO: 401 - protein, 97 aa, Artificial Sequence
  Description of Artificial Sequence: Synthetic polypeptide
AAAISCVGSPECPPKCRAQGCKNGKCMNRKCKCYYCKKYKPYVPVTTNREGCASRCMKYNDELEKCEARMMSMSNTEEDCEQELEDLLYCLDHCHSQ

SEQ ID NO: 402 - protein, 39 aa, Artificial Sequence
  Description of Artificial Sequence: Synthetic polypeptide
EWSSRSCIDTIPKSRCTAFQCKHSMKYRLSFCRKTCGTC

SEQ ID NO: 403 - protein, 16 aa, Artificial Sequence
  Description of Artificial Sequence: Synthetic peptide
RKKRRRESRKKRRRES

SEQ ID NO: 404 - protein, 18 aa, Artificial Sequence
  Description of Artificial Sequence: Synthetic peptide
RKGFYKRKQCKPSRGRKR

SEQ ID NO: 405 - protein, 34 aa, Artificial Sequence
  Description of Artificial Sequence: Synthetic polypeptide
NAATATRGRSAASRPTQRPRAPARSASRPRRPVQ

SEQ ID NO: 406 - protein, 21 aa, Artificial Sequence
  Description of Artificial Sequence: Synthetic peptide
AGYLLGKINLKALAALAKKIL

SEQ ID NO: 407 - protein, 18 aa, Artificial Sequence
  Description of Artificial Sequence: Synthetic peptide
KLALKLALKALKAALKLA

SEQ ID NO: 408 - protein, 28 aa, Artificial Sequence
  Description of Artificial Sequence: Synthetic peptide
MVKSKIGSWILVLFVAMWSDVGLCKKRP

SEQ ID NO: 409 - protein, 22 aa, Artificial Sequence
  Description of Artificial Sequence: Synthetic peptide
MVRRFLVTLRIRRACGPPRVRV

SEQ ID NO: 410 - protein, 30 aa, Artificial Sequence
  Description of Artificial Sequence: Synthetic polypeptide
WEAALAEALAEALAEHLAEALAEALEALAA

SEQ ID NO: 411 - protein, 18 aa, Artificial Sequence
  Description of Artificial Sequence: Synthetic peptide
VRLPPPVRLPPPVRLPPP

SEQ ID NO: 412 - protein, 27 aa, Artificial Sequence
  Description of Artificial Sequence: Synthetic peptide
GLAFLGFLGAAGSTMGAWSQPKKKRKV

SEQ ID NO: 413 - protein, 21 aa, Artificial Sequence
  Description of Artificial Sequence: Synthetic peptide
KETWWETWWTEWSQPKKKRKV

SEQ ID NO: 414 - protein, 8 aa, Artificial Sequence
  Description of Artificial Sequence: Synthetic peptide
WRWRWRWR

SEQ ID NO: 415 - protein, 23 aa, Artificial Sequence
  Description of Artificial Sequence: Synthetic peptide
MGLGLHLLVLAAALQGAKKKRKV

SEQ ID NO: 416 - protein, 17 aa, Artificial Sequence
  Description of Artificial Sequence: Synthetic peptide
AAVALLPAVLLAHLLAP

SEQ ID NO: 417 - protein, 26 aa, Apis mellifera
GIGAVLKVLTTGLPALISWIKRKRQQ

SEQ ID NO: 418 - protein, 20 aa, Artificial Sequence
  Description of Artificial Sequence: Synthetic peptide
HGLASTLTRWAHYNALIRAF

SEQ ID NO: 419 - protein, 13 aa, Human immunodeficiency virus
GRKKRRQRRRPPQ

SEQ ID NO: 420 - protein, 27 aa, Artificial Sequence
  Description of Artificial Sequence: Synthetic peptide
GALFLGFLGAAGSTMGAWSQPKKKRKV

SEQ ID NO: 421 - protein, 9 aa, Artificial Sequence
  Description of Artificial Sequence: Synthetic peptide
RRWWRRWRR

SEQ ID NO: 422 - protein, 13 aa, Artificial Sequence
  Description of Artificial Sequence: Synthetic peptide
CGYGPKKKRKVGG

SEQ ID NO: 423 - protein, 8 aa, Artificial Sequence
  Description of Artificial Sequence: Synthetic peptide
KKKKKKKK

SEQ ID NO: 424 - protein, 10 aa, Artificial Sequence
  Description of Artificial Sequence: Synthetic peptide
RRIPNRRPRR

SEQ ID NO: 425 - protein, 5 aa, Artificial Sequence
  Description of Artificial Sequence: Synthetic peptide
RLRWR

SEQ ID NO: 426 - protein, 20 aa, Artificial Sequence
  Description of Artificial Sequence: Synthetic peptide
KETWWETWWTEWSQPKKRKV

SEQ ID NO: 427 - protein, 18 aa, Artificial Sequence
  Description of Artificial Sequence: Synthetic peptide
QLALQLALQALQAALQLA

SEQ ID NO: 428 - protein, 26 aa, Artificial Sequence
  Description of Artificial Sequence: Synthetic peptide
DPKGDPKGVTVTVTVTVTGKGDPKPD

SEQ ID NO: 429 - protein, 24 aa, Artificial Sequence
  Description of Artificial Sequence: Synthetic peptide
RRIRPRPPRLPRPRPRPLPFPRPG

SEQ ID NO: 430 - protein, 9 aa, Artificial Sequence
  Description of Artificial Sequence: Synthetic peptide
PPRPPRPPR

SEQ ID NO: 431 - protein, 12 aa, Artificial Sequence
  Description of Artificial Sequence: Synthetic peptide
PPRPPRPPRPPR

SEQ ID NO: 432 - protein, 15 aa, Artificial Sequence
  Description of Artificial Sequence: Synthetic peptide
PPRPPRPPRPPRPPR

SEQ ID NO: 433 - protein, 18 aa, Artificial Sequence
  Description of Artificial Sequence: Synthetic peptide
PPRPPRPPRPPRPPRPPR

SEQ ID NO: 434 - protein, 24 aa, Artificial Sequence
  Description of Artificial Sequence: Synthetic peptide
GLFEAIEGFIENGWEGMIDGWYGC

SEQ ID NO: 435 - protein, 20 aa, Artificial Sequence
  Description of Artificial Sequence: Synthetic peptide
GLWRALWRLLRSLWRLLWRA

SEQ ID NO: 436 - protein, 15 aa, Artificial Sequence
  Description of Artificial Sequence: Synthetic peptide
SDLWEMMMVSLACQY

SEQ ID NO: 437 - protein, 12 aa, Artificial Sequence
  Description of Artificial Sequence: Synthetic peptide
TGNYKALHPHNG

SEQ ID NO: 438 - protein, 5 aa, Artificial Sequence
  Description of Artificial Sequence: Synthetic peptide
VPMLK

SEQ ID NO: 439 - protein, 14 aa, Artificial Sequence
  Description of Artificial Sequence: Synthetic peptide
RRRRRRGGRRRRRG

SEQ ID NO: 440 - protein, 19 aa, Artificial Sequence
  Description of Artificial Sequence: Synthetic peptide
KVKVKVKVDPPTKVKVKVK

SEQ ID NO: 441 - protein, 13 aa, Artificial Sequence
  Description of Artificial Sequence: Synthetic peptide
LAGRRRRRRRRRK

SEQ ID NO: 442 - protein, 15 aa, Artificial Sequence
  Description of Artificial Sequence: Synthetic peptide
RLWMRWYSPRTRAYG

SEQ ID NO: 443 - protein, 36 aa, Artificial Sequence
  Description of Artificial Sequence: Synthetic polypeptide
KKKKKKKKKKKKKKKKLRVRLASHLRKLRKRLLRDA

SEQ ID NO: 444 - protein, 19 aa, Artificial Sequence
  Description of Artificial Sequence: Synthetic peptide
TFFYGGSRGKRNNFKTEEY

SEQ ID NO: 445 - protein, 23 aa, Artificial Sequence
  Description of Artificial Sequence: Synthetic peptide
EEEEEEEEPLGLAGRRRRRRRRN

SEQ ID NO: 446 - protein, 23 aa, Artificial Sequence
  Description of Artificial Sequence: Synthetic peptide
KAFAKLAARLYRKALARQLGVAA

SEQ ID NO: 447 - protein, 24 aa, Homo sapiens
LGTYTQDFNKFHTFPQTAIGVGAP

SEQ ID NO: 448 - protein, 34 aa, Artificial Sequence
  Description of Artificial Sequence: Synthetic polypeptide
DAATATRGRSAASRPTQRPRAPARSASRPRRPVE

SEQ ID NO: 449 - protein, 27 aa, Artificial Sequence
  Description of Artificial Sequence: Synthetic peptide
GALFLGFLGAAGSTMGAWSQPKSKRKV

SEQ ID NO: 450 - protein, 16 aa, Homo sapiens
KPKRKRRKKKGHGWSR

SEQ ID NO: 451 - protein, 7 aa, Artificial Sequence
  Description of Artificial Sequence: Synthetic peptide
SGTQEEY

SEQ ID NO: 452 - protein, 13 aa, Artificial Sequence
  Description of Artificial Sequence: Synthetic peptide
RRRRRGGRRRRRG

SEQ ID NO: 453 - protein, 18 aa, Artificial Sequence
  Description of Artificial Sequence: Synthetic peptide
KWKLFKKIGAVLKVLTTG

SEQ ID NO: 454 - protein, 11 aa, Artificial Sequence
  Description of Artificial Sequence: Synthetic peptide
YARAAARQARA

SEQ ID NO: 455 - protein, 68 aa, Artificial Sequence
  Description of Artificial Sequence: Synthetic polypeptide
MKYFTLALTLLFLLLINPCKDMNFAWAESSEKVERASPQQAKYCYEQCNVNKVPFDQCYQMCSPLERS

SEQ ID NO: 456 - protein, 67 aa, Artificial Sequence
  Description of Artificial Sequence: Synthetic polypeptide
GSRLIEDICLPRWGCLWEDDGGGGSGGGGSVRIPVSCKHSGQCLKPCKDAGMRFGKCMNGKCDCTPK

SEQ ID NO: 457 - protein, 65 aa, Artificial Sequence
  Description of Artificial Sequence: Synthetic polypeptide
RLIEDICLPRWGCLWEDDGGGGSGGGGSVRIPVSCKHSGQCLKPCKDAGMRFGKCMNGKCDCTPK